European Patent Specification EP 3 215 624 B1, published November 29, 2023. Title: Transgenic plant comprising a polynucleotide encoding a variable domain of heavy-chain antibody. Applicant: AgroSavfe N.V. The sequence listing filed with the application follows.

SEQUENCE LISTING (368 sequences)

SEQ ID NO: 1 - protein, 115 aa, Artificial Sequence
  VHH sequence 41D01
QVQLQESGGGLVQAGGSLRLSCAASGRTFSRYGMGWFRQLPGKQRELVTSITRGGTTTYADSVKGRFTISRDNAKNTVYLQMNSLKPEDTAVYYCNARSIWRDYWGQGTQVTVSS

SEQ ID NO: 2 - protein, 121 aa, Artificial Sequence
  VHH sequence 56F11
QVQLQESGGGLVQSGGSLRLSCVHSKTTFTRNAMGWYRQALGKERELVATITSGGTTNYADSVKGRFTISMDSAKNTVYLQMNSLKPEDTAVYYCNVNTRRIFGGTVREYWGQGTQVTVSS

SEQ ID NO: 3 - protein, 118 aa, Artificial Sequence
  VHH sequence 40F07
QVQLQESGGGLVQAGGSLRLSCVASGTTFSSYTMGWYRQAPGKQRELLASIEGGGNTDYADSVKGRFTISRDNARNTVYLQMNSLKTEDTAVYYCNAARTWSIFRNYWGQGTQVTVSS

SEQ ID NO: 4 - protein, 116 aa, Artificial Sequence
  VHH sequence 41D06
QVQLQESGGGLVQAGGSLRLSCAASGGIFGINAMRWYRQAPGKQRELVASISSGGNTNYSESVKGRFTISRDDANYTVYLQMNSLKPEDTAVYYCNFVRLWFPDYWGQGTQVTVSS

SEQ ID NO: 5 - protein, 121 aa, Artificial Sequence
  VHH sequence 41G10
QVQLQESGGGLVQPGGSLTLSCAATKTGFSINAMGWYRQAPGKQREMVATITSGGTTNYADSVKGRFAISRDNAKNTVSLQMNTLKPEDTALYYCNTEARRYFTRASQVYWGQGTQVTVSS

SEQ ID NO: 6 - protein, 120 aa, Artificial Sequence
  VHH sequence 41H05
QVQLQESGGGLVQPGGSLRLSCAASGGIFSINAMGWYRQDPGKQREMVATITSGANTNYTDSVKGRFTISRDNAKNTVYLQMNSLKPEDTAVYYCNAVGRRWYGGYVELWGQGTQVTVSS

SEQ ID NO: 7 - protein, 119 aa, Artificial Sequence
  VHH sequence 42C11
QVQLQESGGGLVQPGGSLRLSCAASGSIFSTYVMGWYRQAIGKQRELVATITSSGKTNYAASVKGRFTVSRDITKNTMYLQMNSLKPEDTAVYYCGADRWVLTRWSNYWGQGTQVTVSS

SEQ ID NO: 8 - protein, 116 aa, Artificial Sequence
  VHH sequence 42C12
QVQLQESGGGLVQPGGSLRLSCAASGSISSLGWYRQAPGKQREFVASATSGGDTTYADSVKGRFTISRDNSKNTVYLQMNSLKPEDTAVYYCKGQRGVAWTRKEYWGQGTQVTVSS

SEQ ID NO: 9 - protein, 119 aa, Artificial Sequence
  VHH sequence 50D03
QVQLQESGGGLVQPGGSLRLSCAASGSIFSTYAMGWYRQAIGKQRELVATITSSGKTNYAASVKGRFTISRDITKNTMYLQMNSLKPEDTAVYYCGADRWVLTRWSNYWGQGTQVTVSS

SEQ ID NO: 10 - protein, 120 aa, Artificial Sequence
  VHH sequence 50D07
QVQLQESGGGLVQPGGSLRLSCTASGNIVNIRDMGWYRQVPGKQRELVATITSDQSTNYADSVKGRFTTTRDNAKKTVYLQMDSLKPEDTAGYYCNARVRTVLRGWRDYWGQGTQVTVSS

SEQ ID NO: 11 - protein, 119 aa, Artificial Sequence
  VHH sequence 50E02
QVQLQESGGGLVQPGGSLRLSCAASGSIFSINAMGWYRQAPGKQRELVAAITSDGSTNYADSVKGRFTISRDNAKNTAYLQMNSLKPEDTAVYYCNLRRRTFLKSSDYWGQGTQVTVSS

SEQ ID NO: 12 - protein, 123 aa, Artificial Sequence
  VHH sequence 51B08
QVQLQESGGGLVQAGDSLRLSCAASGRRFGSYAMGWFRQVPGKERELVAGISSGGSTKYADSVRGRFTISRDNAKNTVSLQMKSLKPEDTAVYYCNAKYGRWTYTGRPEYDSWGQGTQVTVSS

SEQ ID NO: 13 - protein, 116 aa, Artificial Sequence
  VHH sequence 51C06
QVQLQESGGGLVQPGGSLRLSCAASGSIFSSDTMGWYRRAPGKQRELVAAITTGGNTNYADSVKGRFTISRDNAKNTVYLQMNSLQPEDTAVYYCNCRRRWSRDFWGQGTQVTVSS

SEQ ID NO: 14 - protein, 119 aa, Artificial Sequence
  VHH sequence 51C08
QVQLQESGGGLVQPGGSLRLSCAASGTIFSIKTMGWYRQAPGKQRELVATISNGGSTNYADSVKGRFTISRDNAKNTVYLQMNSLKPEDTAVYYCNARQQFIGAPYEYWGQGTQVTVSS

SEQ ID NO: 15 - protein, 115 aa, Artificial Sequence
  VHH sequence 52A01
QVQLQESGGGLVQAGGSLRLSCTASGAITFSLGTMGWYRQAPGKQRELVASISTGSTNYADSVKGRFTISRDIIKNILYLQMNSLKPEDTAVYSCNARLLWSNYWGQGTQVTVSS

SEQ ID NO: 16 - protein, 117 aa, Artificial Sequence
  VHH sequence 52B01
QVQLQESGGGLVQAGESLRLSCAASGSTFSINVMGWYRQAPGEQRELVATISRGGSTNYADSVKGRFTISRDNAKVTVYLQMDSLKPEDTAVYYCNAAGWVGVTNYWGQGTQVTVSS

SEQ ID NO: 17 - protein, 117 aa, Artificial Sequence
  VHH sequence 52G05
QVQLQESGGGLVQAGGSLRLSCAASGSTGSISAMGWYRQAPGKQRELVASITRRGSTNYADSVKDRFTISRDNAWNTVYLQMNSLKPEDTAVYYCNARRYYTRNDYWGQGTQVTVSS

SEQ ID NO: 18 - protein, 114 aa, Artificial Sequence
  VHH sequence 53A01
QVQLQESGGGLGQAGGSLRLSCEVSGTTFSINTMGWHRQAPGKQRELVASISSGGWTNYADSVKGRFTISRDNAKKTVYLQMNNLKPEDTAVYYCRWGAIGNWYGQGTQVTVSS

SEQ ID NO: 19 - protein, 117 aa, Artificial Sequence
  VHH sequence 53F05
QVQLQESGGGLVQPGGSLRLSCAASVRIFGLNAMGWYRQGPGKQRELVASITTGGSTNYAEPVKGRFTISRDNANNTVYLQMNNLKPEDTAVYYCNAERRWGLPNYWGQGTQVTVSS

SEQ ID NO: 20 - protein, 126 aa, Artificial Sequence
  VHH sequence 54A02
QVQLQESGGGLVEAGGSLRLSCAASGRTFSRYGMGWFRQAPGKEREFVAANRWSGGSTYYADSVRGRFTISRDNAKNTVYLQMNSLKPEDTAVYYCAAYAHITAWGMRNDYEYDYWGQGTQVTVSS

SEQ ID NO: 21 - protein, 125 aa, Artificial Sequence
  VHH sequence 54B01
QVQLQESGGGLVQAGGSLRLSCAATGRTFSRYTMGWFRQAPGKERDFVAGITWTGGSTDYADSVKGRFTISRDNAKNTVYLQMNSLKPEDTAVYYCAAGNLLRLAGQLRRGYDSWGQGTQVTVSS

SEQ ID NO: 22 - protein, 129 aa, Artificial Sequence
  VHH sequence 54C01
QVQLQESGGGLVQAGGSLRLSCAASGRTGSRYAMGWFRQAPGKEREFVAAISWSGGSTYYADSVKDRFTISRDNAKNTVYLQMHSLKPEDTAVYYCATRNRAGPHYSRGYTAGQEYDYWGQGTQVTVSS

SEQ ID NO: 23 - protein, 121 aa, Artificial Sequence
  VHH sequence 54C04
QVQLQESGGGLVQPGGSLRLSCAASGRIFSINAMGWYRQGPGKERELVVDMTSGGSINYADSVSGRFTISRDNAKNTVYLQMNSLKPEDTAVYYCHANLRTAFWRNGNDYWGQGTQVTVSS

SEQ ID NO: 24 - protein, 115 aa, Artificial Sequence
  VHH sequence 54C08
QVQLQESGGGLVQPGGSLRLSCAASGSISSINAMGWYRQAPGKQRELVASITSGGSTNYADSVKGRFTISRDNAKNTVNLQMNSLKPEDTAVYYCSAGPWYRRSWGRGTQVTVSS

SEQ ID NO: 25 - protein, 116 aa, Artificial Sequence
  VHH sequence 54C10
QVQLQESGGGLVQPGESLRLSCAASASIFWVNDMGWYRQAPGKQRELVAQITRRGSTNYADSVKGRFTISRDNAKDEVYLQMNSLKPEDTAVYYCNADLAVRGRYWGQGTQVTVSS

SEQ ID NO: 26 - protein, 119 aa, Artificial Sequence
  VHH sequence 54C11
QVQLQESGGGLVQPGGSLRLSCAASGSFFPVNDMAWYRQALGNERELVANITRGGSTNYADSVKGRFTISRDNAKNTVYLQMNTLKPEDTAVYYCNVRIGFGWTAKAYWGQGTQVTVSS

SEQ ID NO: 27 - protein, 116 aa, Artificial Sequence
  VHH sequence 54D03
QVQLQESGGGLVQPGGSLRLSCAASGGIFGINAMRWYRQAPGKQRELVASISSGGNTNYSESVKGRFTISRDDANYTVYLQMNSLKPEDTAVYYCNFVRLWFPDYWGQGTQVTVSS

SEQ ID NO: 28 - protein, 116 aa, Artificial Sequence
  VHH sequence 54D06
QVQLQESGGGLVQPGGSLRLSCAASGSTIRINAMGWYRQAPGKQRELVATITRGGITNYADSVKGRFTISRDNAKFTVYLQMNSLKPEDTAVYYCNARSWVGPEYWGQGTQVTVSS

SEQ ID NO: 29 - protein, 120 aa, Artificial Sequence
  VHH sequence 54D10
QVQLQESGGGLVQPGGSLRLSCAASGMTYSIHAMGWYRQAPGKERELVAITSTSGTTDYTDSVKGRFTISRDGANNTVYLQMNSLKSEDTAVYYCHVKTRTWYNGKYDYWGQGTQVTVSS

SEQ ID NO: 30 - protein, 117 aa, Artificial Sequence
  VHH sequence 54E01
QVQLQESGGGLVQPGGSLRLSCTASGSIFSINPMGWYRQAPGKQRELVAAITSGGSTNYADYVKGRFTISRDNAKNVVYLQMNSLKPEDTAVYYCNGRSTLWRRDYWGQGTQVTVSS

SEQ ID NO: 31 - protein, 117 aa, Artificial Sequence
  VHH sequence 54E05
QVQLQESGGGLVQPGGSLRLSCAASGSIFSINTMGWYRQAPGKQRELVAAITNRGSTNYADFVKGRFTISRDNAKNTVYLQMNSLKPDDTAVYYCNAHRSWPRYDSWGQGTQVTVSS

SEQ ID NO: 32 - protein, 118 aa, Artificial Sequence
  VHH sequence 54E10
QVQLQESGGGLVQPGGSLRLSCAASGSIFSFNAMGWYRQAPGKQRELVAAITRGGSTNYADSVKGRFTISRDNANNTVYLQMNSLKPEDTAVYYCNAESRIFRRYDYWGPGTQVTVSS

SEQ ID NO: 33 - protein, 115 aa, Artificial Sequence
  VHH sequence 54F01
QVQLQESGGGLVQPGGSLRLSCVTSGSIFGLNLMGWYRQAPGKQRELVATITRGGSTNYADSVKGRFTISRDNAKKTVYLQMNSLKPEDTAVYYCNVDRGWSSYWGQGTQVTVSS

SEQ ID NO: 34 - protein, 119 aa, Artificial Sequence
  VHH sequence 54F02
QVQLQESGGGLVQPGGSLRLSCVTSGSIRSINTMGWYRQAPGNERELVATITSGGTTNYADSVKNRFTISRDNAKNTVYLQMNSLKPEDTAVYYCNLHQRAWARSYVYWGQGTQVTVSS

SEQ ID NO: 35 - protein, 117 aa, Artificial Sequence
  VHH sequence 54G01
QVQLQESGGGSVQPGGSLRLSCAASGSIFAVNAMGWYRQAPGHQRELVAIISSNSTSNYADSVKGRFTISRDNAKNTVYLQMNSLKPEDTAVYFCYAKRSWFSQEYWGQGTQVTVSS

SEQ ID NO: 36 - protein, 121 aa, Artificial Sequence
  VHH sequence 54G08
QVQLQESGGGLVQPGGSLRLSCAASGSIFSFNLMGWYRQAPGKQRELVAAITSSSNTNYADSVKGRFTISRDNAKNTVYLQMNSLKPEDTAVYYCNAQYTITPWGIKKDYWGQGTQVTVSS

SEQ ID NO: 37 - protein, 120 aa, Artificial Sequence
  VHH sequence 54G09
QVQLQESGGGLMQPGGSLRLSCTASGNIVNIRDMGWYRQVPGKQRELVATITSDQSTNYADSVKGRFTTTRDNAKKTVYLQMDSLKPEDTAGYYCNARVRTVLRGWRDYWGQGTQVTVSS

SEQ ID NO: 38 - protein, 117 aa, Artificial Sequence
  VHH sequence 55B02
QVQLQESGGGLVQPGESLRLSCVGSGSIFNINSMNWYRQASGKQRELVADMRSDGSTNYADSVKGRFTISRDNARKTVYLQMNSLKPEDTAVYYCHANSIFRSRDYWGQGTQVTVSS

SEQ ID NO: 39 - protein, 125 aa, Artificial Sequence
  VHH sequence 55B05
QVQLQESGGGVVQAGDSLRLSCAASGRTFGGYTVAWFRQAPGKEREFVARISWSGIMAYYAESVKGRFTISRDNAKNTVYLQMNSLKPEDTAVYYCASRSQIRSPWSSLDDYDRWGQGTQVTVSS

SEQ ID NO: 40 - protein, 116 aa, Artificial Sequence
  VHH sequence 55C05
QVQLQESGGGLVQPGGSLRLSCVVSGSISSMKAMGWHRQAPGKERELVAQITRGDSTNYADSVKGRFTISRDNAKNTVYLQMNSLKPDDTGVYYCNADRFFGRDYWGKGTQVTVSS

SEQ ID NO: 41 - protein, 120 aa, Artificial Sequence
  VHH sequence 55D08
QVQLQESGGGLVQPGGSLRLSCAASRSILSISAMGWYRQGPGKQREPVATITSAGSSNYSDSVKGRFTISRDNAKNTAYLQMNSLKPEDTAVYYCKTVYSRPLLGPLEVWGQGTQVTVSS

SEQ ID NO: 42 - protein, 115 aa, Artificial Sequence
  VHH sequence 55E02
QVQLQESGGGLVQTGGSLRLSCVASGSMFSSNAMAWYRQAPGKQRELVARILSGGSTNYADSVKGRFTISRGNAKNTVYLQMNSLKPEDTAVYYCNAVRYLVNYWGQGTQVTVSS

SEQ ID NO: 43 - protein, 121 aa, Artificial Sequence
  VHH sequence 55E07
QVQLQESGGGSVQVGDSLTLSCVASGRSLDIYGMGWFRQAPGKEREFVARITSGGSTYYADSVKGRFTLSRDNAKNTVYLQMNSLKPEDTAVYYCAAGVVVATSPKFYAYWGQGTQVTVSS

SEQ ID NO: 44 - protein, 116 aa, Artificial Sequence
  VHH sequence 55E09
QVQLQESGGGLVQAGGSLRLSCAASKRIFSTYTMGWFRQAPGKEREFVAAIIWSGGRTRYADSVKGRFTISRDNARNTVHLQMNSLEPEDTAVYYCYTRRLGTGYWGQGTQVTVSS

SEQ ID NO: 45 - protein, 115 aa, Artificial Sequence
  VHH sequence 55E10
QVQLQESGGGLVQAGGSLRLSCAASGSTFSIQTIGWYRQAPGKQRDRVATISSGGSTNYADSVKGRFTISRDNAKKTVYLQMNNLKPEDTAVYYCNLRYWFRDYWGQGTQVTVSS

SEQ ID NO: 46 - protein, 115 aa, Artificial Sequence
  VHH sequence 55F04
QVQLQESGGGLVQPGGSLRLSCAASGSTFSINVRGWYRQAPGKQRELVATITSDGSTNYADSVKGRFTISRDNAKNTAYLQMNSLKPEDTAVYYCNAVRLFRQYWGQGTQVTVSS

SEQ ID NO: 47 - protein, 125 aa, VHH sequence 55F09
QVQLQESGGGLVQPGGSLRLSCAASGSIFRLNAMGWYRQAPGKQRELVAAITPGGGNTTYADSVKGRFTISRDNALNTIYLQMNSLKPEDTAVYYCNAGGSSRWYSSRYYPGGYWGQGTQVTVSS

SEQ ID NO: 48 - protein, 126 aa, Artificial Sequence
  VHH sequence 55F10
QVQLQESGGGLVQAGGSLRLSCATSGGTFSRYAMGWFRQAPGKERELVATIRRSGSSTYYLDSTKGRFTISRDNAKNTVYLQMNSLKLEDTAVYYCAADSSARALVGGPGNRWDYWGQGTQVTVSS

SEQ ID NO: 49 - protein, 118 aa, Artificial Sequence
  VHH sequence 55G02
QVQLQESGGGLVQPGGSLRLSCAASGSIGSINVMGWYRQYPGKQRELVAFITSGGITNYTDSVKGRFAISRDNAQNTVYLQMNSLTPEDTAVYYCHLKNAKNVRPGYWGQGTQVTVSS

SEQ ID NO: 50 - protein, 116 aa, Artificial Sequence
  VHH sequence 55G08
QVQLQESGGGLVQPGGSLRLSCRASGGIFGINAMRWYRQAPGKQRELVASISSGGTTDYVESVKGRFTISRDNATNTVDLQMSALKPEDTAVYYCNFVRFWFPDYWGQGTQVTVSS

SEQ ID NO: 51 - protein, 116 aa, Artificial Sequence
  VHH sequence 56A05
QVQLQESGGGLVQAGGSLRLSCAASGITFMSNTMGWYRQAPGKQRELVASISSGGSTNYADSVKGRFTISRDNAKKTVYLQMNSLKPEDTAVYYCNARRNVFISSWGQGTQVTVSS

SEQ ID NO: 52 - protein, 114 aa, Artificial Sequence
  VHH sequence 56A06
QVQLQESGGGLVQPGGSLRLSCVASGSISVYGMGWYRQAPGKQRELVARITNIGTTNYADSVKGRFTISRDNAKNTVYLQMNSLQPEDTAVYYCNLRRLGRDYWGQGTQVTVSS

SEQ ID NO: 53 - protein, 118 aa, VHH sequence 56A09
QVQLQESGGGLVQPGGSLRLSCAASRTALRLNSMGWYRQAPGSQRELVATITRGGTTNYADSVKGRFTISREIGNNTVYLQMNSLEPEDTAVYYCNANFGILVGREYWGKGTQVTVSS

SEQ ID NO: 54 - protein, 116 aa, Artificial Sequence
  VHH sequence 56C09
QVQLQESGGGLVQAGGSLRLSCAVSGSIFSILSMAWYRQTPGKQRELVANITSVGSTNYADSVKGRFTISRDIAKKTLYLQMNNLKPEDTAIYYCNTRMPFLGDSWGQGTQVTVSS

SEQ ID NO: 55 - protein, 111 aa, Artificial Sequence
  VHH sequence 56C12
QVQLQESGGGLVQAGGSLRLSCAVSAFSFSNRAVSWYRQAPGKSREWVASISGIRITTYTNSVKGRFIISRDNAKKTVYLQMNDLRPEDTGVYRCYMNRYSGQGTQVTVSS

SEQ ID NO: 56 - protein, 117 aa, Artificial Sequence
  VHH sequence 56D06
QVQLQESGGGSVQPGGSLRLSCAASGTVFFSISAMGWYRQAPGKQRELVAGISRGGSTKYGDFVKGRFTISRDNGKKTIWLQMNNLQPEDTAIYYCRLTSITGTYLWGQGTQVTVSS

SEQ ID NO: 57 - protein, 114 aa, Artificial Sequence
  VHH sequence 56D07
QVQLQESGGGLVQPGGSLRLSCAASGSIFSMKVMGWYRQGPGKLRELVAVITSGGRTNYAESVKGRFTISRDNAKNTVSLQMNSLQPEDTAVYYCYYKTIRPYWGQGTQVTVSS

SEQ ID NO: 58 - protein, 120 aa, Artificial Sequence
  VHH sequence 56D10
QVQLQESGGGLVQAGGSLRLSCAASGITFRITTMGWYRQAPGKQRELVASSSSGGTTNYASSVKGRFTISRDNAKNTVYLQMNSLRPEDTAVYYCNARKFITTPWSTDYWGQGTQVTVSS

SEQ ID NO: 59 - protein, 116 aa, Artificial Sequence
  VHH sequence 56E04
QVQLQESGGGLVQPGDSLRLSCTPSGSIFNHKATGWYRQAPGSQRELVAKITTGGTTNYADSVKGRFTISRDNAKNTVYLQMSSLKPEDTAVYYCNAERYFATTLWGQGTQVTVSS

SEQ ID NO: 60 - protein, 119 aa, Artificial Sequence
  VHH sequence 56E05
QVQLQESGGGLVQAGGSLRLSCAASGITFSNNAGGWYRQAPGQQRELVARISSGGNTNYTDSVKGRFTISRDITKNTLSLQMNNLKPEDSAVYYCNAQRRVILGPRNYWGQGTQVTVSS

SEQ ID NO: 61 - protein, 121 aa, Artificial Sequence
  VHH sequence 56E08
QVQLQESGGGLVQAGGSLRLSCAASGNIFRINDMGWYRQAPGNQRELVATITSANITNYADSVKGRFTISRDNAKNTVYLQMNSLNPEDTAVYYCTAQAKKWRIGPWSDYWGQGTQVTVSS

SEQ ID NO: 62 - protein, 119 aa, Artificial Sequence
  VHH sequence 56F07
QVQLQESGGGLVQPGGSLRLSCAASGRIFSINDMAWYRQAPGKQRELVAIITNDDSTTYADSVKGRFTISRDNAKNTVYLQMNSLKPEDTAVYYCNADINTAIWRRKYWGQGTQVTVSS

SEQ ID NO: 63 - protein, 115 aa, Artificial Sequence
  VHH sequence 56G07
QVQLQESGGGLVQPGGSLRLSCAVSGSRIFIHDMGWHRQAPGEPRELVATITPFGRRNYSEYVKGRFTVSRDIARNTMSLQMSNLKAEDTGMYYCNVRVNGVDYWGQGTQVTVSS

SEQ ID NO: 64 - protein, 119 aa, Artificial Sequence
  VHH sequence 56G08
QVQLQESGGGLVQAGGSLRLSCAISGITFRRPFGISRMGWYRQAPGKERELVATLSRAGTSRYVDSVKGRFTISRDDAKNTLYLQMVSLNPEDTAVYYCYIAQLGTDYWGQGTQVTVSS

SEQ ID NO: 65 - protein, 117 aa, Artificial Sequence
  VHH sequence 56G10
QVQLQESGGGLVQAGGSLRLSCVASGITLRMYQVGWYRQAPGKQRELVAEISSRGTTMYADSVKGRFTISRDGAKNIVYLQMNSLEPEDTAVYYCNARAFAFGRNSWGQGTQVTVSS

SEQ ID NO: 66 - protein, 118 aa, VHH sequence 56H04
QVQLQESGGGSVQAGGSLRLSCAVSGGTFSNKAMGWYRQSSGKQRALVARISTVGTAHYADSVKGRFTVSKDNAGNTLYLQMNSLKPEDTAVYYCNAQAGRLYLRNYWGQGTQVTVSS

SEQ ID NO: 67 - protein, 119 aa, Artificial Sequence
  VHH sequence 56H05
QVQLQESGGGLVQPGESLRLSCVAAASTSITTFNTMAWYRQAPGKQRELVAQINNRDNTEYADSVKGRFIISRGNAKNTSNLQMNDLKSEDTGIYYCNAKRWSWSTGFWGQGTQVTVSS

SEQ ID NO: 68 - protein, 114 aa, Artificial Sequence
  VHH sequence 56H07
QVQLQESGGGLVQAGGSLRLSCTASGLTFALGTMGWYRQAPGKQRELVASISTGSTNYADSVKGRFTISRDIIKNILYLQMNSLKPEDTAVYSCNARLWWSNYWGQGTQVTVSS

SEQ ID NO: 69 - protein, 118 aa, Artificial Sequence
  VHH sequence 56H08
QVQLQESGGGLVQAGGSLRLSCTASGRTSSVNPMGWYRQAPGKQRELVAVISSDGSTNYADSVKGRFTVSRDNAKNTLYLQMNSLKPEDTAVYYCNANRRWSWGSEYWGQGTQVTVSS

SEQ ID NO: 70 - protein, 119 aa, Artificial Sequence
  VHH sequence 57A06
QVQLQESGGGLVQAGGSLRLSCAASGITFTNNAGGWYRQAPGQQRELVARISSGGNTNYTDSVKGRFTISRDITKNTLSLQMNNLKPEDSAVYYCNAQRRVILGPRNYWGQGTQVTVSS

SEQ ID NO: 71 - protein, 116 aa, Artificial Sequence
  VHH sequence 57B01
QVQLQESGGGLVQAGGSLRLSCEAPVSTFNINAMAWYRQAPGKSRELVARISSGGSTNYADSVKGRFTISRDNAKNTVYLQMNSLKPEDTAVYICYVNRHWGWDYWGQGTQVTVSS

SEQ ID NO: 72 - protein, 122 aa, Artificial Sequence
  VHH sequence 57B07
QVQLQESGGGLVQPGGTLRLSCVASGSFRSINAMGWYRQAPGKQRELVATVDSGGYTNYADSVKGRFTISRDNAKNTVYLQMSSLTPEDTAVYYCYAGIYKWPWSVDARDYWGQGTQVTVSS

SEQ ID NO: 73 - protein, 117 aa, Artificial Sequence
  VHH sequence 57B11
QVQLQESGGGLVQAGGSLRLSCAASGSSISMNSMGWYRQAPGKERERVALIRSSGGTYYADSVKGRFTISRDNAKNTVYLQMNNLKPEDTAVYYCQARRTWLSSESWGQGTQVTVSS

SEQ ID NO: 74 - protein, 122 aa, Artificial Sequence
  VHH sequence 57C07
QVQLQESGGGLVQAGGSLRLSCAVSGSTFGINTMGWYRQAPEKQRELVASISRGGMTNYADSVKGRFIISRDNAKNTVYLQMNSLKPEDTAVYVCNAGIRSRWYGGPITTYWGQGTQVTVSS

SEQ ID NO: 75 - protein, 121 aa, Artificial Sequence
  VHH sequence 57C09
QVQLQESGGGLVQAGGSLRLSCAASGSTGSINAMGWYRQGPGKQRDLVASISSGGATNYADSVKGRFTISRDNSKNTVYLQMSSLKPEDTAVYYCNAKKSRWSWSIVHDYWGQGTQVTVSS

SEQ ID NO: 76 - protein, 118 aa, Artificial Sequence
  VHH sequence 57D02
QVQLQESGGGSVQTGGSLTLSCTTSGSIFGRSDMGWYRQAPGKQRELVATITRRSRTNYAEFVKGRFTISRDSAKNLVTLQMNSLKPEDTNVYYCNARWGAGGIFSTWGQGTQVTVSS

SEQ ID NO: 77 - protein, 120 aa, Artificial Sequence
  VHH sequence 57D09
QVQLQESGGGLVQPGESLRLSCAASGSMSIDAMGWYRQAPGDQRELVASITTGGSTNYADSVKGRFTISRDNAKNTVWLQMNSLKPEDTAVYYCNAKVRLRWFRPPSDYWGQGTQVTVSS

SEQ ID NO: 78 - protein, 122 aa, Artificial Sequence
  VHH sequence 57D10
QVQLQESGGGLVQPGGSLRLSCAASGRLLSISTMGWYRRTPEDQREMVASITKDGTTNYADSVKGRLTISRDNAKNTVYLQMNSLKPDDTAVYVCNARATTWVPYRRDAEFWGQGTQVTVSS

SEQ ID NO: 79 - protein, 120 aa, Artificial Sequence
  VHH sequence 57E07
QVQLQESGGGLVQAGGSLRLSCAASGSIFGINDMGWYRQAPGKQRDLVADITRSGSTHYVDSVKGRFTISRDNAKNTVYLQMNSLKPEDTAVYYCNADSGSHWWNRRDYWGQGTQVTVSS

SEQ ID NO: 80 - protein, 118 aa, Artificial Sequence
  VHH sequence 57E11
QVQLQESGGGLVQPGGSLKLSCAASGFTFSINTMGWYRQAPGKQRELVARISRLRVTNYADSVKGRFTISRDNAKNTVYLQMNSLKPEDTAVYYCNAANWGLAGNEYWGQGTQVTVSS

SEQ ID NO: 81 - protein, 116 aa, Artificial Sequence
  VHH sequence 57G01
QVQLQESGGGLVQAGGSLRPSCTASGSTLLINSMGWYRQAPGKQRELVATISNSGTTNYVDAVKGRFAISRDNANHTVYLQMNSLEPEDTAVYYCNAQTFWRRNYWGQGTQVTVSS

SEQ ID NO: 82 - protein, 116 aa, Artificial Sequence
  VHH sequence 57G07
QVQLQESGGGLVQAGGSLRLSCAVSGSTSRINAMGWYRQAPGKKRESVATIRRGGNTKYADSVKGRFTISRDNANNTVYLQLNSLKPEDTAVYYCNAHSWLDYDYWGRGTQVTVSS

SEQ ID NO: 83 - protein, 114 aa, Artificial Sequence
  VHH sequence 57G08
QVQLQESGGGLVQAGGSLRLSCASRRRINGITMGWYRQAPGKQRELVATIDIHNSTKYADSVKGRFIISRDNGKSMLYLQMNSLKPEDTAVYYCNRIPTFGRYWGQGTQVTVSS

SEQ ID NO: 84 - protein, 118 aa, Artificial Sequence
  VHH sequence 57H08
QVQLQESGGGLVQAGGSLRLSCVASGSTFYTFSTKNVGWYRQAPGKQRELVAQQRYDGSTNYADSLQGRFTISRDNAKRTVYLQMNSLKPEDTAVYICNVNRGFISYWGQGTQVTVSS

SEQ ID NO: 85 - protein, 5 aa, Artificial Sequence
  CDR1 of VHH sequence 41D01
RYGMG

SEQ ID NO: 86 - protein, 5 aa, Artificial Sequence
  CDR1 of VHH sequence 56F11
RNAMG

SEQ ID NO: 87 - protein, 5 aa, Artificial Sequence
  CDR1 of VHH sequence 40F07
SYTMG

SEQ ID NO: 88 - protein, 5 aa, Artificial Sequence
  CDR1 of VHH sequence 41D06
INAMR

SEQ ID NO: 89 - protein, 5 aa, Artificial Sequence
  CDR1 of VHH sequence 41G10
INAMG

SEQ ID NO: 90 - protein, 5 aa, Artificial Sequence
  CDR1 of VHH sequence 41H05
INAMG

SEQ ID NO: 91 - protein, 5 aa, Artificial Sequence
  CDR1 of VHH sequence 42C11
TYVMG

SEQ ID NO: 92 - protein, 5 aa, Artificial Sequence
  CDR1 of VHH sequence 42C12
ISSLG

SEQ ID NO: 93 - protein, 5 aa, Artificial Sequence
  CDR1 of VHH sequence 50D03
TYAMG

SEQ ID NO: 94 - protein, 5 aa, Artificial Sequence
  CDR1 of VHH sequence 50D07
IRDMG

SEQ ID NO: 95 - protein, 5 aa, Artificial Sequence
  CDR1 of VHH sequence 50E02
INAMG

SEQ ID NO: 96 - protein, 5 aa, Artificial Sequence
  CDR1 of VHH sequence 51B08
SYAMG

SEQ ID NO: 97 - protein, 5 aa, Artificial Sequence
  CDR1 of VHH sequence 51C06
SDTMG

SEQ ID NO: 98 - protein, 5 aa, Artificial Sequence
  CDR1 of VHH sequence 51C08
IKTMG

SEQ ID NO: 99 - protein, 5 aa, Artificial Sequence
  CDR1 of VHH sequence 52A01
LGTMG

SEQ ID NO: 100 - protein, 5 aa, Artificial Sequence
  CDR1 of VHH sequence 52B01
INVMG

SEQ ID NO: 101 - protein, 5 aa, Artificial Sequence
  CDR1 of VHH sequence 52G05
ISAMG

SEQ ID NO: 102 - protein, 5 aa, Artificial Sequence
  CDR1 of VHH sequence 53A01
INTMG

SEQ ID NO: 103 - protein, 5 aa, Artificial Sequence
  CDR1 of VHH sequence 53F05
LNAMG

SEQ ID NO: 104 - protein, 5 aa, Artificial Sequence
  CDR1 of VHH sequence 54A02
RYGMG

SEQ ID NO: 105 - protein, 5 aa, Artificial Sequence
  CDR1 of VHH sequence 54B01
RYTMG

SEQ ID NO: 106 - protein, 5 aa, Artificial Sequence
  CDR1 of VHH sequence 54C01
RYAMG

SEQ ID NO: 107 - protein, 5 aa, Artificial Sequence
  CDR1 of VHH sequence 54C04
INAMG

SEQ ID NO: 108 - protein, 5 aa, Artificial Sequence
  CDR1 of VHH sequence 54C08
INAMG

SEQ ID NO: 109 - protein, 5 aa, Artificial Sequence
  CDR1 of VHH sequence 54C10
VNDMG

SEQ ID NO: 110 - protein, 5 aa, Artificial Sequence
  CDR1 of VHH sequence 54C11
VNDMA

SEQ ID NO: 111 - protein, 5 aa, Artificial Sequence
  CDR1 of VHH sequence 54D03
INAMR

SEQ ID NO: 112 - protein, 5 aa, Artificial Sequence
  CDR1 of VHH sequence 54D06
INAMG

SEQ ID NO: 113 - protein, 5 aa, Artificial Sequence
  CDR1 of VHH sequence 54D10
IHAMG

SEQ ID NO: 114 - protein, 5 aa, Artificial Sequence
  CDR1 of VHH sequence 54E01
INPMG

SEQ ID NO: 115 - protein, 5 aa, Artificial Sequence
  CDR1 of VHH sequence 54E05
INTMG

SEQ ID NO: 116 - protein, 5 aa, Artificial Sequence
  CDR1 of VHH sequence 54E10
FNAMG

SEQ ID NO: 117 - protein, 5 aa, Artificial Sequence
  CDR1 of VHH sequence 54F01
LNLMG

SEQ ID NO: 118 - protein, 5 aa, Artificial Sequence
  CDR1 of VHH sequence 54F02
INTMG

SEQ ID NO: 119 - protein, 5 aa, Artificial Sequence
  CDR1 of VHH sequence 54G01
VNAMG

SEQ ID NO: 120 - protein, 5 aa, Artificial Sequence
  CDR1 of VHH sequence 54G08
FNLMG

SEQ ID NO: 121 - protein, 5 aa, Artificial Sequence
  CDR1 of VHH sequence 54G09
IRDMG

SEQ ID NO: 122 - protein, 5 aa, Artificial Sequence
  CDR1 of VHH sequence 55B02
INSMN

SEQ ID NO: 123 - protein, 5 aa, Artificial Sequence
  CDR1 of VHH sequence 55B05
GYTVA

SEQ ID NO: 124 - protein, 5 aa, Artificial Sequence
  CDR1 of VHH sequence 55C05
MKAMG

SEQ ID NO: 125 - protein, 5 aa, Artificial Sequence
  CDR1 of VHH sequence 55D08
ISAMG

SEQ ID NO: 126 - protein, 5 aa, Artificial Sequence
  CDR1 of VHH sequence 55E02
SNAMA

SEQ ID NO: 127 - protein, 5 aa, Artificial Sequence
  CDR1 of VHH sequence 55E07
IYGMG

SEQ ID NO: 128 - protein, 5 aa, Artificial Sequence
  CDR1 of VHH sequence 55E09
TYTMG

SEQ ID NO: 129 - protein, 5 aa, Artificial Sequence
  CDR1 of VHH sequence 55E10
IQTIG

SEQ ID NO: 130 - protein, 5 aa, Artificial Sequence
  CDR1 of VHH sequence 55F04
INVRG

SEQ ID NO: 131 - protein, 5 aa, Artificial Sequence
  CDR1 of VHH sequence 55F09
LNAMG

SEQ ID NO: 132 - protein, 5 aa, Artificial Sequence
  CDR1 of VHH sequence 55F10
RYAMG

SEQ ID NO: 133 - protein, 5 aa, Artificial Sequence
  CDR1 of VHH sequence 55G02
INVMG

SEQ ID NO: 134 - protein, 5 aa, Artificial Sequence
  CDR1 of VHH sequence 55G08
INAMR

SEQ ID NO: 135 - protein, 5 aa, Artificial Sequence
  CDR1 of VHH sequence 56A05
SNTMG

SEQ ID NO: 136 - protein, 5 aa, Artificial Sequence
  CDR1 of VHH sequence 56A06
VYGMG

SEQ ID NO: 137 - protein, 5 aa, Artificial Sequence
  CDR1 of VHH sequence 56A09
LNSMG

SEQ ID NO: 138 - protein, 5 aa, Artificial Sequence
  CDR1 of VHH sequence 56C09
ILSMA

SEQ ID NO: 139 - protein, 5 aa, Artificial Sequence
  CDR1 of VHH sequence 56C12
NRAVS

SEQ ID NO: 140 - protein, 5 aa, Artificial Sequence
  CDR1 of VHH sequence 56D06
ISAMG

SEQ ID NO: 141 - protein, 5 aa, Artificial Sequence
  CDR1 of VHH sequence 56D07
MKVMG

SEQ ID NO: 142 - protein, 5 aa, Artificial Sequence
  CDR1 of VHH sequence 56D10
ITTMG

SEQ ID NO: 143 - protein, 5 aa, Artificial Sequence
  CDR1 of VHH sequence 56E04
HKATG

SEQ ID NO: 144 - protein, 5 aa, Artificial Sequence
  CDR1 of VHH sequence 56E05
NNAGG

SEQ ID NO: 145 - protein, 5 aa, Artificial Sequence
  CDR1 of VHH sequence 56E08
INDMG

SEQ ID NO: 146 - protein, 5 aa, Artificial Sequence
  CDR1 of VHH sequence 56F07
INDMA

SEQ ID NO: 147 - protein, 5 aa, Artificial Sequence
  CDR1 of VHH sequence 56G07
IHDMG

SEQ ID NO: 148 - protein, 5 aa, Artificial Sequence
  CDR1 of VHH sequence 56G08
ISRMG

SEQ ID NO: 149 - protein, 5 aa, Artificial Sequence
  CDR1 of VHH sequence 56G10
MYQVG

SEQ ID NO: 150 - protein, 5 aa, Artificial Sequence
  CDR1 of VHH sequence 56H04
NKAMG

SEQ ID NO: 151 - protein, 5 aa, Artificial Sequence
  CDR1 of VHH sequence 56H05
FNTMA

SEQ ID NO: 152 - protein, 5 aa, Artificial Sequence
  CDR1 of VHH sequence 56H07
LGTMG

SEQ ID NO: 153 - protein, 5 aa, Artificial Sequence
  CDR1 of VHH sequence 56H08
VNPMG

SEQ ID NO: 154 - protein, 5 aa, Artificial Sequence
  CDR1 of VHH sequence 57A06
NNAGG

SEQ ID NO: 155 - protein, 5 aa, Artificial Sequence
  CDR1 of VHH sequence 57B01
INAMA

SEQ ID NO: 156 - protein, 5 aa, Artificial Sequence
  CDR1 of VHH sequence 57B07
INAMG

SEQ ID NO: 157 - protein, 5 aa, Artificial Sequence
  CDR1 of VHH sequence 57B11
MNSMG

SEQ ID NO: 158 - protein, 5 aa, Artificial Sequence
  CDR1 of VHH sequence 57C07
INTMG

SEQ ID NO: 159 - protein, 5 aa, Artificial Sequence
  CDR1 of VHH sequence 57C09
INAMG

SEQ ID NO: 160 - protein, 5 aa, Artificial Sequence
  CDR1 of VHH sequence 57D02
RSDMG

SEQ ID NO: 161 - protein, 5 aa, Artificial Sequence
  CDR1 of VHH sequence 57D09
IDAMG

SEQ ID NO: 162 - protein, 5 aa, Artificial Sequence
  CDR1 of VHH sequence 57D10
ISTMG

SEQ ID NO: 163 - protein, 5 aa, Artificial Sequence
  CDR1 of VHH sequence 57E07
INDMG

SEQ ID NO: 164 - protein, 5 aa, Artificial Sequence
  CDR1 of VHH sequence 57E11
INTMG

SEQ ID NO: 165 - protein, 5 aa, Artificial Sequence
  CDR1 of VHH sequence 57G01
INSMG

SEQ ID NO: 166 - protein, 5 aa, Artificial Sequence
  CDR1 of VHH sequence 57G07
INAMG

SEQ ID NO: 167 - protein, 5 aa, Artificial Sequence
  CDR1 of VHH sequence 57G08
GITMG

SEQ ID NO: 168 - protein, 5 aa, Artificial Sequence
  CDR1 of VHH sequence 57H08
TKNVG

SEQ ID NO: 169 - protein, 16 aa, Artificial Sequence
  CDR2 of VHH sequence 41D01
SITRGGTTTYADSVKG

SEQ ID NO: 170 - protein, 16 aa, Artificial Sequence
  CDR2 of VHH sequence 56F11
TITSGGTTNYADSVKG

SEQ ID NO: 171 - protein, 16 aa, Artificial Sequence
  CDR2 of VHH sequence 40F07
SIEGGGNTDYADSVKG

SEQ ID NO: 172 - protein, 16 aa, Artificial Sequence
  CDR2 of VHH sequence 41D06
SISSGGNTNYSESVKG

SEQ ID NO: 173 - protein, 16 aa, Artificial Sequence
  CDR2 of VHH sequence 41G10
TITSGGTTNYADSVKG

SEQ ID NO: 174 - protein, 16 aa, Artificial Sequence
  CDR2 of VHH sequence 41H05
TITSGANTNYTDSVKG

SEQ ID NO: 175 - protein, 16 aa, Artificial Sequence
  CDR2 of VHH sequence 42C11
TITSSGKTNYAASVKG

SEQ ID NO: 176 - protein, 16 aa, Artificial Sequence
  CDR2 of VHH sequence 42C12
SATSGGDTTYADSVKG

SEQ ID NO: 177 - protein, 16 aa, Artificial Sequence
  CDR2 of VHH sequence 50D03
TITSSGKTNYAASVKG

SEQ ID NO: 178 - protein, 16 aa, Artificial Sequence
  CDR2 of VHH sequence 50D07
TITSDQSTNYADSVKG

SEQ ID NO: 179 - protein, 16 aa, Artificial Sequence
  CDR2 of VHH sequence 50E02
AITSDGSTNYADSVKG

SEQ ID NO: 180 - protein, 16 aa, Artificial Sequence
  CDR2 of VHH sequence 51B08
GISSGGSTKYADSVRG

SEQ ID NO: 181 - protein, 16 aa, Artificial Sequence
  CDR2 of VHH sequence 51C06
AITTGGNTNYADSVKG

SEQ ID NO: 182 - protein, 16 aa, Artificial Sequence
  CDR2 of VHH sequence 51C08
TISNGGSTNYADSVKG

SEQ ID NO: 183 - protein, 15 aa, Artificial Sequence
  CDR2 of VHH sequence 52A01
SISTGSTNYADSVKG

SEQ ID NO: 184 - protein, 16 aa, Artificial Sequence
  CDR2 of VHH sequence 52B01
TISRGGSTNYADSVKG

SEQ ID NO: 185 - protein, 16 aa, Artificial Sequence
  CDR2 of VHH sequence 52G05
SITRRGSTNYADSVKD

SEQ ID NO: 186 - protein, 16 aa, Artificial Sequence
  CDR2 of VHH sequence 53A01
SISSGGWTNYADSVKG

SEQ ID NO: 187 - protein, 16 aa, Artificial Sequence
  CDR2 of VHH sequence 53F05
SITTGGSTNYAEPVKG

SEQ ID NO: 188 - protein, 17 aa, Artificial Sequence
  CDR2 of VHH sequence 54A02
ANRWSGGSTYYADSVRG

SEQ ID NO: 189 - protein, 17 aa, Artificial Sequence
  CDR2 of VHH sequence 54B01
GITWTGGSTDYADSVKG

SEQ ID NO: 190 - protein, 17 aa, Artificial Sequence
  CDR2 of VHH sequence 54C01
AISWSGGSTYYADSVKD

SEQ ID NO: 191 - protein, 16 aa, Artificial Sequence
  CDR2 of VHH sequence 54C04
DMTSGGSINYADSVSG

SEQ ID NO: 192 - protein, 16 aa, Artificial Sequence
  CDR2 of VHH sequence 54C08
SITSGGSTNYADSVKG

SEQ ID NO: 193 - protein, 16 aa, Artificial Sequence
  CDR2 of VHH sequence 54C10
QITRRGSTNYADSVKG

SEQ ID NO: 194 - protein, 16 aa, Artificial Sequence
  CDR2 of VHH sequence 54C11
NITRGGSTNYADSVKG

SEQ ID NO: 195 - protein, 16 aa, Artificial Sequence
  CDR2 of VHH sequence 54D03
SISSGGNTNYSESVKG

SEQ ID NO: 196 - protein, 16 aa, Artificial Sequence
  CDR2 of VHH sequence 54D06
TITRGGITNYADSVKG

SEQ ID NO: 197 - protein, 16 aa, Artificial Sequence
  CDR2 of VHH sequence 54D10
ITSTSGTTDYTDSVKG

SEQ ID NO: 198 - protein, 16 aa, Artificial Sequence
  CDR2 of VHH sequence 54E01
AITSGGSTNYADYVKG

SEQ ID NO: 199 - protein, 16 aa, Artificial Sequence
  CDR2 of VHH sequence 54E05
AITNRGSTNYADFVKG

SEQ ID NO: 200 - protein, 16 aa, Artificial Sequence
  CDR2 of VHH sequence 54E10
AITRGGSTNYADSVKG

SEQ ID NO: 201 - protein, 16 aa, Artificial Sequence
  CDR2 of VHH sequence 54F01
TITRGGSTNYADSVKG

SEQ ID NO: 202 - protein, 16 aa, Artificial Sequence
  CDR2 of VHH sequence 54F02
TITSGGTTNYADSVKN

SEQ ID NO: 203 - protein, 16 aa, Artificial Sequence
  CDR2 of VHH sequence 54G01
IISSNSTSNYADSVKG

SEQ ID NO: 204 - protein, 16 aa, Artificial Sequence
  CDR2 of VHH sequence 54G08
AITSSSNTNYADSVKG

SEQ ID NO: 205 - protein, 16 aa, Artificial Sequence
  CDR2 of VHH sequence 54G09
TITSDQSTNYADSVKG

SEQ ID NO: 206 - protein, 16 aa, Artificial Sequence
  CDR2 of VHH sequence 55B02
DMRSDGSTNYADSVKG

SEQ ID NO: 207 - protein, 17 aa, Artificial Sequence
  CDR2 of VHH sequence 55B05
RISWSGIMAYYAESVKG

SEQ ID NO: 208 - protein, 16 aa, Artificial Sequence
  CDR2 of VHH sequence 55C05
QITRGDSTNYADSVKG

SEQ ID NO: 209 - protein, 16 aa, Artificial Sequence
  CDR2 of VHH sequence 55D08
TITSAGSSNYSDSVKG

SEQ ID NO: 210 - protein, 16 aa, Artificial Sequence
  CDR2 of VHH sequence 55E02
RILSGGSTNYADSVKG

SEQ ID NO: 211 - protein, 16 aa, Artificial Sequence
  CDR2 of VHH sequence 55E07
RITSGGSTYYADSVKG

SEQ ID NO: 212 - protein, 17 aa, Artificial Sequence
  CDR2 of VHH sequence 55E09
AIIWSGGRTRYADSVKG

SEQ ID NO: 213 - protein, 16 aa, Artificial Sequence
  CDR2 of VHH sequence 55E10
TISSGGSTNYADSVKG

SEQ ID NO: 214 - protein, 16 aa, Artificial Sequence
  CDR2 of VHH sequence 55F04
TITSDGSTNYADSVKG

SEQ ID NO: 215 - protein, 17 aa, Artificial Sequence
  CDR2 of VHH sequence 55F09
AITPGGGNTTYADSVKG

SEQ ID NO: 216 - protein, 17 aa, Artificial Sequence
  CDR2 of VHH sequence 55F10
TIRRSGSSTYYLDSTKG

SEQ ID NO: 217 - protein, 16 aa, Artificial Sequence
  CDR2 of VHH sequence 55G02
FITSGGITNYTDSVKG

SEQ ID NO: 218 - protein, 16 aa, Artificial Sequence
  CDR2 of VHH sequence 55G08
SISSGGTTDYVESVKG

SEQ ID NO: 219 - protein, 16 aa, Artificial Sequence
  CDR2 of VHH sequence 56A05
SISSGGSTNYADSVKG

SEQ ID NO: 220 - protein, 16 aa, Artificial Sequence
  CDR2 of VHH sequence 56A06
RITNIGTTNYADSVKG

SEQ ID NO: 221 - protein, 16 aa, Artificial Sequence
  CDR2 of VHH sequence 56A09
TITRGGTTNYADSVKG

SEQ ID NO: 222 - protein, 16 aa, Artificial Sequence
  CDR2 of VHH sequence 56C09
NITSVGSTNYADSVKG

SEQ ID NO: 223 - protein, 16 aa, Artificial Sequence
  CDR2 of VHH sequence 56C12
SISGIRITTYTNSVKG

SEQ ID NO: 224 - protein, 16 aa, Artificial Sequence
  CDR2 of VHH sequence 56D07
VITSGGRTNYAESVKG

SEQ ID NO: 225 - protein, 16 aa, Artificial Sequence
  CDR2 of VHH sequence 56D07
VITSGGRTNYAESVKG

SEQ ID NO: 226 - protein, 16 aa, Artificial Sequence
  CDR2 of VHH sequence 56D10
SSSSGGTTNYASSVKG

SEQ ID NO: 227 - protein, 16 aa, Artificial Sequence
  CDR2 of VHH sequence 56E04
KITTGGTTNYADSVKG

SEQ ID NO: 228 - protein, 16 aa, Artificial Sequence
  CDR2 of VHH sequence 56E05
RISSGGNTNYTDSVKG

SEQ ID NO: 229 - protein, 16 aa, Artificial Sequence
  CDR2 of VHH sequence 56E08
TITSANITNYADSVKG

SEQ ID NO: 230 - protein, 16 aa, Artificial Sequence
  CDR2 of VHH sequence 56F07
IITNDDSTTYADSVKG

SEQ ID NO: 231 - protein, 16 aa, Artificial Sequence
  CDR2 of VHH sequence 56G07
TITPFGRRNYSEYVKG

SEQ ID NO: 232 - protein, 16 aa, Artificial Sequence
  CDR2 of VHH sequence 56G08
TLSRAGTSRYVDSVKG

SEQ ID NO: 233 - protein, 16 aa, Artificial Sequence
  CDR2 of VHH sequence 56G10
EISSRGTTMYADSVKG

SEQ ID NO: 234 - protein, 16 aa, Artificial Sequence
  CDR2 of VHH sequence 56H04
RISTVGTAHYADSVKG

SEQ ID NO: 235 - protein, 16 aa, Artificial Sequence
  CDR2 of VHH sequence 56H05
QINNRDNTEYADSVKG

SEQ ID NO: 236 - protein, 15 aa, Artificial Sequence
  CDR2 of VHH sequence 56H07
SISTGSTNYADSVKG

SEQ ID NO: 237 - protein, 16 aa, Artificial Sequence
  CDR2 of VHH sequence 56H08
VISSDGSTNYADSVKG

SEQ ID NO: 238 - protein, 16 aa, Artificial Sequence
  CDR2 of VHH sequence 57A06
RISSGGNTNYTDSVKG

SEQ ID NO: 239 - protein, 16 aa, Artificial Sequence
  CDR2 of VHH sequence 57B01
RISSGGSTNYADSVKG

SEQ ID NO: 240 - protein, 16 aa, Artificial Sequence
  CDR2 of VHH sequence 57B07
TVDSGGYTNYADSVKG

SEQ ID NO: 241 - protein, 16 aa, Artificial Sequence
  CDR2 of VHH sequence 57B11
LIRSSGGTYYADSVKG

SEQ ID NO: 242 - protein, 16 aa, Artificial Sequence
  CDR2 of VHH sequence 57C07
SISRGGMTNYADSVKG

SEQ ID NO: 243 - protein, 16 aa, Artificial Sequence
  CDR2 of VHH sequence 57C09
SISSGGATNYADSVKG

SEQ ID NO: 244 - protein, 16 aa, Artificial Sequence
  CDR2 of VHH sequence 57D02
TITRRSRTNYAEFVKG

SEQ ID NO: 245 - protein, 16 aa, Artificial Sequence
  CDR2 of VHH sequence 57D09
SITTGGSTNYADSVKG

SEQ ID NO: 246 - protein, 16 aa, Artificial Sequence
  CDR2 of VHH sequence 57D10
SITKDGTTNYADSVKG

SEQ ID NO: 247 - protein, 16 aa, Artificial Sequence
  CDR2 of VHH sequence 57E07
DITRSGSTHYVDSVKG

SEQ ID NO: 248 - protein, 16 aa, Artificial Sequence
  CDR2 of VHH sequence 57E11
RISRLRVTNYADSVKG

SEQ ID NO: 249 - protein, 16 aa, Artificial Sequence
  CDR2 of VHH sequence 57G01
TISNSGTTNYVDAVKG

SEQ ID NO: 250 - protein, 16 aa, Artificial Sequence
  CDR2 of VHH sequence 57G07
TIRRGGNTKYADSVKG

SEQ ID NO: 251 - protein, 16 aa, Artificial Sequence
  CDR2 of VHH sequence 57G08
TIDIHNSTKYADSVKG

SEQ ID NO: 252 - protein, 16 aa, Artificial Sequence
  CDR2 of VHH sequence 57H08
QQRYDGSTNYADSLQG

SEQ ID NO: 253 - protein, 7 aa, Artificial Sequence
  CDR3 of VHH sequence 41D01
RSIWRDY

SEQ ID NO: 254 - protein, 11 aa, Artificial Sequence
  CDR3 of VHH sequence 56F07
DINTAIWRRKY

SEQ ID NO: 255 - protein, 10 aa, Artificial Sequence
  CDR3 of VHH sequence 40F07
ARTWSIFRNY

SEQ ID NO: 256 - protein, 8 aa, Artificial Sequence
  CDR3 of VHH sequence 41D06
VRLWFPDY

SEQ ID NO: 257 - protein, 13 aa, Artificial Sequence
  CDR3 of VHH sequence 41G10
EARRYFTRASQVY

SEQ ID NO: 258 - protein, 12 aa, Artificial Sequence
  CDR3 of VHH sequence 41H05
VGRRWYGGYVEL

SEQ ID NO: 259 - protein, 11 aa, Artificial Sequence
  CDR3 of VHH sequence 42C11
DRWVLTRWSNY

SEQ ID NO: 260 - protein, 11 aa, Artificial Sequence
  CDR3 of VHH sequence 42C12
QRGVAWTRKEY

SEQ ID NO: 261 - protein, 11 aa, CDR3 of VHH sequence 50D03
DRWVLTRWSNY

SEQ ID NO: 262 - protein, 12 aa, Artificial Sequence
  CDR3 of VHH sequence 50D07
RVRTVLRGWRDY

SEQ ID NO: 263 - protein, 11 aa, Artificial Sequence
  CDR3 of VHH sequence 50E02
RRRTFLKSSDY

SEQ ID NO: 264 - protein, 15 aa, Artificial Sequence
  CDR3 of VHH sequence 51B08
KYGRWTYTGRPEYDS

SEQ ID NO: 265 - protein, 8 aa, Artificial Sequence
  CDR3 of VHH sequence 51C06
RRRWSRDF

SEQ ID NO: 266 - protein, 11 aa, Artificial Sequence
  CDR3 of VHH sequence 51C08
RQQFIGAPYEY

SEQ ID NO: 267 - protein, 7 aa, Artificial Sequence
  CDR3 of VHH sequence 52A01
RLLWSNY

SEQ ID NO: 268 - protein, 9 aa, Artificial Sequence
  CDR3 of VHH sequence 52B01
AGWVGVTNY

SEQ ID NO: 269 - protein, 9 aa, Artificial Sequence
  CDR3 of VHH sequence 52G05
RRYYTRNDY

SEQ ID NO: 270 - protein, 6 aa, Artificial Sequence
  CDR3 of VHH sequence 53A01
GAIGNW

SEQ ID NO: 271 - protein, 9 aa, Artificial Sequence
  CDR3 of VHH sequence 53F05
ERRWGLPNY

SEQ ID NO: 272 - protein, 17 aa, Artificial Sequence
  CDR3 of VHH sequence 54A02
YAHITAWGMRNDYEYDY

SEQ ID NO: 273 - protein, 16 aa, Artificial Sequence
  CDR3 of VHH sequence 54B01
GNLLRLAGQLRRGYDS

SEQ ID NO: 274 - protein, 20 aa, Artificial Sequence
  CDR3 of VHH sequence 54C01
RNRAGPHYSRGYTAGQEYDY

SEQ ID NO: 275 - protein, 13 aa, Artificial Sequence
  CDR3 of VHH sequence 54C04
NLRTAFWRNGNDY

SEQ ID NO: 276 - protein, 7 aa, Artificial Sequence
  CDR3 of VHH sequence 54C08
GPWYRRS

SEQ ID NO: 277 - protein, 8 aa, Artificial Sequence
  CDR3 of VHH sequence 54C10
DLAVRGRY

SEQ ID NO: 278 - protein, 11 aa, Artificial Sequence
  CDR3 of VHH sequence 54C11
RIGFGWTAKAY

SEQ ID NO: 279 - protein, 8 aa, Artificial Sequence
  CDR3 of VHH sequence 54D03
VRLWFPDY

SEQ ID NO: 280 - protein, 8 aa, Artificial Sequence
  CDR3 of VHH sequence 54D06
RSWVGPEY

SEQ ID NO: 281 - protein, 12 aa, Artificial Sequence
  CDR3 of VHH sequence 54D10
KTRTWYNGKYDY

SEQ ID NO: 282 - protein, 9 aa, Artificial Sequence
  CDR3 of VHH sequence 54E01
RSTLWRRDY

SEQ ID NO: 283 - protein, 9 aa, Artificial Sequence
  CDR3 of VHH sequence 54E05
HRSWPRYDS

SEQ ID NO: 284 - protein, 10 aa, Artificial Sequence
  CDR3 of VHH sequence 54E10
ESRIFRRYDY

SEQ ID NO: 285 - protein, 7 aa, Artificial Sequence
  CDR3 of VHH sequence 54F01
DRGWSSY

SEQ ID NO: 286 - protein, 11 aa, Artificial Sequence
  CDR3 of VHH sequence 54F02
HQRAWARSYVY

SEQ ID NO: 287 - protein, 9 aa, Artificial Sequence
  CDR3 of VHH sequence 54G01
KRSWFSQEY

SEQ ID NO: 288 - protein, 13 aa, Artificial Sequence
  CDR3 of VHH sequence 54G08
QYTITPWGIKKDY

SEQ ID NO: 289 - protein, 12 aa, Artificial Sequence
  CDR3 of VHH sequence 54G09
RVRTVLRGWRDY

SEQ ID NO: 290 - protein, 9 aa, Artificial Sequence
  CDR3 of VHH sequence 55B02
NSIFRSRDY

SEQ ID NO: 291 - protein, 16 aa, Artificial Sequence
  CDR3 of VHH sequence 55B05
RSQIRSPWSSLDDYDR

SEQ ID NO: 292 - protein, 8 aa, Artificial Sequence
  CDR3 of VHH sequence 55C05
DRFFGRDY

SEQ ID NO: 293 - protein, 12 aa, Artificial Sequence
  CDR3 of VHH sequence 55D08
VYSRPLLGPLEV

SEQ ID NO: 294 - protein, 7 aa, Artificial Sequence
  CDR3 of VHH sequence 55E02
VRYLVNY

SEQ ID NO: 295 - protein, 13 aa, Artificial Sequence
  CDR3 of VHH sequence 55E07
GVVVATSPKFYAY

SEQ ID NO: 296 - protein, 7 aa, Artificial Sequence
  CDR3 of VHH sequence 55E09
RRLGTGY

SEQ ID NO: 297 - protein, 7 aa, Artificial Sequence
  CDR3 of VHH sequence 55E10
RYWFRDY

SEQ ID NO: 298 - protein, 7 aa, Artificial Sequence
  CDR3 of VHH sequence 55F04
VRLFRQY

SEQ ID NO: 299 - protein, 16 aa, Artificial Sequence
  CDR3 of VHH sequence 55F09
GGSSRWYSSRYYPGGY

SEQ ID NO: 300 - protein, 17 aa, Artificial Sequence
  CDR3 of VHH sequence 55F10
DSSARALVGGPGNRWDY

SEQ ID NO: 301 - protein, 10 aa, Artificial Sequence
  CDR3 of VHH sequence 55G02
KNAKNVRPGY

SEQ ID NO: 302 - protein, 8 aa, Artificial Sequence
  CDR3 of VHH sequence 55G08
VRFWFPDY

SEQ ID NO: 303 - protein, 8 aa, Artificial Sequence
  CDR3 of VHH sequence 56A05
RRNVFISS

SEQ ID NO: 304 - protein, 7 aa, Artificial Sequence
  CDR3 of VHH sequence 56A06
RRLGRDY

SEQ ID NO: 305 - protein, 10 aa, Artificial Sequence
  CDR3 of VHH sequence 56A09
NFGILVGREY

SEQ ID NO: 306 - protein, 8 aa, Artificial Sequence
  CDR3 of VHH sequence 56C09
RMPFLGDS

SEQ ID NO: 307 - protein, 8 aa, Artificial Sequence
  CDR3 of VHH sequence 56D06
TSITGTYL

SEQ ID NO: 308 - protein, 6 aa, Artificial Sequence
  CDR3 of VHH sequence 56D07
KTIRPY

SEQ ID NO: 309 - protein, 12 aa, Artificial Sequence
  CDR3 of VHH sequence 56D10
RKFITTPWSTDY

SEQ ID NO: 310 - protein, 8 aa, Artificial Sequence
  CDR3 of VHH sequence 56E04
ERYFATTL

SEQ ID NO: 311 - protein, 11 aa, Artificial Sequence
  CDR3 of VHH sequence 56E05
QRRVILGPRNY

SEQ ID NO: 312 - protein, 13 aa, Artificial Sequence
  CDR3 of VHH sequence 56E08
QAKKWRIGPWSDY

SEQ ID NO: 313 - protein, 13 aa, Artificial Sequence
  CDR3 of VHH sequence 56F11
NTRRIFGGTVREY

SEQ ID NO: 314 - protein, 7 aa, Artificial Sequence
  CDR3 of VHH sequence 56G07
RVNGVDY

SEQ ID NO: 315 - protein, 7 aa, Artificial Sequence
  CDR3 of VHH sequence 56G08
AQLGTDY

SEQ ID NO: 316 - protein, 9 aa, Artificial Sequence
  CDR3 of VHH sequence 56G10
RAFAFGRNS

SEQ ID NO: 317 - protein, 10 aa, Artificial Sequence
  CDR3 of VHH sequence 56H04
QAGRLYLRNY

SEQ ID NO: 318 - protein, 9 aa, Artificial Sequence
  CDR3 of VHH sequence 56H05
KRWSWSTGF

SEQ ID NO: 319 - protein, 7 aa, Artificial Sequence
  CDR3 of VHH sequence 56H07
RLWWSNY

SEQ ID NO: 320 - protein, 10 aa, Artificial Sequence
  CDR3 of VHH sequence 56H08
NRRWSWGSEY

SEQ ID NO: 321 - protein, 11 aa, Artificial Sequence
  CDR3 of VHH sequence 57A06
QRRVILGPRNY

SEQ ID NO: 322 - protein, 8 aa, Artificial Sequence
  CDR3 of VHH sequence 57B01
NRHWGWDY

SEQ ID NO: 323 - protein, 14 aa, Artificial Sequence
  CDR3 of VHH sequence 57B07
GIYKWPWSVDARDY

SEQ ID NO: 324 - protein, 9 aa, Artificial Sequence
  CDR3 of VHH sequence 57B11
RRTWLSSES

SEQ ID NO: 325 - protein, 14 aa, Artificial Sequence
  CDR3 of VHH sequence 57C07
GIRSRWYGGPITTY

SEQ ID NO: 326 - protein, 13 aa, Artificial Sequence
  CDR3 of VHH sequence 57C09
KKSRWSWSIVHDY

SEQ ID NO: 327 - protein, 10 aa, Artificial Sequence
  CDR3 of VHH sequence 57D02
RWGAGGIFST

SEQ ID NO: 328 - protein, 13 aa, Artificial Sequence
  CDR3 of VHH sequence 57D09
KVRLRWFRPPSDY

SEQ ID NO: 329 - protein, 14 aa, Artificial Sequence
  CDR3 of VHH sequence 57D10
RATTWVPYRRDAEF

SEQ ID NO: 330 - protein, 12 aa, Artificial Sequence
  CDR3 of VHH sequence 57E07
DSGSHWWNRRDY

SEQ ID NO: 331 - protein, 10 aa, Artificial Sequence
  CDR3 of VHH sequence 57E11
ANWGLAGNEY

SEQ ID NO: 332 - protein, 8 aa, Artificial Sequence
  CDR3 of VHH sequence 57G01
QTFWRRNY

SEQ ID NO: 333 - protein, 8 aa, Artificial Sequence
  CDR3 of VHH sequence 57G07
HSWLDYDY

SEQ ID NO: 334 - protein, 7 aa, Artificial Sequence
  CDR3 of VHH sequence 57G08
IPTFGRY

SEQ ID NO: 335 - protein, 7 aa, Artificial Sequence
  CDR3 of VHH sequence 57H08
NRGFISY

SEQ ID NO: 336 - DNA, 345 bp, Artificial Sequence
  VHH 41D01
caggttcagctgcaggaatctggtggtggacttgttcaagctggtggatctcttagactctcttgcgctgcttctggaaggaccttctctagatatggaatgggatggttcaggcagctccctggaaaacagagagagcttgttacctctatcaccaggggtggaactaccacctacgctgattctgtgaagggaaggttcaccatctctagggataacgctaagaacaccgtgtacctccagatgaactctctcaagcctgaggataccgctgtgtactactgcaacgctagatctatttggagggattactggggacagggaactcaggtcaccgtttcttca

SEQ ID NO: 337 - DNA, 363 bp, Artificial Sequence
  VHH 56F11
caggttcagctgcaggaatctggtggtggacttgttcagtctggtggatctctcagactctcttgcgtgcactctaagaccaccttcaccagaaatgctatgggatggtacagacaggctctcggaaaagagagagagcttgttgctaccatcacctctggtggaactaccaactacgctgattctgtgaagggaaggttcaccatctctatggattctgctaagaacaccgtgtacctccagatgaactctctcaagcctgaggataccgctgtgtactactgcaacgtgaacaccagaaggatcttcggaggaaccgttagagaatactggggacaaggtactcaggtcaccgtttcttca

SEQ ID NO: 338 - DNA, 456 bp, Artificial Sequence
  41D01_His_KDEL
atggcaaacaagcttttcttggtgtgcgctaccttcgctctttgcttccttttgactaacgctcaggttcagctgcaggaatctggtggtggacttgttcaagctggtggatctcttagactctcttgcgctgcttctggaaggaccttctctagatatggaatgggatggttcaggcagctccctggaaaacagagagagcttgttacctctatcaccaggggtggaactaccacctacgctgattctgtgaagggaaggttcaccatctctagggataacgctaagaacaccgtgtacctccagatgaactctctcaagcctgaggataccgctgtgtactactgcaacgctagatctatttggagggattactggggacagggaactcaggtcaccgtttcttcagcggccgcacatcatcatcaccatcatggtgctgctaaggatgagctt

SEQ ID NO: 339 - DNA, 1131 bp, Artificial Sequence
  sec_41D01_hinge_Fc_His
atggcaaacaagcttttcttggtgtgcgctaccttcgctctttgcttccttttgactaacgctcaggttcagctgcaggaatctggtggtggacttgttcaagctggtggatctcttagactctcttgcgctgcttctggaaggaccttctctagatatggaatgggatggttcaggcagctccctggaaaacagagagagcttgttacctctatcaccaggggtggaactaccacctacgctgattctgtgaagggaaggttcaccatctctagggataacgctaagaacaccgtgtacctccagatgaactctctcaagcctgaggataccgctgtgtactactgcaacgctagatctatttggagggattactggggacagggaactcaggtcaccgtttcttcacctagaatccctaagccttctacccctcctggatcttcttgtcctcctggaaatatcctcggtggaccttctgtgttcatcttcccacctaagcctaaggatgctctcatgatctcactcacccctaaggttacatgcgttgtggtggatgtgtctgaggatgatcctgatgtgcacgtgtcatggttcgtggataacaaagaggtgcacactgcttggactcagcctagagaagctcagtacaactctaccttcagggtggtgtctgctctccctatccaacaccaagattggatgaggggtaaagagttcaagtgcaaggtgaacaacaaggctctccctgctcctatcgagaggactatctctaaacctaagggaagggctcagacccctcaagtgtatacaattcctccacctagggaacagatgtctaagaagaaggtttcactcacttgcctcgtgaccaacttcttcagtgaggctatctctgttgagtgggagaggaatggtgagcttgagcaggattacaagaacacccctcctatcctcgattctgatggaacctacttcctctactctaagctcaccgtggataccgattcttggttgcagggtgagatcttcacttgctctgttgtgcatgaggctctccacaaccatcacacccagaagaacctcagtagatctcctggtaaagcggccgcacatcatcatcaccatcat

SEQ ID NO: 340 - DNA, 807 bp, Artificial Sequence
  sec_41D01-9GS-41D01_His
atggcaaacaagcttttcttggtgtgcgctaccttcgctctttgcttccttttgactaacgctcaggttcaattgcaagagtctggtggtggacttgttcaggctggtggatctcttagactttcttgcgctgcttctggaaggaccttctctagatatggaatgggatggttcaggcagctccctggaaaacagagagagcttgttacctctatcaccaggggtggaactaccacctacgctgattctgtgaagggaaggttcaccatctctagggataacgctaagaacaccgtgtacctccagatgaactctctcaagcctgaggataccgctgtgtactactgcaacgctagatctatttggagggattactggggacagggaactcaggtcaccgtttcttcaggtggtggtggaagtggtggtggttctcaagttcaactgcaggaatcaggtggtggattggtgcaagctggtggttctttgaggttgtcatgtgctgctagtggtaggaccttcagtaggtacggtatgggatggtttagacagttgcctggtaagcagagggaactcgtgacttcaatcactagaggtggaaccactacttacgcagatagtgttaagggaagattcactatcagtagagataatgcaaagaacactgtttacttgcaaatgaactcattgaagccagaggatacagcagtttattactgtaacgcaagaagtatttggagagattattggggtcaaggtactcaagtgaccgttagttcagcggccgcacatcatcatcaccatcat

SEQ ID NO: 341 - DNA, 435 bp, Artificial Seqeunce
  sec_41D01_His
atggcaaacaagcttttcttggtgtgcgctaccttcgctctttgcttccttttgactaacgctcaggttcagctgcaggaatctggtggtggacttgttcaagctggtggatctcttagactctcttgcgctgcttctggaaggaccttctctagatatggaatgggatggttcaggcagctccctggaaaacagagagagcttgttacctctatcaccaggggtggaactaccacctacgctgattctgtgaagggaaggttcaccatctctagggataacgctaagaacaccgtgtacctccagatgaactctctcaagcctgaggataccgctgtgtactactgcaacgctagatctatttggagggattactggggacagggaactcaggtcaccgtttcttcagcggccgcacatcatcatcaccatcat

SEQ ID NO: 342 - DNA, 375 bp, Artificial Sequence
  cyto_41D01_His
atgcaggttcagctgcaggaatctggtggtggacttgttcaagctggtggatctcttagactctcttgcgctgcttctggaaggaccttctctagatatggaatgggatggttcaggcagctccctggaaaacagagagagcttgttacctctatcaccaggggtggaactaccacctacgctgattctgtgaagggaaggttcaccatctctagggataacgctaagaacaccgtgtacctccagatgaactctctcaagcctgaggataccgctgtgtactactgcaacgctagatctatttggagggattactggggacagggaactcaggtcaccgtttcttcagcggccgcacatcatcatcaccatcat

SEQ ID NO: 343 - DNA, 474 bp, Artificial Sequence
  56F11_His_KDEL
atggcaaacaagcttttcttggtgtgcgctaccttcgctctttgcttccttttgactaacgctcaggttcagctgcaggaatctggtggtggacttgttcagtctggtggatctctcagactctcttgcgtgcactctaagaccaccttcaccagaaatgctatgggatggtacagacaggctctcggaaaagagagagagcttgttgctaccatcacctctggtggaactaccaactacgctgattctgtgaagggaaggttcaccatctctatggattctgctaagaacaccgtgtacctccagatgaactctctcaagcctgaggataccgctgtgtactactgcaacgtgaacaccagaaggatcttcggaggaaccgttagagaatactggggacaaggtactcaggtcaccgtttcttcagcggccgcacatcatcatcaccatcatggtgctgctaaggatgagctt

SEQ ID NO: 344 - DNA, 1149 bp, Artificial Sequence
  sec_56F11_hinge_Fc_His
atggcaaacaagcttttcttggtgtgcgctaccttcgctctttgcttccttttgactaacgctcaggttcagctgcaggaatctggtggtggacttgttcagtctggtggatctctcagactctcttgcgtgcactctaagaccaccttcaccagaaatgctatgggatggtacagacaggctctcggaaaagagagagagcttgttgctaccatcacctctggtggaactaccaactacgctgattctgtgaagggaaggttcaccatctctatggattctgctaagaacaccgtgtacctccagatgaactctctcaagcctgaggataccgctgtgtactactgcaacgtgaacaccagaaggatcttcggaggaaccgttagagaatactggggacaaggtactcaggtcaccgtttcttcacctagaatccctaagccttctacccctcctggatcttcttgtcctcctggaaatatcctcggaggaccttcagtgttcatcttcccacctaagcctaaggatgctctcatgatctcactcacccctaaggttacatgcgttgtggtggatgtgtctgaggatgatcctgatgtgcacgtgtcatggttcgtggataacaaagaggtgcacactgcttggactcagcctagagaagctcagtacaactctaccttcagggtggtgtctgctctccctatccaacaccaagattggatgaggggtaaagagttcaagtgcaaggtgaacaacaaggctctccctgctcctatcgagaggactatctctaaacctaagggaagggctcagacccctcaagtgtatacaattcctccacctagggaacagatgtctaagaagaaggtttcactcacttgcctcgtgaccaacttcttcagtgaggctatctctgttgagtgggagaggaatggtgagcttgagcaggattacaagaacacccctcctatcctcgattctgatggaacctacttcctctactctaagctcaccgtggataccgattcttggttgcagggtgagatcttcacttgctctgttgtgcatgaggctctccacaaccatcacacccagaagaacctcagtagatctcctggtaaagcggccgcacatcatcatcaccatcat

SEQ ID NO: 345 - DNA, 843 bp, Artificial Sequence
  sec_56F11-9GS-56F11_His
atggcaaacaagcttttcttggtgtgcgctaccttcgctctttgcttccttttgactaacgctcaggttcaattgcaagagtctggtggtggactcgtgcaatctggtggatctcttagactctcttgcgtgcactctaagaccaccttcaccagaaatgctatgggatggtacagacaggctctcggaaaagagagagagcttgttgctaccatcacctctggtggaactaccaactacgctgattctgtgaagggaaggttcaccatctctatggattctgctaagaacaccgtgtacctccagatgaactctctcaagcctgaggataccgctgtgtactactgcaacgtgaacaccagaaggatcttcggaggaaccgttagagaatactggggacaaggtactcaggtcaccgtttcttcaggtggtggtggaagtggtggtggttctcaagttcaactgcaggaatcaggtggtggattggttcagtctggtggttctctcaggttgtcatgcgttcacagtaagactactttcactaggaacgcaatgggatggtataggcaagcacttggtaaagagagggaactcgttgcaactatcacaagtggtggaaccactaattacgcagatagtgttaagggaagattcactattagtatggatagtgcaaagaacactgtttacttgcaaatgaactcattgaagccagaggatacagcagtttattactgtaatgttaacactagaagaattttcggtggtactgtgagagagtattggggacagggaacccaggttacagttagttcagcggccgcacatcatcaccatcaccat

SEQ ID NO: 346 - DNA, 453 bp, Artificial Sequence
  sec_56F11_His
atggcaaacaagcttttcttggtgtgcgctaccttcgctctttgcttccttttgactaacgctcaggttcagctgcaggaatctggtggtggacttgttcagtctggtggatctctcagactctcttgcgtgcactctaagaccaccttcaccagaaatgctatgggatggtacagacaggctctcggaaaagagagagagcttgttgctaccatcacctctggtggaactaccaactacgctgattctgtgaagggaaggttcaccatctctatggattctgctaagaacaccgtgtacctccagatgaactctctcaagcctgaggataccgctgtgtactactgcaacgtgaacaccagaaggatcttcggaggaaccgttagagaatactggggacaaggtactcaggtcaccgtttcttcagcggccgcacatcatcatcaccatcat

SEQ ID NO: 347 - DNA, 393 bp, Artificial Sequence
  cyto_56F11_His
atgcaggttcagctgcaggaatctggtggtggacttgttcagtctggtggatctctcagactctcttgcgtgcactctaagaccaccttcaccagaaatgctatgggatggtacagacaggctctcggaaaagagagagagcttgttgctaccatcacctctggtggaactaccaactacgctgattctgtgaagggaaggttcaccatctctatggattctgctaagaacaccgtgtacctccagatgaactctctcaagcctgaggataccgctgtgtactactgcaacgtgaacaccagaaggatcttcggaggaaccgttagagaatactggggacaaggtactcaggtcaccgtttcttcagcggccgcacatcatcatcaccatcat

SEQ ID NO: 348 - protein, 6 aa, Artificial Sequence
  His
HHHHHH

SEQ ID NO: 349 - protein, 4 aa, Artificial Sequence
  ER retention signal
KDEL

SEQ ID NO: 350 - protein, 21 aa, Artificial Sequence
  2S2 secretion signal
MANKLFLVCATFALCFLLTNA

SEQ ID NO: 351 - protein, 217 aa, Artificial Sequence
  Fc region
PGNILGGPSVFIFPPKPKDALMISLTPKVTCVVVDVSEDDPDVHVSWFVDNKEVHTAWTQPREAQYNSTFRVVSALPIQHQDWMRGKEFKCKVNNKALPAPIERTISKPKGRAQTPQVYTIPPPREQMSKKKVSLTCLVTNFFSEAISVEWERNGELEQDYKNTPPILDSDGTYFLYSKLTVDTDSWLQGEIFTCSVVHEALHNHHTQKNLSRSPGK

SEQ ID NO: 352 - protein, 9 aa, Artificial Sequence
  9GS spacer
GGGGSGGGS

SEQ ID NO: 353 - protein, 15 aa, Artificial Sequence
  hinge
PRIPKPSTPPGSSCP

SEQ ID NO: 354 - DNA, 1027 bp, Artificial Sequence
  CaMV 35S promoter
actagagccaagctgatctcctttgccccggagatcaccatggacgactttctctatctctacgatctaggaagaaagttcgacggagaaggtgacgataccatgttcaccaccgataatgagaagattagcctcttcaatttcagaaagaatgctgacccacagatggttagagaggcctacgcggcaggtctcatcaagacgatctacccgagtaataatctccaggagatcaaataccttcccaagaaggttaaagatgcagtcaaaagattcaggactaactgcatcaagaacacagagaaagatatatttctcaagatcagaagtactattccagtatggacgattcaaggcttgcttcataaaccaaggcaagtaatagagattggagtctctaagaaagtagttcctactgaatcaaaggccatggagtcaaaaattcagatcgaggatctaacagaactcgccgtgaagactggcgaacagttcatacagagtcttttacgactcaatgacaagaagaaaatcttcgtcaacatggtggagcacgacactctcgtctactccaagaatatcaaagatacagtctcagaagaccaaagggctattgagacttttcaacaaagggtaatatcgggaaacctcctcggattccattgcccagctatctgtcacttcatcaaaaggacagtagaaaaggaaggtggcacctacaaatgccatcattgcgataaaggaaaggctatcgttcaagatgcctctgccgacagtggtcccaaagatggacccccacccacgaggagcatcgtggaaaaagaagacgttccaaccacgtcttcaaagcaagtggattgatgtgatatctccactgacgtaagggatgacgcacaatcccactatccttcgcaagacccttcctctatataaggaagttcatttcatttggagaggactccggtatttttacaacaataccacaacaaaacaaacaacaaacaacattacaatttactattctagtcga

SEQ ID NO: 355 - DNA, 18 bp, Artificial Sequence
  pMA_FW primer
ttgtaaaacgacggccag

SEQ ID NO: 356 - DNA, 20 bp, Artificial Sequence
  pMA_REV primer
ggaaacagctatgaccatgt

SEQ ID NO: 357 - DNA, 36 bp, Artificial Sequence
  pMA_CYTO primer
ccggaattcccaccatgcaggttcagctgcaggaat

SEQ ID NO: 358 - DNA, 11159 bp, Artificial Sequence
  pK7WG2
ggccctctagaggatccccgggtaccctcgaattatcatacatgagaattaagggagtcacgttatgacccccgccgatgacgcgggacaagccgttttacgtttggaactgacagaaccgcaacgttgaaggagccactcagccgcgggtttctggagtttaatgagctaagcacatacgtcagaaaccattattgcgcgttcaaaagtcgcctaaggtcactatcagctagcaaatatttcttgtcaaaaatgctccactgacgttccataaattcccctcggtatccaattagagtctcatattcactctcaactcgatcgaggcatgattgaacaagatggattgcacgcaggttctccggccgcttgggtggagaggctattcggctatgactgggcacaacagacaatcggctgctctgatgccgccgtgttccggctgtcagcgcaggggcgcccggttctttttgtcaagaccgacctgtccggtgccctgaatgaactccaagacgaggcagcgcggctatcgtggctggccacgacgggcgttccttgcgcagctgtgctcgacgttgtcactgaagcgggaagggactggctgctattgggcgaagtgccggggcaggatctcctgtcatctcaccttgctcctgccgagaaagtatccatcatggctgatgcaatgcggcggctgcatacgcttgatccggctacctgcccattcgaccaccaagcgaaacatcgcatcgagcgagcacgtactcggatggaagccggtcttgtcgatcaggatgatctggacgaagagcatcaggggctcgcgccagccgaactgttcgccaggctcaaggcgcggatgcccgacggcgaggatctcgtcgtgacccacggcgatgcctgcttgccgaatatcatggtggaaaatggccgcttttctggattcatcgactgtggccggctgggtgtggcggaccgctatcaggacatagcgttggctacccgtgatattgctgaagagcttggcggcgaatgggctgaccgcttcctcgtgctttacggtatcgccgctcccgattcgcagcgcatcgccttctatcgccttcttgacgagttcttctgagcgggactctggggttcggactctagctagagtcaagcagatcgttcaaacatttggcaataaagtttcttaagattgaatcctgttgccggtcttgcgatgattatcatataatttctgttgaattacgttaagcatgtaataattaacatgtaatgcatgacgttatttatgagatgggtttttatgattagagtcccgcaattatacatttaatacgcgatagaaaacaaaatatagcgcgcaaactaggataaattatcgcgcgcggtgtcatctatgttactagatcgaccggcatgcaagctgataattcaattcggcgttaattcagtacattaaaaacgtccgcaatgtgttattaagttgtctaagcgtcaatttgtttacaccacaatatatcctgccaccagccagccaacagctccccgaccggcagctcggcacaaaatcaccactcgatacaggcagcccatcagtccgggacggcgtcagcgggagagccgttgtaaggcggcagactttgctcatgttaccgatgctattcggaagaacggcaactaagctgccgggtttgaaacacggatgatctcgcggagggtagcatgttgattgtaacgatgacagagcgttgctgcctgtgatcaattcgggcacgaacccagtggacataagcctcgttcggttcgtaagctgtaatgcaagtagcgtaactgccgtcacgcaactggtccagaaccttgaccgaacgcagcggtggtaacggcgcagtggcggttttcatggcttcttgttatgacatgtttttttggggtacagtctatgcctcgggcatccaagcagcaagcgcgttacgccgtgggtcgatgtttgatgttatggagcagcaacgatgttacgcagcagggcagtcgccctaaaacaaagttaaacatcatgggggaagcggtgatcgccgaagtatcgactcaactatcagaggtagttggcgtcatcgagcgccatctcgaaccgacgttgctggccgtacatttgtacggctccgcagtggatggcggcctgaagccacacagtgatattgatttgctggttacggtgaccgtaaggcttgatgaaacaacgcggcgagctttgatcaacgaccttttggaaacttcggcttcccctggagagagcgagattctccgcgctgtagaagtcaccattgttgtgcacgacgacatcattccgtggcgttatccagctaagcgcgaactgcaatttggagaatggcagcgcaatgacattcttgcaggtatcttcgagccagccacgatcgacattgatctggctatcttgctgacaaaagcaagagaacatagcgttgccttggtaggtccagcggcggaggaactctttgatccggttcctgaacaggatctatttgaggcgctaaatgaaaccttaacgctatggaactcgccgcccgactgggctggcgatgagcgaaatgtagtgcttacgttgtcccgcatttggtacagcgcagtaaccggcaaaatcgcgccgaaggatgtcgctgccgactgggcaatggagcgcctgccggcccagtatcagcccgtcatacttgaagctagacaggcttatcttggacaagaagaagatcgcttggcctcgcgcgcagatcagttggaagaatttgtccactacgtgaaaggcgagatcaccaaggtagtcggcaaataatgtctagctagaaattcgttcaagccgacgccgcttcgccggcgttaactcaagcgattagatgcactaagcacataattgctcacagccaaactatcaggtcaagtctgcttttattatttttaagcgtgcataataagccctacacaaattgggagatatatcatgcatgaccaaaatcccttaacgtgagttttcgttccactgagcgtcagaccccgtagaaaagatcaaaggatcttcttgagatcctttttttctgcgcgtaatctgctgcttgcaaacaaaaaaaccaccgctaccagcggtggtttgtttgccggatcaagagctaccaactctttttccgaaggtaactggcttcagcagagcgcagataccaaatactgtccttctagtgtagccgtagttaggccaccacttcaagaactctgtagcaccgcctacatacctcgctctgctaatcctgttaccagtggctgctgccagtggcgataagtcgtgtcttaccgggttggactcaagacgatagttaccggataaggcgcagcggtcgggctgaacggggggttcgtgcacacagcccagcttggagcgaacgacctacaccgaactgagatacctacagcgtgagctatgagaaagcgccacgcttcccgaagggagaaaggcggacaggtatccggtaagcggcagggtcggaacaggagagcgcacgagggagcttccagggggaaacgcctggtatctttatagtcctgtcgggtttcgccacctctgacttgagcgtcgatttttgtgatgctcgtcaggggggcggagcctatggaaaaacgccagcaacgcggcctttttacggttcctggccttttgctggccttttgctcacatgttctttcctgcgttatcccctgattctgtggataaccgtattaccgcctttgagtgagctgataccgctcgccgcagccgaacgaccgagcgcagcgagtcagtgagcgaggaagcggaagagcgcctgatgcggtattttctccttacgcatctgtgcggtatttcacaccgcatatggtgcactctcagtacaatctgctctgatgccgcatagttaagccagtatacactccgctatcgctacgtgactgggtcatggctgcgccccgacacccgccaacacccgctgacgcgccctgacgggcttgtctgctcccggcatccgcttacagacaagctgtgaccgtctccgggagctgcatgtgtcagaggttttcaccgtcatcaccgaaacgcgcgaggcagggtgccttgatgtgggcgccggcggtcgagtggcgacggcgcggcttgtccgcgccctggtagattgcctggccgtaggccagccatttttgagcggccagcggccgcgataggccgacgcgaagcggcggggcgtagggagcgcagcgaccgaagggtaggcgctttttgcagctcttcggctgtgcgctggccagacagttatgcacaggccaggcgggttttaagagttttaataagttttaaagagttttaggcggaaaaatcgccttttttctcttttatatcagtcacttacatgtgtgaccggttcccaatgtacggctttgggttcccaatgtacgggttccggttcccaatgtacggctttgggttcccaatgtacgtgctatccacaggaaagagaccttttcgacctttttcccctgctagggcaatttgccctagcatctgctccgtacattaggaaccggcggatgcttcgccctcgatcaggttgcggtagcgcatgactaggatcgggccagcctgccccgcctcctccttcaaatcgtactccggcaggtcatttgacccgatcagcttgcgcacggtgaaacagaacttcttgaactctccggcgctgccactgcgttcgtagatcgtcttgaacaaccatctggcttctgccttgcctgcggcgcggcgtgccaggcggtagagaaaacggccgatgccgggatcgatcaaaaagtaatcggggtgaaccgtcagcacgtccgggttcttgccttctgtgatctcgcggtacatccaatcagctagctcgatctcgatgtactccggccgcccggtttcgctctttacgatcttgtagcggctaatcaaggcttcaccctcggataccgtcaccaggcggccgttcttggccttcttcgtacgctgcatggcaacgtgcgtggtgtttaaccgaatgcaggtttctaccaggtcgtctttctgctttccgccatcggctcgccggcagaacttgagtacgtccgcaacgtgtggacggaacacgcggccgggcttgtctcccttcccttcccggtatcggttcatggattcggttagatgggaaaccgccatcagtaccaggtcgtaatcccacacactggccatgccggccggccctgcggaaacctctacgtgcccgtctggaagctcgtagcggatcacctcgccagctcgtcggtcacgcttcgacagacggaaaacggccacgtccatgatgctgcgactatcgcgggtgcccacgtcatagagcatcggaacgaaaaaatctggttgctcgtcgcccttgggcggcttcctaatcgacggcgcaccggctgccggcggttgccgggattctttgcggattcgatcagcggccgcttgccacgattcaccggggcgtgcttctgcctcgatgcgttgccgctgggcggcctgcgcggccttcaacttctccaccaggtcatcacccagcgccgcgccgatttgtaccgggccggatggtttgcgaccgtcacgccgattcctcgggcttgggggttccagtgccattgcagggccggcagacaacccagccgcttacgcctggccaaccgcccgttcctccacacatggggcattccacggcgtcggtgcctggttgttcttgattttccatgccgcctcctttagccgctaaaattcatctactcatttattcatttgctcatttactctggtagctgcgcgatgtattcagatagcagctcggtaatggtcttgccttggcgtaccgcgtacatcttcagcttggtgtgatcctccgccggcaactgaaagttgacccgcttcatggctggcgtgtctgccaggctggccaacgttgcagccttgctgctgcgtgcgctcggacggccggcacttagcgtgtttgtgcttttgctcattttctctttacctcattaactcaaatgagttttgatttaatttcagcggccagcgcctggacctcgcgggcagcgtcgccctcgggttctgattcaagaacggttgtgccggcggcggcagtgcctgggtagctcacgcgctgcgtgatacgggactcaagaatgggcagctcgtacccggccagcgcctcggcaacctcaccgccgatgcgcgtgcctttgatcgcccgcgacacgacaaaggccgcttgtagccttccatccgtgacctcaatgcgctgcttaaccagctccaccaggtcggcggtggcccatatgtcgtaagggcttggctgcaccggaatcagcacgaagtcggctgccttgatcgcggacacagccaagtccgccgcctggggcgctccgtcgatcactacgaagtcgcgccggccgatggccttcacgtcgcggtcaatcgtcgggcggtcgatgccgacaacggttagcggttgatcttcccgcacggccgcccaatcgcgggcactgccctggggatcggaatcgactaacagaacatcggccccggcgagttgcagggcgcgggctagatgggttgcgatggtcgtcttgcctgacccgcctttctggttaagtacagcgataaccttcatgcgttccccttgcgtatttgtttatttactcatcgcatcatatacgcagcgaccgcatgacgcaagctgttttactcaaatacacatcacctttttagacggcggcgctcggtttcttcagcggccaagctggccggccaggccgccagcttggcatcagacaaaccggccaggatttcatgcagccgcacggttgagacgtgcgcgggcggctcgaacacgtacccggccgcgatcatctccgcctcgatctcttcggtaatgaaaaacggttcgtcctggccgtcctggtgcggtttcatgcttgttcctcttggcgttcattctcggcggccgccagggcgtcggcctcggtcaatgcgtcctcacggaaggcaccgcgccgcctggcctcggtgggcgtcacttcctcgctgcgctcaagtgcgcggtacagggtcgagcgatgcacgccaagcagtgcagccgcctctttcacggtgcggccttcctggtcgatcagctcgcgggcgtgcgcgatctgtgccggggtgagggtagggcgggggccaaacttcacgcctcgggccttggcggcctcgcgcccgctccgggtgcggtcgatgattagggaacgctcgaactcggcaatgccggcgaacacggtcaacaccatgcggccggccggcgtggtggtgtcggcccacggctctgccaggctacgcaggcccgcgccggcctcctggatgcgctcggcaatgtccagtaggtcgcgggtgctgcgggccaggcggtctagcctggtcactgtcacaacgtcgccagggcgtaggtggtcaagcatcctggccagctccgggcggtcgcgcctggtgccggtgatcttctcggaaaacagcttggtgcagccggccgcgtgcagttcggcccgttggttggtcaagtcctggtcgtcggtgctgacgcgggcatagcccagcaggccagcggcggcgctcttgttcatggcgtaatgtctccggttctagtcgcaagtattctactttatgcgactaaaacacgcgacaagaaaacgccaggaaaagggcagggcggcagcctgtcgcgtaacttaggacttgtgcgacatgtcgttttcagaagacggctgcactgaacgtcagaagccgactgcactatagcagcggaggggttggatcaaagtactttgatcccgaggggaaccctgtggttggcatgcacatacaaatggacgaacggataaaccttttcacgcccttttaaatatccgttattctaataaacgctcttttctcttaggtttacccgccaatatatcctgtcaaacactgatagtttaaactgaaggcgggaaacgacaatctgatccaagctcaagctaagcttgagctctcccatatggtcgactagagccaagctgatctcctttgccccggagatcaccatggacgactttctctatctctacgatctaggaagaaagttcgacggagaaggtgacgataccatgttcaccaccgataatgagaagattagcctcttcaatttcagaaagaatgctgacccacagatggttagagaggcctacgcggcaggtctcatcaagacgatctacccgagtaataatctccaggagatcaaataccttcccaagaaggttaaagatgcagtcaaaagattcaggactaactgcatcaagaacacagagaaagatatatttctcaagatcagaagtactattccagtatggacgattcaaggcttgcttcataaaccaaggcaagtaatagagattggagtctctaagaaagtagttcctactgaatcaaaggccatggagtcaaaaattcagatcgaggatctaacagaactcgccgtgaagactggcgaacagttcatacagagtcttttacgactcaatgacaagaagaaaatcttcgtcaacatggtggagcacgacactctcgtctactccaagaatatcaaagatacagtctcagaagaccaaagggctattgagacttttcaacaaagggtaatatcgggaaacctcctcggattccattgcccagctatctgtcacttcatcaaaaggacagtagaaaaggaaggtggcacctacaaatgccatcattgcgataaaggaaaggctatcgttcaagatgcctctgccgacagtggtcccaaagatggacccccacccacgaggagcatcgtggaaaaagaagacgttccaaccacgtcttcaaagcaagtggattgatgtgatatctccactgacgtaagggatgacgcacaatcccactatccttcgcaagacccttcctctatataaggaagttcatttcatttggagaggactccggtatttttacaacaataccacaacaaaacaaacaacaaacaacattacaatttactattctagtcgacctgcaggcggccgcactagtgatatcacaagtttgtacaaaaaagctgaacgagaaacgtaaaatgatataaatatcaatatattaaattagattttgcataaaaaacagactacataatactgtaaaacacaacatatccagtcactatggcggccgcattaggcaccccaggctttacactttatgcttccggctcgtataatgtgtggattttgagttaggatccggcgagattttcaggagctaaggaagctaaaatggagaaaaaaatcactggatataccaccgttgatatatcccaatggcatcgtaaagaacattttgaggcatttcagtcagttgctcaatgtacctataaccagaccgttcagctggatattacggcctttttaaagaccgtaaagaaaaataagcacaagttttatccggcctttattcacattcttgcccgcctgatgaatgctcatccggaattccgtatggcaatgaaagacggtgagctggtgatatgggatagtgttcacccttgttacaccgttttccatgagcaaactgaaacgttttcatcgctctggagtgaataccacgacgatttccggcagtttctacacatatattcgcaagatgtggcgtgttacggtgaaaacctggcctatttccctaaagggtttattgagaatatgtttttcgtctcagccaatccctgggtgagtttcaccagttttgatttaaacgtggccaatatggacaacttcttcgcccccgttttcaccatgggcaaatattatacgcaaggcgacaaggtgctgatgccgctggcgattcaggttcatcatgccgtctgtgatggcttccatgtcggcagaatgcttaatgaattacaacagtactgcgatgagtggcagggcggggcgtaaacgcgtggatccggcttactaaaagccagataacagtatgcgtatttgcgcgctgatttttgcggtataagaatatatactgatatgtatacccgaagtatgtcaaaaagaggtgtgctatgaagcagcgtattacagtgacagttgacagcgacagctatcagttgctcaaggcatatatgatgtcaatatctccggtctggtaagcacaaccatgcagaatgaagcccgtcgtctgcgtgccgaacgctggaaagcggaaaatcaggaagggatggctgaggtcgcccggtttattgaaatgaacggctcttttgctgacgagaacagggactggtgaaatgcagtttaaggtttacacctataaaagagagagccgttatcgtctgtttgtggatgtacagagtgatattattgacacgcccgggcgacggatggtgatccccctggccagtgcacgtctgctgtcagataaagtctcccgtgaactttacccggtggtgcatatcggggatgaaagctggcgcatgatgaccaccgatatggccagtgtgccggtctccgttatcggggaagaagtggctgatctcagccaccgcgaaaatgacatcaaaaacgccattaacctgatgttctggggaatataaatgtcaggctcccttatacacagccagtctgcaggtcgaccatagtgactggatatgttgtgttttacagtattatgtagtctgttttttatgcaaaatctaatttaatatattgatatttatatcattttacgtttctcgttcagctttcttgtacaaagtggtgatatcccgcggccatgctagagtccgcaaaaatcaccagtctctctctacaaatctatctctctctatttttctccagaataatgtgtgagtagttcccagataagggaattagggttcttatagggtttcgctcatgtgttgagcatataagaaacccttagtatgtatttgtatttgtaaaatacttctatcaataaaatttctaattcctaaaaccaaaatccagtgacctgcaggcatgcgacgtcg

SEQ ID NO: 359 - DNA, 9966 bp, Artificial Sequence
  pK7WG2-35S:41D01_His_KDEL
ggccctctagaggatccccgggtaccgcgaattatcatacatgagaattaagggagtcacgttatgacccccgccgatgacgcgggacaagccgttttacgtttggaactgacagaaccgcaacgttgaaggagccactcagccgcgggtttctggagtttaatgagctaagcacatacgtcagaaaccattattgcgcgttcaaaagtcgcctaaggtcactatcagctagcaaatatttcttgtcaaaaatgctccactgacgttccataaattcccctcggtatccaattagagtctcatattcactctcaactcgatcgaggcatgattgaacaagatggattgcacgcaggttctccggccgcttgggtggagaggctattcggctatgactgggcacaacagacaatcggctgctctgatgccgccgtgttccggctgtcagcgcaggggcgcccggttctttttgtcaagaccgacctgtccggtgccctgaatgaactccaagacgaggcagcgcggctatcgtggctggccacgacgggcgttccttgcgcagctgtgctcgacgttgtcactgaagcgggaagggactggctgctattgggcgaagtgccggggcaggatctcctgtcatctcaccttgctcctgccgagaaagtatccatcatggctgatgcaatgcggcggctgcatacgcttgatccggctacctgcccattcgaccaccaagcgaaacatcgcatcgagcgaggacgtactcggatggaagccggtcttgtcgatcaggatgatctggacgaagagcatcaggggctcgcgccagccgaactgttcgccaggctcaaggcgcggatgcccgacggcgaggatctcgtcgtgacccagggcgatgcctgcttgccgaatatcatggtggaaaatggccgcttttctggattcatcgactgtggccggctgggtgtggcggaccgctatcaggacatagcgttggctacccgtgatattgctgaagagcttggcggcgaatgggctgaccgcttcctcgtgctttacggtatcgccgctcccgattcgcagcgcatcgccttctatcgccttcttgacgagttcttctgagcgggactctggggttcggactctagctagagtcaagcagatcgttcaaacatttggcaataaagtttcttaagattgaatcctgttgccggtcttgcgatgattatcatataatttctgttgaattacgttaagcatgtaataattaacatgtaatgcatgacgttatttatgagatgggttttttgattagagtcccgcaattatacatttaatacgcgatagaaaacaaaatatagcgcgcaaactaggataaattatcgcgcgcggtgtcatctatgttactagatcgaccggcatgcaagctgataattcaattcggcgttaattcagtacattaaaaacgtccgcaatgtgttattaagttgtctaagcgtcaatttgtttacaccacaatatatcctgccaccagccagccaacagctccccgaccggcagctcggcacaaaatcaccactcgatacaggcagcccatcagtccgggacggcgtcagcgggagagccgttgtaaggcggcagactttgctcatgttaccgatgctattcggaagaacggcaactaagctgccgggtttgaaacacggatgatctcgcggagggtagcatgttgattgtaacgatgacagagcgttgctgcctgtgatcaattcgggcacgaacccagtggacataagcctcgttcggttcgtaagctgtaatgcaagtagcgtaactgccgtcacgcaactggtccagaaccttgaccgaacgcagcggtggtaacggcgcagtggcggttttcatggcttcttgttatgacatgtttttttggggtacagtctatgcctcgggcatccaagcagcaagcgcgttacgccgtgggtcgatgtttgatgttatggagcagcaacgatgttacgcagcagggcagtcgccctaaaacaaagttaaacatcatgggggaagcggtgatcgccgaagtatcgactcaactatcagaggtagttggcgtcatcgagcgccatctcgaaccgacgttgctggccgtacatttgtacggctccgcagtggatggcggcctgaagccacacagtgatattgatttgctggttacggtgaccgtaaggcttgatgaaacaacgcggcgagctttgatcaacgaccttttggaaacttcggcttcccctggagagagcgagattctccgcgctgtagaagtcaccattgttgtgcacgacgacatcattccgtggcgttatccagctaagcgcgaactgcaatttggagaatggcagcgcaatgacattcttgcaggtatcttcgagccagccacgatcgacattgatctggctatcttgctgacaaaagcaagagaacatagcgttgccttggtaggtccagcggcggaggaactctttgatccggttcctgaacaggatctatttgaggcgctaaatgaaaccttaacgctatggaactcgccgcccgactgggctggcgatgagcgaaatgtagtgcttacgttgtcccgcatttggtacagcgcagtaaccggcaaaatcgcgccgaaggatgtcgctgccgactgggcaatggagcgcctgccggcccagtatcagcccgtcatacttgaagctagacaggcttatcttggacaagaagaagatcgcttggcctcgcgcgcagatcagttggaagaatttgtccactacgtgaaaggcgagatcaccaaggtagtcggcaaataatgtctagctagaaattcgttcaagccgacgccgcttcgccggcgttaactcaagcgattagatgcactaagcacataattgctcacagccaaactatcaggtcaagtctgcttttattatttttaagcgtgcataataagccctacacaaattgggagatatatcatgcatgaccaaaatcccttaacgtgagttttcgttccactgagcgtcagaccccgtagaaaagatcaaaggatcttcttgagatcctttttttctgcgcgtaatctgctgcttgcaaacaaaaaaaccaccgctaccagcggtggtttgtttgccggatcaagagctaccaactctttttccgaaggtaactggcttcagcagagcgcagataccaaatactgtccttctagtgtagccgtagttaggccaccacttcaagaactctgtagcaccgcctacatacctcgctctgctaatcctgttaccagtggctgctgccagtggcgataagtcgtgtcttaccgggttggactcaagacgatagttaccggataaggcgcagcggtcgggctgaacggggggttcgtgcacacagcccagcttggagcgaacgacctacaccgaactgagatacctacagcgtgagctatgagaaagcgccacgcttcccgaagggagaaaggcggacaggtatccggtaagcggcagggtcggaacaggagagcgcacgagggagcttccagggggaaacgcctggtatctttatagtcctgtcgggtttcgccacctctgacttgagcgtcgatttttgtgatgctcgtcaggggggcggagcctatggaaaaacgccagcaacgcggcctttttacggttcctggccttttgctggccttttgctcacatgttctttcctgcgttatcccctgattctgtggataaccgtattaccgcctttgagtgagctgataccgctcgccgcagccgaacgaccgagcgcagcgagtcagtgagcgaggaagcggaagagcgcctgatgcggtattttctccttacgcatctgtgcggtatttcacaccgcatatggtgcactctcagtacaatctgctctgatgccgcatagttaagccagtatacactccgctatcgctacgtgactgggtcatggctgcgccccgacacccgccaacacccgctgacgcgccctgacgggcttgtctgctcccggcatccgcttacagacaagctgtgaccgtctccgggagctgcatgtgtcagaggttttcaccgtcatcaccgaaacgcgcgaggcagggtgccttgatgtgggcgccggcggtcgagtggcgacggcgcggcttgtccgcgccctggtagattgcctggccgtaggccagccatttttgagcggccagcggccgcgataggccgacgcgaagcggcggggcgtagggagcgcagcgaccgaagggtaggcgctttttgcagctcttcggctgtgcgctggccagacagttatgcacaggccaggcgggttttaagagttttaataagttttaaagagttttaggcggaaaaatcgccttttttctcttttatatcagtcacttacatgtgtgaccggttcccaatgtacggctttgggttcccaatgtacgggttccggttcccaatgtacggctttgggttcccaatgtacgtgctatccacaggaaagagaccttttcgacctttttcccctgctagggcaatttgccctagcatctgctccgtacattaggaaccggcggatgcttcgccctcgatcaggttgcggtagcgcatgactaggatcgggccagcctgccccgcctcctccttcaaatcgtactccggcaggtcatttgacccgatcagcttgcgcacggtgaaacagaacttcttgaactctccggcgctgccactgcgttcgtagatcgtcttgaacaaccatctggcttctgccttgcctgcggcgcggcgtgccaggcggtagagaaaacggccgatgccgggatcgatcaaaaagtaatcggggtgaaccgtcagcacgtccgggttcttgccttctgtgatctcgcggtacatccaatcagctagctcgatctcgatgtactccggccgcccggtttcgctctttacgatcttgtagcggctaatcaaggcttcaccctcggataccgtcaccaggcggccgttcttggccttcttcgtacgctgcatggcaacgtgcgtggtgtttaaccgaatgcaggtttctaccaggtcgtctttctgctttccgccatcggctcgccggcagaacttgagtacgtccgcaacgtgtggacggaacacgcggccgggcttgtctcccttcccttcccggtatcggttcatggattcggttagatgggaaaccgccatcagtaccaggtcgtaatcccacacactggccatgccggccggccctgcggaaacctctacgtgcccgtctggaagctcgtagcggatcacctcgccagctcgtcggtcacgcttcgacagacggaaaacggccacgtccatgatgctgcgactatcgcgggtgcccacgtcatagagcatcggaacgaaaaaatctggttgctcgtcgcccttgggcggcttcctaatcgacggcgcaccggctgccggcggttgccgggattctttgcggattcgatcagcggccgcttgccacgattcaccggggcgtgcttctgcctcgatgcgttgccgctgggcggcctgcgcggccttcaacttctccaccaggtcatcacccagcgccgcgccgatttgtaccgggccggatggtttgcgaccgtcacgccgattcctcgggcttgggggttccagtgccattgcagggccggcagacaacccagccgcttacgcctggccaaccgcccgttcctccacacatggggcattccacggcgtcggtgcctggttgttcttgattttccatgccgcctcctttagccgctaaaattcatctactcatttattcatttgctcatttactctggtagctgcgcgatgtattcagatagcagctcggtaatggtcttgccttggcgtaccgcgtacatcttcagcttggtgtgatcctccgccggcaactgaaagttgacccgcttcatggctggcgtgtctgccaggctggccaacgttgcagccttgctgctgcgtgcgctcggacggccggcacttagcgtgtttgtgcttttgctcattttctctttacctcattaactcaaatgagttttgatttaatttcagcggccagcgcctggacctcgcgggcagcgtcgccctcgggttctgattcaagaacggttgtgccggcggcggcagtgcctgggtagctcacgcgctgcgtgatacgggactcaagaatgggcagctcgtacccggccagcgcctcggcaacctcaccgccgatgcgcgtgcctttgatcgcccgcgacacgacaaaggccgcttgtagccttccatccgtgacctcaatgcgctgcttaaccagctccaccaggtcggcggtggcccatatgtcgtaagggcttggctgcaccggaatcagcacgaagtcggctgccttgatcgcggacacagccaagtccgccgcctggggcgctccgtcgatcactacgaagtcgcgccggccgatggccttcacgtcgcggtcaatcgtcgggcggtcgatgccgacaacggttagcggttgatcttcccgcacggccgcccaatcgcgggcactgccctggggatcggaatcgactaacagaacatcggccccggcgagttgcagggcgcgggctagatgggttgcgatggtcgtcttgcctgacccgcctttctggttaagtacagcgataaccttcatgcgttccccttgcgtatttgtttatttactcatcgcatcatatacgcagcgaccgcatgacgcaagctgttttactcaaatacacatcacctttttagacggcggcgctcggtttcttcagcggccaagctggccggccaggccgccagcttggcatcagacaaaccggccaggatttcatgcagccgcacggttgagacgtgcgcgggcggctcgaacacgtacccggccgcgatcatctccgcctcgatctcttcggtaatgaaaaacggttcgtcctggccgtcctggtgcggtttcatgcttgttcctcttggcgttcattctcggcggccgccagggcgtcggcctcggtcaatgcgtcctcacggaaggcaccgcgccgcctggcctcggtgggcgtcacttcctcgctgcgctcaagtgcgcggtacagggtcgagcgatgcacgccaagcagtgcagccgcctctttcacggtgcggccttcctggtcgatcagctcgcgggcgtgcgcgatctgtgccggggtgagggtagggcgggggccaaacttcacgcctcgggccttggcggcctcgcgcccgctccgggtgcggtcgatgattagggaacgctcgaactcggcaatgccggcgaacacggtcaacaccatgcggccggccggcgtggtggtgtcggcccacggctctgccaggctacgcaggcccgcgccggcctcctggatgcgctcggcaatgtccagtaggtcgcgggtgctgcgggccaggcggtctagcctggtcactgtcacaacgtcgccagggcgtaggtggtcaagcatcctggccagctccgggcggtcgcgcctggtgccggtgatcttctcggaaaacagcttggtgcagccggccgcgtgcagttcggcccgttggttggtcaagtcctggtcgtcggtgctgacgcgggcatagcccagcaggccagcggcggcgctcttgttcatggcgtaatgtctccggttctagtcgcaagtattctactttatgcgactaaaacacgcgacaagaaaacgccaggaaaagggcagggcggcagcctgtcgcgtaacttaggacttgtgcgacatgtcgttttcagaagacggctgcactgaacgtcagaagccgactgcactatagcagcggaggggttggatcaaagtactttgatcccgaggggaaccctgtggttggcatgcacatacaaatggacgaacggataaaccttttcacgcccttttaaatatccgttattctaataaacgctcttttctcttaggtttacccgccaatatatcctgtcaaacactgatagtttaaactgaaggcgggaaacgacaatctgatccaagctcaagctaagcttgagctctcccatatggtcgagatctcctttgccccggagatcaccatggacgactttctctatctctacgatctaggaagaaagttcgacggagaaggtgacgataccatgttcaccaccgataatgagaagattagcctcttcaatttcagaaagaatgctgacccacagatggttagagaggcctacgcggcaggtctcatcaagacgatctacccgagtaataatctccaggagatcaaataccttcccaagaaggttaaagatgcagtcaaaagattcaggactaactgcatcaagaacacagagaaagatatatttctcaagatcagaagtactattccagtatggacgattcaaggcttgcttcataaaccaaggcaagtaatagagattggagtctctaagaaagtagttcctactgaatcaaaggccatggagtcaaaaattcagatcgaggatctaacagaactcgccgtgaagactggcgaacagttcatacagagtcttttacgactcaatgacaagaagaaaatcttcgtcaacatggtggagcacgacactctcgtctactccaagaatatcaaagatacagtctcagaagaccaaagggctattgagacttttcaacaaagggtaatatcgggaaacctcctcggattccattgcccagctatctgtcacttcatcaaaaggacagtagaaaaggaaggtggcacctacaaatgccatcattgcgataaaggaaaggctatcgttcaagatgcccctgccgacagtggtcccaaagatggacccccacccacgaggagcatcgtggaaaaagaagacgttccaaccacgtcttcaaagcaagtggattgatgtgatatctccactgacgtaagggatgacgcacaatcccactatccttcgcaagacccttcctctatataaggaagttcatttcatttggagaggactccggtatttttacaacaattaccacaacaaaacaaacaacaaacaacattacaatttactattctagtcgacctgcaggcggccgcactagtgatatcacaagtttgtacaaaaaagcaggctgaattcccaccatggcaaacaagcttttcttggtgtgcgctaccttcgctctttgcttccttttgactaacgctcaggttcagctgcaggaatctggtggtggacttgttcaagctggtggatctcttagactctcttgcgctgcttctggaaggaccttctctagatatggaatgggatggttcaggcagctccctggaaaacagagagagcttgttacctctatcaccaggggtggaactaccacctacgctgattctgtgaagggaaggttcaccatctctagggataacgctaagaacaccgtgtacctccagatgaactctctcaagcctgaggataccgctgtgtactactgcaacgctagatctatttggagggattactggggacagggaactcaggtcaccgtttcttcagcggccgcacatcatcatcaccatcatggtgctgctaaggatgagctttgaggatccacccagctttcttgtacaaagtggtgatatcccgcggccatgctagagtccgcaaaaatcaccagtctctctctacaaatctatctctctctatttttctccagaataatgtgtgagtagttcccagataagggaattagggttcttatagggtttcgctcatgtgttgagcatataagaaacccttagtatgtatttgtatttgtaaaatacttctatcaataaaatttctaattcctaaaaccaaaatccagtgacctgcaggcatgcgacgtcg

SEQ ID NO: 360 - DNA, 10641 bp, Artificial Sequence
  pK7WG2-35S:sec_41D01_hinge_Fc_His
ggccctctagaggatccccgggtaccgcgaattatcatacatgagaattaagggagtcacgttatgacccccgccgatgacgcgggacaagccgttttacgtttggaactgacagaaccgcaacgttgaaggagccactcagccgcgggtttctggagtttaatgagctaagcacatacgtcagaaaccattattgcgcgttcaaaagtcgcctaaggtcactatcagctagcaaatatttcttgtcaaaaatgctccactgacgttccataaattcccctcggtatccaattagagtctcatattcactctcaactcgatcgaggcatgattgaacaagatggattgcacgcaggttctccggccgcttgggtggagaggctattcggctatgactgggcacaacagacaatcggctgctctgatgccgccgtgttccggctgtcagcgcaggggcgcccggttctttttgtcaagaccgacctgtccggtgccctgaatgaactccaagacgaggcagcgcggctatcgtggctggccacgacgggcgttccttgcgcagctgtgctcgacgttgtcactgaagcgggaagggactggctgctattgggcgaagtgccggggcaggatctcctgtcatctcaccttgctcctgccgagaaagtatccatcatggctgatgcaatgcggcggctgcatacgcttgatccggctacctgcccattcgaccaccaagcgaaacatcgcatcgagcgaggacgtactcggatggaagccggtcttgtcgatcaggatgatctggacgaagagcatcaggggctcgcgccagccgaactgttcgccaggctcaaggcgcggatgcccgacggcgaggatctcgtcgtgacccagggcgatgcctgcttgccgaatatcatggtggaaaatggccgcttttctggattcatcgactgtggccggctgggtgtggcggaccgctatcaggacatagcgttggctacccgtgatattgctgaagagcttggcggcgaatgggctgaccgcttcctcgtgctttacggtatcgccgctcccgattcgcagcgcatcgccttctatcgccttcttgacgagttcttctgagcgggactctggggttcggactctagctagagtcaagcagatcgttcaaacatttggcaataaagtttcttaagattgaatcctgttgccggtcttgcgatgattatcatataatttctgttgaattacgttaagcatgtaataattaacatgtaatgcatgacgttatttatgagatgggttttttgattagagtcccgcaattatacatttaatacgcgatagaaaacaaaatatagcgcgcaaactaggataaattatcgcgcgcggtgtcatctatgttactagatcgaccggcatgcaagctgataattcaattcggcgttaattcagtacattaaaaacgtccgcaatgtgttattaagttgtctaagcgtcaatttgtttacaccacaatatatcctgccaccagccagccaacagctccccgaccggcagctcggcacaaaatcaccactcgatacaggcagcccatcagtccgggacggcgtcagcgggagagccgttgtaaggcggcagactttgctcatgttaccgatgctattcggaagaacggcaactaagctgccgggtttgaaacacggatgatctcgcggagggtagcatgttgattgtaacgatgacagagcgttgctgcctgtgatcaattcgggcacgaacccagtggacataagcctcgttcggttcgtaagctgtaatgcaagtagcgtaactgccgtcacgcaactggtccagaaccttgaccgaacgcagcggtggtaacggcgcagtggcggttttcatggcttcttgttatgacatgtttttttggggtacagtctatgcctcgggcatccaagcagcaagcgcgttacgccgtgggtcgatgtttgatgttatggagcagcaacgatgttacgcagcagggcagtcgccctaaaacaaagttaaacatcatgggggaagcggtgatcgccgaagtatcgactcaactatcagaggtagttggcgtcatcgagcgccatctcgaaccgacgttgctggccgtacatttgtacggctccgcagtggatggcggcctgaagccacacagtgatattgatttgctggttacggtgaccgtaaggcttgatgaaacaacgcggcgagctttgatcaacgaccttttggaaacttcggcttcccctggagagagcgagattctccgcgctgtagaagtcaccattgttgtgcacgacgacatcattccgtggcgttatccagctaagcgcgaactgcaatttggagaatggcagcgcaatgacattcttgcaggtatcttcgagccagccacgatcgacattgatctggctatcttgctgacaaaagcaagagaacatagcgttgccttggtaggtccagcggcggaggaactctttgatccggttcctgaacaggatctatttgaggcgctaaatgaaaccttaacgctatggaactcgccgcccgactgggctggcgatgagcgaaatgtagtgcttacgttgtcccgcatttggtacagcgcagtaaccggcaaaatcgcgccgaaggatgtcgctgccgactgggcaatggagcgcctgccggcccagtatcagcccgtcatacttgaagctagacaggcttatcttggacaagaagaagatcgcttggcctcgcgcgcagatcagttggaagaatttgtccactacgtgaaaggcgagatcaccaaggtagtcggcaaataatgtctagctagaaattcgttcaagccgacgccgcttcgccggcgttaactcaagcgattagatgcactaagcacataattgctcacagccaaactatcaggtcaagtctgcttttattatttttaagcgtgcataataagccctacacaaattgggagatatatcatgcatgaccaaaatcccttaacgtgagttttcgttccactgagcgtcagaccccgtagaaaagatcaaaggatcttcttgagatcctttttttctgcgcgtaatctgctgcttgcaaacaaaaaaaccaccgctaccagcggtggtttgtttgccggatcaagagctaccaactctttttccgaaggtaactggcttcagcagagcgcagataccaaatactgtccttctagtgtagccgtagttaggccaccacttcaagaactctgtagcaccgcctacatacctcgctctgctaatcctgttaccagtggctgctgccagtggcgataagtcgtgtcttaccgggttggactcaagacgatagttaccggataaggcgcagcggtcgggctgaacggggggttcgtgcacacagcccagcttggagcgaacgacctacaccgaactgagatacctacagcgtgagctatgagaaagcgccacgcttcccgaagggagaaaggcggacaggtatccggtaagcggcagggtcggaacaggagagcgcacgagggagcttccagggggaaacgcctggtatctttatagtcctgtcgggtttcgccacctctgacttgagcgtcgatttttgtgatgctcgtcaggggggcggagcctatggaaaaacgccagcaacgcggcctttttacggttcctggccttttgctggccttttgctcacatgttctttcctgcgttatcccctgattctgtggataaccgtattaccgcctttgagtgagctgataccgctcgccgcagccgaacgaccgagcgcagcgagtcagtgagcgaggaagcggaagagcgcctgatgcggtattttctccttacgcatctgtgcggtatttcacaccgcatatggtgcactctcagtacaatctgctctgatgccgcatagttaagccagtatacactccgctatcgctacgtgactgggtcatggctgcgccccgacacccgccaacacccgctgacgcgccctgacgggcttgtctgctcccggcatccgcttacagacaagctgtgaccgtctccgggagctgcatgtgtcagaggttttcaccgtcatcaccgaaacgcgcgaggcagggtgccttgatgtgggcgccggcggtcgagtggcgacggcgcggcttgtccgcgccctggtagattgcctggccgtaggccagccatttttgagcggccagcggccgcgataggccgacgcgaagcggcggggcgtagggagcgcagcgaccgaagggtaggcgctttttgcagctcttcggctgtgcgctggccagacagttatgcacaggccaggcgggttttaagagttttaataagttttaaagagttttaggcggaaaaatcgccttttttctcttttatatcagtcacttacatgtgtgaccggttcccaatgtacggctttgggttcccaatgtacgggttccggttcccaatgtacggctttgggttcccaatgtacgtgctatccacaggaaagagaccttttcgacctttttcccctgctagggcaatttgccctagcatctgctccgtacattaggaaccggcggatgcttcgccctcgatcaggttgcggtagcgcatgactaggatcgggccagcctgccccgcctcctccttcaaatcgtactccggcaggtcatttgacccgatcagcttgcgcacggtgaaacagaacttcttgaactctccggcgctgccactgcgttcgtagatcgtcttgaacaaccatctggcttctgccttgcctgcggcgcggcgtgccaggcggtagagaaaacggccgatgccgggatcgatcaaaaagtaatcggggtgaaccgtcagcacgtccgggttcttgccttctgtgatctcgcggtacatccaatcagctagctcgatctcgatgtactccggccgcccggtttcgctctttacgatcttgtagcggctaatcaaggcttcaccctcggataccgtcaccaggcggccgttcttggccttcttcgtacgctgcatggcaacgtgcgtggtgtttaaccgaatgcaggtttctaccaggtcgtctttctgctttccgccatcggctcgccggcagaacttgagtacgtccgcaacgtgtggacggaacacgcggccgggcttgtctcccttcccttcccggtatcggttcatggattcggttagatgggaaaccgccatcagtaccaggtcgtaatcccacacactggccatgccggccggccctgcggaaacctctacgtgcccgtctggaagctcgtagcggatcacctcgccagctcgtcggtcacgcttcgacagacggaaaacggccacgtccatgatgctgcgactatcgcgggtgcccacgtcatagagcatcggaacgaaaaaatctggttgctcgtcgcccttgggcggcttcctaatcgacggcgcaccggctgccggcggttgccgggattctttgcggattcgatcagcggccgcttgccacgattcaccggggcgtgcttctgcctcgatgcgttgccgctgggcggcctgcgcggccttcaacttctccaccaggtcatcacccagcgccgcgccgatttgtaccgggccggatggtttgcgaccgtcacgccgattcctcgggcttgggggttccagtgccattgcagggccggcagacaacccagccgcttacgcctggccaaccgcccgttcctccacacatggggcattccacggcgtcggtgcctggttgttcttgattttccatgccgcctcctttagccgctaaaattcatctactcatttattcatttgctcatttactctggtagctgcgcgatgtattcagatagcagctcggtaatggtcttgccttggcgtaccgcgtacatcttcagcttggtgtgatcctccgccggcaactgaaagttgacccgcttcatggctggcgtgtctgccaggctggccaacgttgcagccttgctgctgcgtgcgctcggacggccggcacttagcgtgtttgtgcttttgctcattttctctttacctcattaactcaaatgagttttgatttaatttcagcggccagcgcctggacctcgcgggcagcgtcgccctcgggttctgattcaagaacggttgtgccggcggcggcagtgcctgggtagctcacgcgctgcgtgatacgggactcaagaatgggcagctcgtacccggccagcgcctcggcaacctcaccgccgatgcgcgtgcctttgatcgcccgcgacacgacaaaggccgcttgtagccttccatccgtgacctcaatgcgctgcttaaccagctccaccaggtcggcggtggcccatatgtcgtaagggcttggctgcaccggaatcagcacgaagtcggctgccttgatcgcggacacagccaagtccgccgcctggggcgctccgtcgatcactacgaagtcgcgccggccgatggccttcacgtcgcggtcaatcgtcgggcggtcgatgccgacaacggttagcggttgatcttcccgcacggccgcccaatcgcgggcactgccctggggatcggaatcgactaacagaacatcggccccggcgagttgcagggcgcgggctagatgggttgcgatggtcgtcttgcctgacccgcctttctggttaagtacagcgataaccttcatgcgttccccttgcgtatttgtttatttactcatcgcatcatatacgcagcgaccgcatgacgcaagctgttttactcaaatacacatcacctttttagacggcggcgctcggtttcttcagcggccaagctggccggccaggccgccagcttggcatcagacaaaccggccaggatttcatgcagccgcacggttgagacgtgcgcgggcggctcgaacacgtacccggccgcgatcatctccgcctcgatctcttcggtaatgaaaaacggttcgtcctggccgtcctggtgcggtttcatgcttgttcctcttggcgttcattctcggcggccgccagggcgtcggcctcggtcaatgcgtcctcacggaaggcaccgcgccgcctggcctcggtgggcgtcacttcctcgctgcgctcaagtgcgcggtacagggtcgagcgatgcacgccaagcagtgcagccgcctctttcacggtgcggccttcctggtcgatcagctcgcgggcgtgcgcgatctgtgccggggtgagggtagggcgggggccaaacttcacgcctcgggccttggcggcctcgcgcccgctccgggtgcggtcgatgattagggaacgctcgaactcggcaatgccggcgaacacggtcaacaccatgcggccggccggcgtggtggtgtcggcccacggctctgccaggctacgcaggcccgcgccggcctcctggatgcgctcggcaatgtccagtaggtcgcgggtgctgcgggccaggcggtctagcctggtcactgtcacaacgtcgccagggcgtaggtggtcaagcatcctggccagctccgggcggtcgcgcctggtgccggtgatcttctcggaaaacagcttggtgcagccggccgcgtgcagttcggcccgttggttggtcaagtcctggtcgtcggtgctgacgcgggcatagcccagcaggccagcggcggcgctcttgttcatggcgtaatgtctccggttctagtcgcaagtattctactttatgcgactaaaacacgcgacaagaaaacgccaggaaaagggcagggcggcagcctgtcgcgtaacttaggacttgtgcgacatgtcgttttcagaagacggctgcactgaacgtcagaagccgactgcactatagcagcggaggggttggatcaaagtactttgatcccgaggggaaccctgtggttggcatgcacatacaaatggacgaacggataaaccttttcacgcccttttaaatatccgttattctaataaacgctcttttctcttaggtttacccgccaatatatcctgtcaaacactgatagtttaaactgaaggcgggaaacgacaatctgatccaagctcaagctaagcttgagctctcccatatggtcgagatctcctttgccccggagatcaccatggacgactttctctatctctacgatctaggaagaaagttcgacggagaaggtgacgataccatgttcaccaccgataatgagaagattagcctcttcaatttcagaaagaatgctgacccacagatggttagagaggcctacgcggcaggtctcatcaagacgatctacccgagtaataatctccaggagatcaaataccttcccaagaaggttaaagatgcagtcaaaagattcaggactaactgcatcaagaacacagagaaagatatatttctcaagatcagaagtactattccagtatggacgattcaaggcttgcttcataaaccaaggcaagtaatagagattggagtctctaagaaagtagttcctactgaatcaaaggccatggagtcaaaaattcagatcgaggatctaacagaactcgccgtgaagactggcgaacagttcatacagagtcttttacgactcaatgacaagaagaaaatcttcgtcaacatggtggagcacgacactctcgtctactccaagaatatcaaagatacagtctcagaagaccaaagggctattgagacttttcaacaaagggtaatatcgggaaacctcctcggattccattgcccagctatctgtcacttcatcaaaaggacagtagaaaaggaaggtggcacctacaaatgccatcattgcgataaaggaaaggctatcgttcaagatgcccctgccgacagtggtcccaaagatggacccccacccacgaggagcatcgtggaaaaagaagacgttccaaccacgtcttcaaagcaagtggattgatgtgatatctccactgacgtaagggatgacgcacaatcccactatccttcgcaagacccttcctctatataaggaagttcatttcatttggagaggactccggtatttttacaacaattaccacaacaaaacaaacaacaaacaacattacaatttactattctagtcgacctgcaggcggccgcactagtgatatcacaagtttgtacaaaaaagcaggctgaattcccaccatggcaaacaagcttttcttggtgtgcgctaccttcgctctttgcttccttttgactaacgctcaggttcagctgcaggaatctggtggtggacttgttcaagctggtggatctcttagactctcttgcgctgcttctggaaggaccttctctagatatggaatgggatggttcaggcagctccctggaaaacagagagagcttgttacctctatcaccaggggtggaactaccacctacgctgattctgtgaagggaaggttcaccatctctagggataacgctaagaacaccgtgtacctccagatgaactctctcaagcctgaggataccgctgtgtactactgcaacgctagatctatttggagggattactggggacagggaactcaggtcaccgtttcttcacctagaatccctaagccttctacccctcctggatcttcttgtcctcctggaaatatcctcggtggaccttctgtgttcatcttcccacctaagcctaaggatgctctcatgatctcactcacccctaaggttacatgcgttgtggtggatgtgtctgaggatgatcctgatgtgcacgtgtcatggttcgtggataacaaagaggtgcacactgcttggactcagcctagagaagctcagtacaactctaccttcagggtggtgtctgctctccctatccaacaccaagattggatgaggggtaaagagttcaagtgcaaggtgaacaacaaggctctccctgctcctatcgagaggactatctctaaacctaagggaagggctcagacccctcaagtgtatacaattcctccacctagggaacagatgtctaagaagaaggtttcactcacttgcctcgtgaccaacttcttcagtgaggctatctctgttgagtgggagaggaatggtgagcttgagcaggattacaagaacacccctcctatcctcgattctgatggaacctacttcctctactctaagctcaccgtggataccgattcttggttgcagggtgagatcttcacttgctctgttgtgcatgaggctctccacaaccatcacacccagaagaacctcagtagatctcctggtaaagcggccgcacatcatcatcaccatcattgaggatccacccagctttcttgtacaaagtggtgatatcccgcggccatgctagagtccgcaaaaatcaccagtctctctctacaaatctatctctctctatttttctccagaataatgtgtgagtagttcccagataagggaattagggttcttatagggtttcgctcatgtgttgagcatataagaaacccttagtatgtatttgtatttgtaaaatacttctatcaataaaatttctaattcctaaaaccaaaatccagtgacctgcaggcatgcgacgtcg

SEQ ID NO: 361 - DNA, 10317 bp, Artificial Sequence
  pK7WG2-35S: sec_41D01-9GS-41D01_His
ggccctctagaggatccccgggtaccgcgaattatcatacatgagaattaagggagtcacgttatgacccccgccgatgacgcgggacaagccgttttacgtttggaactgacagaaccgcaacgttgaaggagccactcagccgcgggtttctggagtttaatgagctaagcacatacgtcagaaaccattattgcgcgttcaaaagtcgcctaaggtcactatcagctagcaaatatttcttgtcaaaaatgctccactgacgttccataaattcccctcggtatccaattagagtctcatattcactctcaactcgatcgaggcatgattgaacaagatggattgcacgcaggttctccggccgcttgggtggagaggctattcggctatgactgggcacaacagacaatcggctgctctgatgccgccgtgttccggctgtcagcgcaggggcgcccggttctttttgtcaagaccgacctgtccggtgccctgaatgaactccaagacgaggcagcgcggctatcgtggctggccacgacgggcgttccttgcgcagctgtgctcgacgttgtcactgaagcgggaagggactggctgctattgggcgaagtgccggggcaggatctcctgtcatctcaccttgctcctgccgagaaagtatccatcatggctgatgcaatgcggcggctgcatacgcttgatccggctacctgcccattcgaccaccaagcgaaacatcgcatcgagcgaggacgtactcggatggaagccggtcttgtcgatcaggatgatctggacgaagagcatcaggggctcgcgccagccgaactgttcgccaggctcaaggcgcggatgcccgacggcgaggatctcgtcgtgacccagggcgatgcctgcttgccgaatatcatggtggaaaatggccgcttttctggattcatcgactgtggccggctgggtgtggcggaccgctatcaggacatagcgttggctacccgtgatattgctgaagagcttggcggcgaatgggctgaccgcttcctcgtgctttacggtatcgccgctcccgattcgcagcgcatcgccttctatcgccttcttgacgagttcttctgagcgggactctggggttcggactctagctagagtcaagcagatcgttcaaacatttggcaataaagtttcttaagattgaatcctgttgccggtcttgcgatgattatcatataatttctgttgaattacgttaagcatgtaataattaacatgtaatgcatgacgttatttatgagatgggttttttgattagagtcccgcaattatacatttaatacgcgatagaaaacaaaatatagcgcgcaaactaggataaattatcgcgcgcggtgtcatctatgttactagatcgaccggcatgcaagctgataattcaattcggcgttaattcagtacattaaaaacgtccgcaatgtgttattaagttgtctaagcgtcaatttgtttacaccacaatatatcctgccaccagccagccaacagctccccgaccggcagctcggcacaaaatcaccactcgatacaggcagcccatcagtccgggacggcgtcagcgggagagccgttgtaaggcggcagactttgctcatgttaccgatgctattcggaagaacggcaactaagctgccgggtttgaaacacggatgatctcgcggagggtagcatgttgattgtaacgatgacagagcgttgctgcctgtgatcaattcgggcacgaacccagtggacataagcctcgttcggttcgtaagctgtaatgcaagtagcgtaactgccgtcacgcaactggtccagaaccttgaccgaacgcagcggtggtaacggcgcagtggcggttttcatggcttcttgttatgacatgtttttttggggtacagtctatgcctcgggcatccaagcagcaagcgcgttacgccgtgggtcgatgtttgatgttatggagcagcaacgatgttacgcagcagggcagtcgccctaaaacaaagttaaacatcatgggggaagcggtgatcgccgaagtatcgactcaactatcagaggtagttggcgtcatcgagcgccatctcgaaccgacgttgctggccgtacatttgtacggctccgcagtggatggcggcctgaagccacacagtgatattgatttgctggttacggtgaccgtaaggcttgatgaaacaacgcggcgagctttgatcaacgaccttttggaaacttcggcttcccctggagagagcgagattctccgcgctgtagaagtcaccattgttgtgcacgacgacatcattccgtggcgttatccagctaagcgcgaactgcaatttggagaatggcagcgcaatgacattcttgcaggtatcttcgagccagccacgatcgacattgatctggctatcttgctgacaaaagcaagagaacatagcgttgccttggtaggtccagcggcggaggaactctttgatccggttcctgaacaggatctatttgaggcgctaaatgaaaccttaacgctatggaactcgccgcccgactgggctggcgatgagcgaaatgtagtgcttacgttgtcccgcatttggtacagcgcagtaaccggcaaaatcgcgccgaaggatgtcgctgccgactgggcaatggagcgcctgccggcccagtatcagcccgtcatacttgaagctagacaggcttatcttggacaagaagaagatcgcttggcctcgcgcgcagatcagttggaagaatttgtccactacgtgaaaggcgagatcaccaaggtagtcggcaaataatgtctagctagaaattcgttcaagccgacgccgcttcgccggcgttaactcaagcgattagatgcactaagcacataattgctcacagccaaactatcaggtcaagtctgcttttattatttttaagcgtgcataataagccctacacaaattgggagatatatcatgcatgaccaaaatcccttaacgtgagttttcgttccactgagcgtcagaccccgtagaaaagatcaaaggatcttcttgagatcctttttttctgcgcgtaatctgctgcttgcaaacaaaaaaaccaccgctaccagcggtggtttgtttgccggatcaagagctaccaactctttttccgaaggtaactggcttcagcagagcgcagataccaaatactgtccttctagtgtagccgtagttaggccaccacttcaagaactctgtagcaccgcctacatacctcgctctgctaatcctgttaccagtggctgctgccagtggcgataagtcgtgtcttaccgggttggactcaagacgatagttaccggataaggcgcagcggtcgggctgaacggggggttcgtgcacacagcccagcttggagcgaacgacctacaccgaactgagatacctacagcgtgagctatgagaaagcgccacgcttcccgaagggagaaaggcggacaggtatccggtaagcggcagggtcggaacaggagagcgcacgagggagcttccagggggaaacgcctggtatctttatagtcctgtcgggtttcgccacctctgacttgagcgtcgatttttgtgatgctcgtcaggggggcggagcctatggaaaaacgccagcaacgcggcctttttacggttcctggccttttgctggccttttgctcacatgttctttcctgcgttatcccctgattctgtggataaccgtattaccgcctttgagtgagctgataccgctcgccgcagccgaacgaccgagcgcagcgagtcagtgagcgaggaagcggaagagcgcctgatgcggtattttctccttacgcatctgtgcggtatttcacaccgcatatggtgcactctcagtacaatctgctctgatgccgcatagttaagccagtatacactccgctatcgctacgtgactgggtcatggctgcgccccgacacccgccaacacccgctgacgcgccctgacgggcttgtctgctcccggcatccgcttacagacaagctgtgaccgtctccgggagctgcatgtgtcagaggttttcaccgtcatcaccgaaacgcgcgaggcagggtgccttgatgtgggcgccggcggtcgagtggcgacggcgcggcttgtccgcgccctggtagattgcctggccgtaggccagccatttttgagcggccagcggccgcgataggccgacgcgaagcggcggggcgtagggagcgcagcgaccgaagggtaggcgctttttgcagctcttcggctgtgcgctggccagacagttatgcacaggccaggcgggttttaagagttttaataagttttaaagagttttaggcggaaaaatcgccttttttctcttttatatcagtcacttacatgtgtgaccggttcccaatgtacggctttgggttcccaatgtacgggttccggttcccaatgtacggctttgggttcccaatgtacgtgctatccacaggaaagagaccttttcgacctttttcccctgctagggcaatttgccctagcatctgctccgtacattaggaaccggcggatgcttcgccctcgatcaggttgcggtagcgcatgactaggatcgggccagcctgccccgcctcctccttcaaatcgtactccggcaggtcatttgacccgatcagcttgcgcacggtgaaacagaacttcttgaactctccggcgctgccactgcgttcgtagatcgtcttgaacaaccatctggcttctgccttgcctgcggcgcggcgtgccaggcggtagagaaaacggccgatgccgggatcgatcaaaaagtaatcggggtgaaccgtcagcacgtccgggttcttgccttctgtgatctcgcggtacatccaatcagctagctcgatctcgatgtactccggccgcccggtttcgctctttacgatcttgtagcggctaatcaaggcttcaccctcggataccgtcaccaggcggccgttcttggccttcttcgtacgctgcatggcaacgtgcgtggtgtttaaccgaatgcaggtttctaccaggtcgtctttctgctttccgccatcggctcgccggcagaacttgagtacgtccgcaacgtgtggacggaacacgcggccgggcttgtctcccttcccttcccggtatcggttcatggattcggttagatgggaaaccgccatcagtaccaggtcgtaatcccacacactggccatgccggccggccctgcggaaacctctacgtgcccgtctggaagctcgtagcggatcacctcgccagctcgtcggtcacgcttcgacagacggaaaacggccacgtccatgatgctgcgactatcgcgggtgcccacgtcatagagcatcggaacgaaaaaatctggttgctcgtcgcccttgggcggcttcctaatcgacggcgcaccggctgccggcggttgccgggattctttgcggattcgatcagcggccgcttgccacgattcaccggggcgtgcttctgcctcgatgcgttgccgctgggcggcctgcgcggccttcaacttctccaccaggtcatcacccagcgccgcgccgatttgtaccgggccggatggtttgcgaccgtcacgccgattcctcgggcttgggggttccagtgccattgcagggccggcagacaacccagccgcttacgcctggccaaccgcccgttcctccacacatggggcattccacggcgtcggtgcctggttgttcttgattttccatgccgcctcctttagccgctaaaattcatctactcatttattcatttgctcatttactctggtagctgcgcgatgtattcagatagcagctcggtaatggtcttgccttggcgtaccgcgtacatcttcagcttggtgtgatcctccgccggcaactgaaagttgacccgcttcatggctggcgtgtctgccaggctggccaacgttgcagccttgctgctgcgtgcgctcggacggccggcacttagcgtgtttgtgcttttgctcattttctctttacctcattaactcaaatgagttttgatttaatttcagcggccagcgcctggacctcgcgggcagcgtcgccctcgggttctgattcaagaacggttgtgccggcggcggcagtgcctgggtagctcacgcgctgcgtgatacgggactcaagaatgggcagctcgtacccggccagcgcctcggcaacctcaccgccgatgcgcgtgcctttgatcgcccgcgacacgacaaaggccgcttgtagccttccatccgtgacctcaatgcgctgcttaaccagctccaccaggtcggcggtggcccatatgtcgtaagggcttggctgcaccggaatcagcacgaagtcggctgccttgatcgcggacacagccaagtccgccgcctggggcgctccgtcgatcactacgaagtcgcgccggccgatggccttcacgtcgcggtcaatcgtcgggcggtcgatgccgacaacggttagcggttgatcttcccgcacggccgcccaatcgcgggcactgccctggggatcggaatcgactaacagaacatcggccccggcgagttgcagggcgcgggctagatgggttgcgatggtcgtcttgcctgacccgcctttctggttaagtacagcgataaccttcatgcgttccccttgcgtatttgtttatttactcatcgcatcatatacgcagcgaccgcatgacgcaagctgttttactcaaatacacatcacctttttagacggcggcgctcggtttcttcagcggccaagctggccggccaggccgccagcttggcatcagacaaaccggccaggatttcatgcagccgcacggttgagacgtgcgcgggcggctcgaacacgtacccggccgcgatcatctccgcctcgatctcttcggtaatgaaaaacggttcgtcctggccgtcctggtgcggtttcatgcttgttcctcttggcgttcattctcggcggccgccagggcgtcggcctcggtcaatgcgtcctcacggaaggcaccgcgccgcctggcctcggtgggcgtcacttcctcgctgcgctcaagtgcgcggtacagggtcgagcgatgcacgccaagcagtgcagccgcctctttcacggtgcggccttcctggtcgatcagctcgcgggcgtgcgcgatctgtgccggggtgagggtagggcgggggccaaacttcacgcctcgggccttggcggcctcgcgcccgctccgggtgcggtcgatgattagggaacgctcgaactcggcaatgccggcgaacacggtcaacaccatgcggccggccggcgtggtggtgtcggcccacggctctgccaggctacgcaggcccgcgccggcctcctggatgcgctcggcaatgtccagtaggtcgcgggtgctgcgggccaggcggtctagcctggtcactgtcacaacgtcgccagggcgtaggtggtcaagcatcctggccagctccgggcggtcgcgcctggtgccggtgatcttctcggaaaacagcttggtgcagccggccgcgtgcagttcggcccgttggttggtcaagtcctggtcgtcggtgctgacgcgggcatagcccagcaggccagcggcggcgctcttgttcatggcgtaatgtctccggttctagtcgcaagtattctactttatgcgactaaaacacgcgacaagaaaacgccaggaaaagggcagggcggcagcctgtcgcgtaacttaggacttgtgcgacatgtcgttttcagaagacggctgcactgaacgtcagaagccgactgcactatagcagcggaggggttggatcaaagtactttgatcccgaggggaaccctgtggttggcatgcacatacaaatggacgaacggataaaccttttcacgcccttttaaatatccgttattctaataaacgctcttttctcttaggtttacccgccaatatatcctgtcaaacactgatagtttaaactgaaggcgggaaacgacaatctgatccaagctcaagctaagcttgagctctcccatatggtcgagatctcctttgccccggagatcaccatggacgactttctctatctctacgatctaggaagaaagttcgacggagaaggtgacgataccatgttcaccaccgataatgagaagattagcctcttcaatttcagaaagaatgctgacccacagatggttagagaggcctacgcggcaggtctcatcaagacgatctacccgagtaataatctccaggagatcaaataccttcccaagaaggttaaagatgcagtcaaaagattcaggactaactgcatcaagaacacagagaaagatatatttctcaagatcagaagtactattccagtatggacgattcaaggcttgcttcataaaccaaggcaagtaatagagattggagtctctaagaaagtagttcctactgaatcaaaggccatggagtcaaaaattcagatcgaggatctaacagaactcgccgtgaagactggcgaacagttcatacagagtcttttacgactcaatgacaagaagaaaatcttcgtcaacatggtggagcacgacactctcgtctactccaagaatatcaaagatacagtctcagaagaccaaagggctattgagacttttcaacaaagggtaatatcgggaaacctcctcggattccattgcccagctatctgtcacttcatcaaaaggacagtagaaaaggaaggtggcacctacaaatgccatcattgcgataaaggaaaggctatcgttcaagatgcccctgccgacagtggtcccaaagatggacccccacccacgaggagcatcgtggaaaaagaagacgttccaaccacgtcttcaaagcaagtggattgatgtgatatctccactgacgtaagggatgacgcacaatcccactatccttcgcaagacccttcctctatataaggaagttcatttcatttggagaggactccggtatttttacaacaattaccacaacaaaacaaacaacaaacaacattacaatttactattctagtcgacctgcaggcggccgcactagtgatatcacaagtttgtacaaaaaagcaggctgaattcccaccatggcaaacaagcttttcttggtgtgcgctaccttcgctctttgcttccttttgactaacgctcaggttcaattgcaagagtctggtggtggacttgttcaggctggtggatctcttagactttcttgcgctgcttctggaaggaccttctctagatatggaatgggatggttcaggcagctccctggaaaacagagagagcttgttacctctatcaccaggggtggaactaccacctacgctgattctgtgaagggaaggttcaccatctctagggataacgctaagaacaccgtgtacctccagatgaactctctcaagcctgaggataccgctgtgtactactgcaacgctagatctatttggagggattactggggacagggaactcaggtcaccgtttcttcaggtggtggtggaagtggtggtggttctcaagttcaactgcaggaatcaggtggtggattggtgcaagctggtggttctttgaggttgtcatgtgctgctagtggtaggaccttcagtaggtacggtatgggatggtttagacagttgcctggtaagcagagggaactcgtgacttcaatcactagaggtggaaccactacttacgcagatagtgttaagggaagattcactatcagtagagataatgcaaagaacactgtttacttgcaaatgaactcattgaagccagaggatacagcagtttattactgtaacgcaagaagtatttggagagattattggggtcaaggtactcaagtgaccgttagttcagcggccgcacatcatcatcaccatcattgaggatccacccagctttcttgtacaaagtggtgatatcccgcggccatgctagagtccgcaaaaatcaccagtctctctctacaaatctatctctctctatttttctccagaataatgtgtgagtagttcccagataagggaattagggttcttatagggtttcgctcatgtgttgagcatataagaaacccttagtatgtatttgtatttgtaaaatacttctatcaataaaatttctaattcctaaaaccaaaatccagtgacctgcaggcatgcgacgtcg

SEQ ID NO: 362 - DNA, 9945 bp, Artificial Sequence
  pK7WG2-35S: sec_41D01_His
ggccctctagaggatccccgggtaccgcgaattatcatacatgagaattaagggagtcacgttatgacccccgccgatgacgcgggacaagccgttttacgtttggaactgacagaaccgcaacgttgaaggagccactcagccgcgggtttctggagtttaatgagctaagcacatacgtcagaaaccattattgcgcgttcaaaagtcgcctaaggtcactatcagctagcaaatatttcttgtcaaaaatgctccactgacgttccataaattcccctcggtatccaattagagtctcatattcactctcaactcgatcgaggcatgattgaacaagatggattgcacgcaggttctccggccgcttgggtggagaggctattcggctatgactgggcacaacagacaatcggctgctctgatgccgccgtgttccggctgtcagcgcaggggcgcccggttctttttgtcaagaccgacctgtccggtgccctgaatgaactccaagacgaggcagcgcggctatcgtggctggccacgacgggcgttccttgcgcagctgtgctcgacgttgtcactgaagcgggaagggactggctgctattgggcgaagtgccggggcaggatctcctgtcatctcaccttgctcctgccgagaaagtatccatcatggctgatgcaatgcggcggctgcatacgcttgatccggctacctgcccattcgaccaccaagcgaaacatcgcatcgagcgaggacgtactcggatggaagccggtcttgtcgatcaggatgatctggacgaagagcatcaggggctcgcgccagccgaactgttcgccaggctcaaggcgcggatgcccgacggcgaggatctcgtcgtgacccagggcgatgcctgcttgccgaatatcatggtggaaaatggccgcttttctggattcatcgactgtggccggctgggtgtggcggaccgctatcaggacatagcgttggctacccgtgatattgctgaagagcttggcggcgaatgggctgaccgcttcctcgtgctttacggtatcgccgctcccgattcgcagcgcatcgccttctatcgccttcttgacgagttcttctgagcgggactctggggttcggactctagctagagtcaagcagatcgttcaaacatttggcaataaagtttcttaagattgaatcctgttgccggtcttgcgatgattatcatataatttctgttgaattacgttaagcatgtaataattaacatgtaatgcatgacgttatttatgagatgggttttttgattagagtcccgcaattatacatttaatacgcgatagaaaacaaaatatagcgcgcaaactaggataaattatcgcgcgcggtgtcatctatgttactagatcgaccggcatgcaagctgataattcaattcggcgttaattcagtacattaaaaacgtccgcaatgtgttattaagttgtctaagcgtcaatttgtttacaccacaatatatcctgccaccagccagccaacagctccccgaccggcagctcggcacaaaatcaccactcgatacaggcagcccatcagtccgggacggcgtcagcgggagagccgttgtaaggcggcagactttgctcatgttaccgatgctattcggaagaacggcaactaagctgccgggtttgaaacacggatgatctcgcggagggtagcatgttgattgtaacgatgacagagcgttgctgcctgtgatcaattcgggcacgaacccagtggacataagcctcgttcggttcgtaagctgtaatgcaagtagcgtaactgccgtcacgcaactggtccagaaccttgaccgaacgcagcggtggtaacggcgcagtggcggttttcatggcttcttgttatgacatgtttttttggggtacagtctatgcctcgggcatccaagcagcaagcgcgttacgccgtgggtcgatgtttgatgttatggagcagcaacgatgttacgcagcagggcagtcgccctaaaacaaagttaaacatcatgggggaagcggtgatcgccgaagtatcgactcaactatcagaggtagttggcgtcatcgagcgccatctcgaaccgacgttgctggccgtacatttgtacggctccgcagtggatggcggcctgaagccacacagtgatattgatttgctggttacggtgaccgtaaggcttgatgaaacaacgcggcgagctttgatcaacgaccttttggaaacttcggcttcccctggagagagcgagattctccgcgctgtagaagtcaccattgttgtgcacgacgacatcattccgtggcgttatccagctaagcgcgaactgcaatttggagaatggcagcgcaatgacattcttgcaggtatcttcgagccagccacgatcgacattgatctggctatcttgctgacaaaagcaagagaacatagcgttgccttggtaggtccagcggcggaggaactctttgatccggttcctgaacaggatctatttgaggcgctaaatgaaaccttaacgctatggaactcgccgcccgactgggctggcgatgagcgaaatgtagtgcttacgttgtcccgcatttggtacagcgcagtaaccggcaaaatcgcgccgaaggatgtcgctgccgactgggcaatggagcgcctgccggcccagtatcagcccgtcatacttgaagctagacaggcttatcttggacaagaagaagatcgcttggcctcgcgcgcagatcagttggaagaatttgtccactacgtgaaaggcgagatcaccaaggtagtcggcaaataatgtctagctagaaattcgttcaagccgacgccgcttcgccggcgttaactcaagcgattagatgcactaagcacataattgctcacagccaaactatcaggtcaagtctgcttttattatttttaagcgtgcataataagccctacacaaattgggagatatatcatgcatgaccaaaatcccttaacgtgagttttcgttccactgagcgtcagaccccgtagaaaagatcaaaggatcttcttgagatcctttttttctgcgcgtaatctgctgcttgcaaacaaaaaaaccaccgctaccagcggtggtttgtttgccggatcaagagctaccaactctttttccgaaggtaactggcttcagcagagcgcagataccaaatactgtccttctagtgtagccgtagttaggccaccacttcaagaactctgtagcaccgcctacatacctcgctctgctaatcctgttaccagtggctgctgccagtggcgataagtcgtgtcttaccgggttggactcaagacgatagttaccggataaggcgcagcggtcgggctgaacggggggttcgtgcacacagcccagcttggagcgaacgacctacaccgaactgagatacctacagcgtgagctatgagaaagcgccacgcttcccgaagggagaaaggcggacaggtatccggtaagcggcagggtcggaacaggagagcgcacgagggagcttccagggggaaacgcctggtatctttatagtcctgtcgggtttcgccacctctgacttgagcgtcgatttttgtgatgctcgtcaggggggcggagcctatggaaaaacgccagcaacgcggcctttttacggttcctggccttttgctggccttttgctcacatgttctttcctgcgttatcccctgattctgtggataaccgtattaccgcctttgagtgagctgataccgctcgccgcagccgaacgaccgagcgcagcgagtcagtgagcgaggaagcggaagagcgcctgatgcggtattttctccttacgcatctgtgcggtatttcacaccgcatatggtgcactctcagtacaatctgctctgatgccgcatagttaagccagtatacactccgctatcgctacgtgactgggtcatggctgcgccccgacacccgccaacacccgctgacgcgccctgacgggcttgtctgctcccggcatccgcttacagacaagctgtgaccgtctccgggagctgcatgtgtcagaggttttcaccgtcatcaccgaaacgcgcgaggcagggtgccttgatgtgggcgccggcggtcgagtggcgacggcgcggcttgtccgcgccctggtagattgcctggccgtaggccagccatttttgagcggccagcggccgcgataggccgacgcgaagcggcggggcgtagggagcgcagcgaccgaagggtaggcgctttttgcagctcttcggctgtgcgctggccagacagttatgcacaggccaggcgggttttaagagttttaataagttttaaagagttttaggcggaaaaatcgccttttttctcttttatatcagtcacttacatgtgtgaccggttcccaatgtacggctttgggttcccaatgtacgggttccggttcccaatgtacggctttgggttcccaatgtacgtgctatccacaggaaagagaccttttcgacctttttcccctgctagggcaatttgccctagcatctgctccgtacattaggaaccggcggatgcttcgccctcgatcaggttgcggtagcgcatgactaggatcgggccagcctgccccgcctcctccttcaaatcgtactccggcaggtcatttgacccgatcagcttgcgcacggtgaaacagaacttcttgaactctccggcgctgccactgcgttcgtagatcgtcttgaacaaccatctggcttctgccttgcctgcggcgcggcgtgccaggcggtagagaaaacggccgatgccgggatcgatcaaaaagtaatcggggtgaaccgtcagcacgtccgggttcttgccttctgtgatctcgcggtacatccaatcagctagctcgatctcgatgtactccggccgcccggtttcgctctttacgatcttgtagcggctaatcaaggcttcaccctcggataccgtcaccaggcggccgttcttggccttcttcgtacgctgcatggcaacgtgcgtggtgtttaaccgaatgcaggtttctaccaggtcgtctttctgctttccgccatcggctcgccggcagaacttgagtacgtccgcaacgtgtggacggaacacgcggccgggcttgtctcccttcccttcccggtatcggttcatggattcggttagatgggaaaccgccatcagtaccaggtcgtaatcccacacactggccatgccggccggccctgcggaaacctctacgtgcccgtctggaagctcgtagcggatcacctcgccagctcgtcggtcacgcttcgacagacggaaaacggccacgtccatgatgctgcgactatcgcgggtgcccacgtcatagagcatcggaacgaaaaaatctggttgctcgtcgcccttgggcggcttcctaatcgacggcgcaccggctgccggcggttgccgggattctttgcggattcgatcagcggccgcttgccacgattcaccggggcgtgcttctgcctcgatgcgttgccgctgggcggcctgcgcggccttcaacttctccaccaggtcatcacccagcgccgcgccgatttgtaccgggccggatggtttgcgaccgtcacgccgattcctcgggcttgggggttccagtgccattgcagggccggcagacaacccagccgcttacgcctggccaaccgcccgttcctccacacatggggcattccacggcgtcggtgcctggttgttcttgattttccatgccgcctcctttagccgctaaaattcatctactcatttattcatttgctcatttactctggtagctgcgcgatgtattcagatagcagctcggtaatggtcttgccttggcgtaccgcgtacatcttcagcttggtgtgatcctccgccggcaactgaaagttgacccgcttcatggctggcgtgtctgccaggctggccaacgttgcagccttgctgctgcgtgcgctcggacggccggcacttagcgtgtttgtgcttttgctcattttctctttacctcattaactcaaatgagttttgatttaatttcagcggccagcgcctggacctcgcgggcagcgtcgccctcgggttctgattcaagaacggttgtgccggcggcggcagtgcctgggtagctcacgcgctgcgtgatacgggactcaagaatgggcagctcgtacccggccagcgcctcggcaacctcaccgccgatgcgcgtgcctttgatcgcccgcgacacgacaaaggccgcttgtagccttccatccgtgacctcaatgcgctgcttaaccagctccaccaggtcggcggtggcccatatgtcgtaagggcttggctgcaccggaatcagcacgaagtcggctgccttgatcgcggacacagccaagtccgccgcctggggcgctccgtcgatcactacgaagtcgcgccggccgatggccttcacgtcgcggtcaatcgtcgggcggtcgatgccgacaacggttagcggttgatcttcccgcacggccgcccaatcgcgggcactgccctggggatcggaatcgactaacagaacatcggccccggcgagttgcagggcgcgggctagatgggttgcgatggtcgtcttgcctgacccgcctttctggttaagtacagcgataaccttcatgcgttccccttgcgtatttgtttatttactcatcgcatcatatacgcagcgaccgcatgacgcaagctgttttactcaaatacacatcacctttttagacggcggcgctcggtttcttcagcggccaagctggccggccaggccgccagcttggcatcagacaaaccggccaggatttcatgcagccgcacggttgagacgtgcgcgggcggctcgaacacgtacccggccgcgatcatctccgcctcgatctcttcggtaatgaaaaacggttcgtcctggccgtcctggtgcggtttcatgcttgttcctcttggcgttcattctcggcggccgccagggcgtcggcctcggtcaatgcgtcctcacggaaggcaccgcgccgcctggcctcggtgggcgtcacttcctcgctgcgctcaagtgcgcggtacagggtcgagcgatgcacgccaagcagtgcagccgcctctttcacggtgcggccttcctggtcgatcagctcgcgggcgtgcgcgatctgtgccggggtgagggtagggcgggggccaaacttcacgcctcgggccttggcggcctcgcgcccgctccgggtgcggtcgatgattagggaacgctcgaactcggcaatgccggcgaacacggtcaacaccatgcggccggccggcgtggtggtgtcggcccacggctctgccaggctacgcaggcccgcgccggcctcctggatgcgctcggcaatgtccagtaggtcgcgggtgctgcgggccaggcggtctagcctggtcactgtcacaacgtcgccagggcgtaggtggtcaagcatcctggccagctccgggcggtcgcgcctggtgccggtgatcttctcggaaaacagcttggtgcagccggccgcgtgcagttcggcccgttggttggtcaagtcctggtcgtcggtgctgacgcgggcatagcccagcaggccagcggcggcgctcttgttcatggcgtaatgtctccggttctagtcgcaagtattctactttatgcgactaaaacacgcgacaagaaaacgccaggaaaagggcagggcggcagcctgtcgcgtaacttaggacttgtgcgacatgtcgttttcagaagacggctgcactgaacgtcagaagccgactgcactatagcagcggaggggttggatcaaagtactttgatcccgaggggaaccctgtggttggcatgcacatacaaatggacgaacggataaaccttttcacgcccttttaaatatccgttattctaataaacgctcttttctcttaggtttacccgccaatatatcctgtcaaacactgatagtttaaactgaaggcgggaaacgacaatctgatccaagctcaagctaagcttgagctctcccatatggtcgagatctcctttgccccggagatcaccatggacgactttctctatctctacgatctaggaagaaagttcgacggagaaggtgacgataccatgttcaccaccgataatgagaagattagcctcttcaatttcagaaagaatgctgacccacagatggttagagaggcctacgcggcaggtctcatcaagacgatctacccgagtaataatctccaggagatcaaataccttcccaagaaggttaaagatgcagtcaaaagattcaggactaactgcatcaagaacacagagaaagatatatttctcaagatcagaagtactattccagtatggacgattcaaggcttgcttcataaaccaaggcaagtaatagagattggagtctctaagaaagtagttcctactgaatcaaaggccatggagtcaaaaattcagatcgaggatctaacagaactcgccgtgaagactggcgaacagttcatacagagtcttttacgactcaatgacaagaagaaaatcttcgtcaacatggtggagcacgacactctcgtctactccaagaatatcaaagatacagtctcagaagaccaaagggctattgagacttttcaacaaagggtaatatcgggaaacctcctcggattccattgcccagctatctgtcacttcatcaaaaggacagtagaaaaggaaggtggcacctacaaatgccatcattgcgataaaggaaaggctatcgttcaagatgcccctgccgacagtggtcccaaagatggacccccacccacgaggagcatcgtggaaaaagaagacgttccaaccacgtcttcaaagcaagtggattgatgtgatatctccactgacgtaagggatgacgcacaatcccactatccttcgcaagacccttcctctatataaggaagttcatttcatttggagaggactccggtatttttacaacaattaccacaacaaaacaaacaacaaacaacattacaatttactattctagtcgacctgcaggcggccgcactagtgatatcacaagtttgtacaaaaaagcaggctgaattcccaccatggcaaacaagcttttcttggtgtgcgctaccttcgctctttgcttccttttgactaacgctcaggttcagctgcaggaatctggtggtggacttgttcaagctggtggatctcttagactctcttgcgctgcttctggaaggaccttctctagatatggaatgggatggttcaggcagctccctggaaaacagagagagcttgttacctctatcaccaggggtggaactaccacctacgctgattctgtgaagggaaggttcaccatctctagggataacgctaagaacaccgtgtacctccagatgaactctctcaagcctgaggataccgctgtgtactactgcaacgctagatctatttggagggattactggggacagggaactcaggtcaccgtttcttcagcggccgcacatcatcatcaccatcattgaggatccacccagctttcttgtacaaagtggtgatatcccgcggccatgctagagtccgcaaaaatcaccagtctctctctacaaatctatctctctctatttttctccagaataatgtgtgagtagttcccagataagggaattagggttcttatagggtttcgctcatgtgttgagcatataagaaacccttagtatgtatttgtatttgtaaaatacttctatcaataaaatttctaattcctaaaaccaaaatccagtgacctgcaggcatgcgacgtcg

SEQ ID NO: 363 - DNA, 9885 bp, Artificial Sequence
  pK7WG2-35S: cyto_41D01_His
ggccctctagaggatccccgggtaccgcgaattatcatacatgagaattaagggagtcacgttatgacccccgccgatgacgcgggacaagccgttttacgtttggaactgacagaaccgcaacgttgaaggagccactcagccgcgggtttctggagtttaatgagctaagcacatacgtcagaaaccattattgcgcgttcaaaagtcgcctaaggtcactatcagctagcaaatatttcttgtcaaaaatgctccactgacgttccataaattcccctcggtatccaattagagtctcatattcactctcaactcgatcgaggcatgattgaacaagatggattgcacgcaggttctccggccgcttgggtggagaggctattcggctatgactgggcacaacagacaatcggctgctctgatgccgccgtgttccggctgtcagcgcaggggcgcccggttctttttgtcaagaccgacctgtccggtgccctgaatgaactccaagacgaggcagcgcggctatcgtggctggccacgacgggcgttccttgcgcagctgtgctcgacgttgtcactgaagcgggaagggactggctgctattgggcgaagtgccggggcaggatctcctgtcatctcaccttgctcctgccgagaaagtatccatcatggctgatgcaatgcggcggctgcatacgcttgatccggctacctgcccattcgaccaccaagcgaaacatcgcatcgagcgaggacgtactcggatggaagccggtcttgtcgatcaggatgatctggacgaagagcatcaggggctcgcgccagccgaactgttcgccaggctcaaggcgcggatgcccgacggcgaggatctcgtcgtgacccagggcgatgcctgcttgccgaatatcatggtggaaaatggccgcttttctggattcatcgactgtggccggctgggtgtggcggaccgctatcaggacatagcgttggctacccgtgatattgctgaagagcttggcggcgaatgggctgaccgcttcctcgtgctttacggtatcgccgctcccgattcgcagcgcatcgccttctatcgccttcttgacgagttcttctgagcgggactctggggttcggactctagctagagtcaagcagatcgttcaaacatttggcaataaagtttcttaagattgaatcctgttgccggtcttgcgatgattatcatataatttctgttgaattacgttaagcatgtaataattaacatgtaatgcatgacgttatttatgagatgggttttttgattagagtcccgcaattatacatttaatacgcgatagaaaacaaaatatagcgcgcaaactaggataaattatcgcgcgcggtgtcatctatgttactagatcgaccggcatgcaagctgataattcaattcggcgttaattcagtacattaaaaacgtccgcaatgtgttattaagttgtctaagcgtcaatttgtttacaccacaatatatcctgccaccagccagccaacagctccccgaccggcagctcggcacaaaatcaccactcgatacaggcagcccatcagtccgggacggcgtcagcgggagagccgttgtaaggcggcagactttgctcatgttaccgatgctattcggaagaacggcaactaagctgccgggtttgaaacacggatgatctcgcggagggtagcatgttgattgtaacgatgacagagcgttgctgcctgtgatcaattcgggcacgaacccagtggacataagcctcgttcggttcgtaagctgtaatgcaagtagcgtaactgccgtcacgcaactggtccagaaccttgaccgaacgcagcggtggtaacggcgcagtggcggttttcatggcttcttgttatgacatgtttttttggggtacagtctatgcctcgggcatccaagcagcaagcgcgttacgccgtgggtcgatgtttgatgttatggagcagcaacgatgttacgcagcagggcagtcgccctaaaacaaagttaaacatcatgggggaagcggtgatcgccgaagtatcgactcaactatcagaggtagttggcgtcatcgagcgccatctcgaaccgacgttgctggccgtacatttgtacggctccgcagtggatggcggcctgaagccacacagtgatattgatttgctggttacggtgaccgtaaggcttgatgaaacaacgcggcgagctttgatcaacgaccttttggaaacttcggcttcccctggagagagcgagattctccgcgctgtagaagtcaccattgttgtgcacgacgacatcattccgtggcgttatccagctaagcgcgaactgcaatttggagaatggcagcgcaatgacattcttgcaggtatcttcgagccagccacgatcgacattgatctggctatcttgctgacaaaagcaagagaacatagcgttgccttggtaggtccagcggcggaggaactctttgatccggttcctgaacaggatctatttgaggcgctaaatgaaaccttaacgctatggaactcgccgcccgactgggctggcgatgagcgaaatgtagtgcttacgttgtcccgcatttggtacagcgcagtaaccggcaaaatcgcgccgaaggatgtcgctgccgactgggcaatggagcgcctgccggcccagtatcagcccgtcatacttgaagctagacaggcttatcttggacaagaagaagatcgcttggcctcgcgcgcagatcagttggaagaatttgtccactacgtgaaaggcgagatcaccaaggtagtcggcaaataatgtctagctagaaattcgttcaagccgacgccgcttcgccggcgttaactcaagcgattagatgcactaagcacataattgctcacagccaaactatcaggtcaagtctgcttttattatttttaagcgtgcataataagccctacacaaattgggagatatatcatgcatgaccaaaatcccttaacgtgagttttcgttccactgagcgtcagaccccgtagaaaagatcaaaggatcttcttgagatcctttttttctgcgcgtaatctgctgcttgcaaacaaaaaaaccaccgctaccagcggtggtttgtttgccggatcaagagctaccaactctttttccgaaggtaactggcttcagcagagcgcagataccaaatactgtccttctagtgtagccgtagttaggccaccacttcaagaactctgtagcaccgcctacatacctcgctctgctaatcctgttaccagtggctgctgccagtggcgataagtcgtgtcttaccgggttggactcaagacgatagttaccggataaggcgcagcggtcgggctgaacggggggttcgtgcacacagcccagcttggagcgaacgacctacaccgaactgagatacctacagcgtgagctatgagaaagcgccacgcttcccgaagggagaaaggcggacaggtatccggtaagcggcagggtcggaacaggagagcgcacgagggagcttccagggggaaacgcctggtatctttatagtcctgtcgggtttcgccacctctgacttgagcgtcgatttttgtgatgctcgtcaggggggcggagcctatggaaaaacgccagcaacgcggcctttttacggttcctggccttttgctggccttttgctcacatgttctttcctgcgttatcccctgattctgtggataaccgtattaccgcctttgagtgagctgataccgctcgccgcagccgaacgaccgagcgcagcgagtcagtgagcgaggaagcggaagagcgcctgatgcggtattttctccttacgcatctgtgcggtatttcacaccgcatatggtgcactctcagtacaatctgctctgatgccgcatagttaagccagtatacactccgctatcgctacgtgactgggtcatggctgcgccccgacacccgccaacacccgctgacgcgccctgacgggcttgtctgctcccggcatccgcttacagacaagctgtgaccgtctccgggagctgcatgtgtcagaggttttcaccgtcatcaccgaaacgcgcgaggcagggtgccttgatgtgggcgccggcggtcgagtggcgacggcgcggcttgtccgcgccctggtagattgcctggccgtaggccagccatttttgagcggccagcggccgcgataggccgacgcgaagcggcggggcgtagggagcgcagcgaccgaagggtaggcgctttttgcagctcttcggctgtgcgctggccagacagttatgcacaggccaggcgggttttaagagttttaataagttttaaagagttttaggcggaaaaatcgccttttttctcttttatatcagtcacttacatgtgtgaccggttcccaatgtacggctttgggttcccaatgtacgggttccggttcccaatgtacggctttgggttcccaatgtacgtgctatccacaggaaagagaccttttcgacctttttcccctgctagggcaatttgccctagcatctgctccgtacattaggaaccggcggatgcttcgccctcgatcaggttgcggtagcgcatgactaggatcgggccagcctgccccgcctcctccttcaaatcgtactccggcaggtcatttgacccgatcagcttgcgcacggtgaaacagaacttcttgaactctccggcgctgccactgcgttcgtagatcgtcttgaacaaccatctggcttctgccttgcctgcggcgcggcgtgccaggcggtagagaaaacggccgatgccgggatcgatcaaaaagtaatcggggtgaaccgtcagcacgtccgggttcttgccttctgtgatctcgcggtacatccaatcagctagctcgatctcgatgtactccggccgcccggtttcgctctttacgatcttgtagcggctaatcaaggcttcaccctcggataccgtcaccaggcggccgttcttggccttcttcgtacgctgcatggcaacgtgcgtggtgtttaaccgaatgcaggtttctaccaggtcgtctttctgctttccgccatcggctcgccggcagaacttgagtacgtccgcaacgtgtggacggaacacgcggccgggcttgtctcccttcccttcccggtatcggttcatggattcggttagatgggaaaccgccatcagtaccaggtcgtaatcccacacactggccatgccggccggccctgcggaaacctctacgtgcccgtctggaagctcgtagcggatcacctcgccagctcgtcggtcacgcttcgacagacggaaaacggccacgtccatgatgctgcgactatcgcgggtgcccacgtcatagagcatcggaacgaaaaaatctggttgctcgtcgcccttgggcggcttcctaatcgacggcgcaccggctgccggcggttgccgggattctttgcggattcgatcagcggccgcttgccacgattcaccggggcgtgcttctgcctcgatgcgttgccgctgggcggcctgcgcggccttcaacttctccaccaggtcatcacccagcgccgcgccgatttgtaccgggccggatggtttgcgaccgtcacgccgattcctcgggcttgggggttccagtgccattgcagggccggcagacaacccagccgcttacgcctggccaaccgcccgttcctccacacatggggcattccacggcgtcggtgcctggttgttcttgattttccatgccgcctcctttagccgctaaaattcatctactcatttattcatttgctcatttactctggtagctgcgcgatgtattcagatagcagctcggtaatggtcttgccttggcgtaccgcgtacatcttcagcttggtgtgatcctccgccggcaactgaaagttgacccgcttcatggctggcgtgtctgccaggctggccaacgttgcagccttgctgctgcgtgcgctcggacggccggcacttagcgtgtttgtgcttttgctcattttctctttacctcattaactcaaatgagttttgatttaatttcagcggccagcgcctggacctcgcgggcagcgtcgccctcgggttctgattcaagaacggttgtgccggcggcggcagtgcctgggtagctcacgcgctgcgtgatacgggactcaagaatgggcagctcgtacccggccagcgcctcggcaacctcaccgccgatgcgcgtgcctttgatcgcccgcgacacgacaaaggccgcttgtagccttccatccgtgacctcaatgcgctgcttaaccagctccaccaggtcggcggtggcccatatgtcgtaagggcttggctgcaccggaatcagcacgaagtcggctgccttgatcgcggacacagccaagtccgccgcctggggcgctccgtcgatcactacgaagtcgcgccggccgatggccttcacgtcgcggtcaatcgtcgggcggtcgatgccgacaacggttagcggttgatcttcccgcacggccgcccaatcgcgggcactgccctggggatcggaatcgactaacagaacatcggccccggcgagttgcagggcgcgggctagatgggttgcgatggtcgtcttgcctgacccgcctttctggttaagtacagcgataaccttcatgcgttccccttgcgtatttgtttatttactcatcgcatcatatacgcagcgaccgcatgacgcaagctgttttactcaaatacacatcacctttttagacggcggcgctcggtttcttcagcggccaagctggccggccaggccgccagcttggcatcagacaaaccggccaggatttcatgcagccgcacggttgagacgtgcgcgggcggctcgaacacgtacccggccgcgatcatctccgcctcgatctcttcggtaatgaaaaacggttcgtcctggccgtcctggtgcggtttcatgcttgttcctcttggcgttcattctcggcggccgccagggcgtcggcctcggtcaatgcgtcctcacggaaggcaccgcgccgcctggcctcggtgggcgtcacttcctcgctgcgctcaagtgcgcggtacagggtcgagcgatgcacgccaagcagtgcagccgcctctttcacggtgcggccttcctggtcgatcagctcgcgggcgtgcgcgatctgtgccggggtgagggtagggcgggggccaaacttcacgcctcgggccttggcggcctcgcgcccgctccgggtgcggtcgatgattagggaacgctcgaactcggcaatgccggcgaacacggtcaacaccatgcggccggccggcgtggtggtgtcggcccacggctctgccaggctacgcaggcccgcgccggcctcctggatgcgctcggcaatgtccagtaggtcgcgggtgctgcgggccaggcggtctagcctggtcactgtcacaacgtcgccagggcgtaggtggtcaagcatcctggccagctccgggcggtcgcgcctggtgccggtgatcttctcggaaaacagcttggtgcagccggccgcgtgcagttcggcccgttggttggtcaagtcctggtcgtcggtgctgacgcgggcatagcccagcaggccagcggcggcgctcttgttcatggcgtaatgtctccggttctagtcgcaagtattctactttatgcgactaaaacacgcgacaagaaaacgccaggaaaagggcagggcggcagcctgtcgcgtaacttaggacttgtgcgacatgtcgttttcagaagacggctgcactgaacgtcagaagccgactgcactatagcagcggaggggttggatcaaagtactttgatcccgaggggaaccctgtggttggcatgcacatacaaatggacgaacggataaaccttttcacgcccttttaaatatccgttattctaataaacgctcttttctcttaggtttacccgccaatatatcctgtcaaacactgatagtttaaactgaaggcgggaaacgacaatctgatccaagctcaagctaagcttgagctctcccatatggtcgagatctcctttgccccggagatcaccatggacgactttctctatctctacgatctaggaagaaagttcgacggagaaggtgacgataccatgttcaccaccgataatgagaagattagcctcttcaatttcagaaagaatgctgacccacagatggttagagaggcctacgcggcaggtctcatcaagacgatctacccgagtaataatctccaggagatcaaataccttcccaagaaggttaaagatgcagtcaaaagattcaggactaactgcatcaagaacacagagaaagatatatttctcaagatcagaagtactattccagtatggacgattcaaggcttgcttcataaaccaaggcaagtaatagagattggagtctctaagaaagtagttcctactgaatcaaaggccatggagtcaaaaattcagatcgaggatctaacagaactcgccgtgaagactggcgaacagttcatacagagtcttttacgactcaatgacaagaagaaaatcttcgtcaacatggtggagcacgacactctcgtctactccaagaatatcaaagatacagtctcagaagaccaaagggctattgagacttttcaacaaagggtaatatcgggaaacctcctcggattccattgcccagctatctgtcacttcatcaaaaggacagtagaaaaggaaggtggcacctacaaatgccatcattgcgataaaggaaaggctatcgttcaagatgcccctgccgacagtggtcccaaagatggacccccacccacgaggagcatcgtggaaaaagaagacgttccaaccacgtcttcaaagcaagtggattgatgtgatatctccactgacgtaagggatgacgcacaatcccactatccttcgcaagacccttcctctatataaggaagttcatttcatttggagaggactccggtatttttacaacaattaccacaacaaaacaaacaacaaacaacattacaatttactattctagtcgacctgcaggcggccgcactagtgatatcacaagtttgtacaaaaaagcaggctgaattcccaccatgcaggttcagctgcaggaatctggtggtggacttgttcaagctggtggatctcttagactctcttgcgctgcttctggaaggaccttctctagatatggaatgggatggttcaggcagctccctggaaaacagagagagcttgttacctctatcaccaggggtggaactaccacctacgctgattctgtgaagggaaggttcaccatctctagggataacgctaagaacaccgtgtacctccagatgaactctctcaagcctgaggataccgctgtgtactactgcaacgctagatctatttggagggattactggggacagggaactcaggtcaccgtttcttcagcggccgcacatcatcatcaccatcattgaggatccacccagctttcttgtacaaagtggtgatatcccgcggccatgctagagtccgcaaaaatcaccagtctctctctacaaatctatctctctctatttttctccagaataatgtgtgagtagttcccagataagggaattagggttcttatagggtttcgctcatgtgttgagcatataagaaacccttagtatgtatttgtatttgtaaaatacttctatcaataaaatttctaattcctaaaaccaaaatccagtgacctgcaggcatgcgacgtcg

SEQ ID NO: 364 - DNA, 9984 bp, Artificial Sequence
  pK7WG2-35S: 56F11_His_KDEL
ggccctctagaggatccccgggtaccgcgaattatcatacatgagaattaagggagtcacgttatgacccccgccgatgacgcgggacaagccgttttacgtttggaactgacagaaccgcaacgttgaaggagccactcagccgcgggtttctggagtttaatgagctaagcacatacgtcagaaaccattattgcgcgttcaaaagtcgcctaaggtcactatcagctagcaaatatttcttgtcaaaaatgctccactgacgttccataaattcccctcggtatccaattagagtctcatattcactctcaactcgatcgaggcatgattgaacaagatggattgcacgcaggttctccggccgcttgggtggagaggctattcggctatgactgggcacaacagacaatcggctgctctgatgccgccgtgttccggctgtcagcgcaggggcgcccggttctttttgtcaagaccgacctgtccggtgccctgaatgaactccaagacgaggcagcgcggctatcgtggctggccacgacgggcgttccttgcgcagctgtgctcgacgttgtcactgaagcgggaagggactggctgctattgggcgaagtgccggggcaggatctcctgtcatctcaccttgctcctgccgagaaagtatccatcatggctgatgcaatgcggcggctgcatacgcttgatccggctacctgcccattcgaccaccaagcgaaacatcgcatcgagcgaggacgtactcggatggaagccggtcttgtcgatcaggatgatctggacgaagagcatcaggggctcgcgccagccgaactgttcgccaggctcaaggcgcggatgcccgacggcgaggatctcgtcgtgacccagggcgatgcctgcttgccgaatatcatggtggaaaatggccgcttttctggattcatcgactgtggccggctgggtgtggcggaccgctatcaggacatagcgttggctacccgtgatattgctgaagagcttggcggcgaatgggctgaccgcttcctcgtgctttacggtatcgccgctcccgattcgcagcgcatcgccttctatcgccttcttgacgagttcttctgagcgggactctggggttcggactctagctagagtcaagcagatcgttcaaacatttggcaataaagtttcttaagattgaatcctgttgccggtcttgcgatgattatcatataatttctgttgaattacgttaagcatgtaataattaacatgtaatgcatgacgttatttatgagatgggttttttgattagagtcccgcaattatacatttaatacgcgatagaaaacaaaatatagcgcgcaaactaggataaattatcgcgcgcggtgtcatctatgttactagatcgaccggcatgcaagctgataattcaattcggcgttaattcagtacattaaaaacgtccgcaatgtgttattaagttgtctaagcgtcaatttgtttacaccacaatatatcctgccaccagccagccaacagctccccgaccggcagctcggcacaaaatcaccactcgatacaggcagcccatcagtccgggacggcgtcagcgggagagccgttgtaaggcggcagactttgctcatgttaccgatgctattcggaagaacggcaactaagctgccgggtttgaaacacggatgatctcgcggagggtagcatgttgattgtaacgatgacagagcgttgctgcctgtgatcaattcgggcacgaacccagtggacataagcctcgttcggttcgtaagctgtaatgcaagtagcgtaactgccgtcacgcaactggtccagaaccttgaccgaacgcagcggtggtaacggcgcagtggcggttttcatggcttcttgttatgacatgtttttttggggtacagtctatgcctcgggcatccaagcagcaagcgcgttacgccgtgggtcgatgtttgatgttatggagcagcaacgatgttacgcagcagggcagtcgccctaaaacaaagttaaacatcatgggggaagcggtgatcgccgaagtatcgactcaactatcagaggtagttggcgtcatcgagcgccatctcgaaccgacgttgctggccgtacatttgtacggctccgcagtggatggcggcctgaagccacacagtgatattgatttgctggttacggtgaccgtaaggcttgatgaaacaacgcggcgagctttgatcaacgaccttttggaaacttcggcttcccctggagagagcgagattctccgcgctgtagaagtcaccattgttgtgcacgacgacatcattccgtggcgttatccagctaagcgcgaactgcaatttggagaatggcagcgcaatgacattcttgcaggtatcttcgagccagccacgatcgacattgatctggctatcttgctgacaaaagcaagagaacatagcgttgccttggtaggtccagcggcggaggaactctttgatccggttcctgaacaggatctatttgaggcgctaaatgaaaccttaacgctatggaactcgccgcccgactgggctggcgatgagcgaaatgtagtgcttacgttgtcccgcatttggtacagcgcagtaaccggcaaaatcgcgccgaaggatgtcgctgccgactgggcaatggagcgcctgccggcccagtatcagcccgtcatacttgaagctagacaggcttatcttggacaagaagaagatcgcttggcctcgcgcgcagatcagttggaagaatttgtccactacgtgaaaggcgagatcaccaaggtagtcggcaaataatgtctagctagaaattcgttcaagccgacgccgcttcgccggcgttaactcaagcgattagatgcactaagcacataattgctcacagccaaactatcaggtcaagtctgcttttattatttttaagcgtgcataataagccctacacaaattgggagatatatcatgcatgaccaaaatcccttaacgtgagttttcgttccactgagcgtcagaccccgtagaaaagatcaaaggatcttcttgagatcctttttttctgcgcgtaatctgctgcttgcaaacaaaaaaaccaccgctaccagcggtggtttgtttgccggatcaagagctaccaactctttttccgaaggtaactggcttcagcagagcgcagataccaaatactgtccttctagtgtagccgtagttaggccaccacttcaagaactctgtagcaccgcctacatacctcgctctgctaatcctgttaccagtggctgctgccagtggcgataagtcgtgtcttaccgggttggactcaagacgatagttaccggataaggcgcagcggtcgggctgaacggggggttcgtgcacacagcccagcttggagcgaacgacctacaccgaactgagatacctacagcgtgagctatgagaaagcgccacgcttcccgaagggagaaaggcggacaggtatccggtaagcggcagggtcggaacaggagagcgcacgagggagcttccagggggaaacgcctggtatctttatagtcctgtcgggtttcgccacctctgacttgagcgtcgatttttgtgatgctcgtcaggggggcggagcctatggaaaaacgccagcaacgcggcctttttacggttcctggccttttgctggccttttgctcacatgttctttcctgcgttatcccctgattctgtggataaccgtattaccgcctttgagtgagctgataccgctcgccgcagccgaacgaccgagcgcagcgagtcagtgagcgaggaagcggaagagcgcctgatgcggtattttctccttacgcatctgtgcggtatttcacaccgcatatggtgcactctcagtacaatctgctctgatgccgcatagttaagccagtatacactccgctatcgctacgtgactgggtcatggctgcgccccgacacccgccaacacccgctgacgcgccctgacgggcttgtctgctcccggcatccgcttacagacaagctgtgaccgtctccgggagctgcatgtgtcagaggttttcaccgtcatcaccgaaacgcgcgaggcagggtgccttgatgtgggcgccggcggtcgagtggcgacggcgcggcttgtccgcgccctggtagattgcctggccgtaggccagccatttttgagcggccagcggccgcgataggccgacgcgaagcggcggggcgtagggagcgcagcgaccgaagggtaggcgctttttgcagctcttcggctgtgcgctggccagacagttatgcacaggccaggcgggttttaagagttttaataagttttaaagagttttaggcggaaaaatcgccttttttctcttttatatcagtcacttacatgtgtgaccggttcccaatgtacggctttgggttcccaatgtacgggttccggttcccaatgtacggctttgggttcccaatgtacgtgctatccacaggaaagagaccttttcgacctttttcccctgctagggcaatttgccctagcatctgctccgtacattaggaaccggcggatgcttcgccctcgatcaggttgcggtagcgcatgactaggatcgggccagcctgccccgcctcctccttcaaatcgtactccggcaggtcatttgacccgatcagcttgcgcacggtgaaacagaacttcttgaactctccggcgctgccactgcgttcgtagatcgtcttgaacaaccatctggcttctgccttgcctgcggcgcggcgtgccaggcggtagagaaaacggccgatgccgggatcgatcaaaaagtaatcggggtgaaccgtcagcacgtccgggttcttgccttctgtgatctcgcggtacatccaatcagctagctcgatctcgatgtactccggccgcccggtttcgctctttacgatcttgtagcggctaatcaaggcttcaccctcggataccgtcaccaggcggccgttcttggccttcttcgtacgctgcatggcaacgtgcgtggtgtttaaccgaatgcaggtttctaccaggtcgtctttctgctttccgccatcggctcgccggcagaacttgagtacgtccgcaacgtgtggacggaacacgcggccgggcttgtctcccttcccttcccggtatcggttcatggattcggttagatgggaaaccgccatcagtaccaggtcgtaatcccacacactggccatgccggccggccctgcggaaacctctacgtgcccgtctggaagctcgtagcggatcacctcgccagctcgtcggtcacgcttcgacagacggaaaacggccacgtccatgatgctgcgactatcgcgggtgcccacgtcatagagcatcggaacgaaaaaatctggttgctcgtcgcccttgggcggcttcctaatcgacggcgcaccggctgccggcggttgccgggattctttgcggattcgatcagcggccgcttgccacgattcaccggggcgtgcttctgcctcgatgcgttgccgctgggcggcctgcgcggccttcaacttctccaccaggtcatcacccagcgccgcgccgatttgtaccgggccggatggtttgcgaccgtcacgccgattcctcgggcttgggggttccagtgccattgcagggccggcagacaacccagccgcttacgcctggccaaccgcccgttcctccacacatggggcattccacggcgtcggtgcctggttgttcttgattttccatgccgcctcctttagccgctaaaattcatctactcatttattcatttgctcatttactctggtagctgcgcgatgtattcagatagcagctcggtaatggtcttgccttggcgtaccgcgtacatcttcagcttggtgtgatcctccgccggcaactgaaagttgacccgcttcatggctggcgtgtctgccaggctggccaacgttgcagccttgctgctgcgtgcgctcggacggccggcacttagcgtgtttgtgcttttgctcattttctctttacctcattaactcaaatgagttttgatttaatttcagcggccagcgcctggacctcgcgggcagcgtcgccctcgggttctgattcaagaacggttgtgccggcggcggcagtgcctgggtagctcacgcgctgcgtgatacgggactcaagaatgggcagctcgtacccggccagcgcctcggcaacctcaccgccgatgcgcgtgcctttgatcgcccgcgacacgacaaaggccgcttgtagccttccatccgtgacctcaatgcgctgcttaaccagctccaccaggtcggcggtggcccatatgtcgtaagggcttggctgcaccggaatcagcacgaagtcggctgccttgatcgcggacacagccaagtccgccgcctggggcgctccgtcgatcactacgaagtcgcgccggccgatggccttcacgtcgcggtcaatcgtcgggcggtcgatgccgacaacggttagcggttgatcttcccgcacggccgcccaatcgcgggcactgccctggggatcggaatcgactaacagaacatcggccccggcgagttgcagggcgcgggctagatgggttgcgatggtcgtcttgcctgacccgcctttctggttaagtacagcgataaccttcatgcgttccccttgcgtatttgtttatttactcatcgcatcatatacgcagcgaccgcatgacgcaagctgttttactcaaatacacatcacctttttagacggcggcgctcggtttcttcagcggccaagctggccggccaggccgccagcttggcatcagacaaaccggccaggatttcatgcagccgcacggttgagacgtgcgcgggcggctcgaacacgtacccggccgcgatcatctccgcctcgatctcttcggtaatgaaaaacggttcgtcctggccgtcctggtgcggtttcatgcttgttcctcttggcgttcattctcggcggccgccagggcgtcggcctcggtcaatgcgtcctcacggaaggcaccgcgccgcctggcctcggtgggcgtcacttcctcgctgcgctcaagtgcgcggtacagggtcgagcgatgcacgccaagcagtgcagccgcctctttcacggtgcggccttcctggtcgatcagctcgcgggcgtgcgcgatctgtgccggggtgagggtagggcgggggccaaacttcacgcctcgggccttggcggcctcgcgcccgctccgggtgcggtcgatgattagggaacgctcgaactcggcaatgccggcgaacacggtcaacaccatgcggccggccggcgtggtggtgtcggcccacggctctgccaggctacgcaggcccgcgccggcctcctggatgcgctcggcaatgtccagtaggtcgcgggtgctgcgggccaggcggtctagcctggtcactgtcacaacgtcgccagggcgtaggtggtcaagcatcctggccagctccgggcggtcgcgcctggtgccggtgatcttctcggaaaacagcttggtgcagccggccgcgtgcagttcggcccgttggttggtcaagtcctggtcgtcggtgctgacgcgggcatagcccagcaggccagcggcggcgctcttgttcatggcgtaatgtctccggttctagtcgcaagtattctactttatgcgactaaaacacgcgacaagaaaacgccaggaaaagggcagggcggcagcctgtcgcgtaacttaggacttgtgcgacatgtcgttttcagaagacggctgcactgaacgtcagaagccgactgcactatagcagcggaggggttggatcaaagtactttgatcccgaggggaaccctgtggttggcatgcacatacaaatggacgaacggataaaccttttcacgcccttttaaatatccgttattctaataaacgctcttttctcttaggtttacccgccaatatatcctgtcaaacactgatagtttaaactgaaggcgggaaacgacaatctgatccaagctcaagctaagcttgagctctcccatatggtcgagatctcctttgccccggagatcaccatggacgactttctctatctctacgatctaggaagaaagttcgacggagaaggtgacgataccatgttcaccaccgataatgagaagattagcctcttcaatttcagaaagaatgctgacccacagatggttagagaggcctacgcggcaggtctcatcaagacgatctacccgagtaataatctccaggagatcaaataccttcccaagaaggttaaagatgcagtcaaaagattcaggactaactgcatcaagaacacagagaaagatatatttctcaagatcagaagtactattccagtatggacgattcaaggcttgcttcataaaccaaggcaagtaatagagattggagtctctaagaaagtagttcctactgaatcaaaggccatggagtcaaaaattcagatcgaggatctaacagaactcgccgtgaagactggcgaacagttcatacagagtcttttacgactcaatgacaagaagaaaatcttcgtcaacatggtggagcacgacactctcgtctactccaagaatatcaaagatacagtctcagaagaccaaagggctattgagacttttcaacaaagggtaatatcgggaaacctcctcggattccattgcccagctatctgtcacttcatcaaaaggacagtagaaaaggaaggtggcacctacaaatgccatcattgcgataaaggaaaggctatcgttcaagatgcccctgccgacagtggtcccaaagatggacccccacccacgaggagcatcgtggaaaaagaagacgttccaaccacgtcttcaaagcaagtggattgatgtgatatctccactgacgtaagggatgacgcacaatcccactatccttcgcaagacccttcctctatataaggaagttcatttcatttggagaggactccggtatttttacaacaattaccacaacaaaacaaacaacaaacaacattacaatttactattctagtcgacctgcaggcggccgcactagtgatatcacaagtttgtacaaaaaagcaggctgaattcccaccatggcaaacaagcttttcttggtgtgcgctaccttcgctctttgcttccttttgactaacgctcaggttcagctgcaggaatctggtggtggacttgttcagtctggtggatctctcagactctcttgcgtgcactctaagaccaccttcaccagaaatgctatgggatggtacagacaggctctcggaaaagagagagagcttgttgctaccatcacctctggtggaactaccaactacgctgattctgtgaagggaaggttcaccatctctatggattctgctaagaacaccgtgtacctccagatgaactctctcaagcctgaggataccgctgtgtactactgcaacgtgaacaccagaaggatcttcggaggaaccgttagagaatactggggacaaggtactcaggtcaccgtttcttcagcggccgcacatcatcatcaccatcatggtgctgctaaggatgagctttgaggatccacccagctttcttgtacaaagtggtgatatcccgcggccatgctagagtccgcaaaaatcaccagtctctctctacaaatctatctctctctatttttctccagaataatgtgtgagtagttcccagataagggaattagggttcttatagggtttcgctcatgtgttgagcatataagaaacccttagtatgtatttgtatttgtaaaatacttctatcaataaaatttctaattcctaaaaccaaaatccagtgacctgcaggcatgcgacgtcg

SEQ ID NO: 365 - DNA, 10659 bp, Artificial Sequence
  pK7WG2-35S: sec_56F11_hinge_Fc_His
ggccctctagaggatccccgggtaccgcgaattatcatacatgagaattaagggagtcacgttatgacccccgccgatgacgcgggacaagccgttttacgtttggaactgacagaaccgcaacgttgaaggagccactcagccgcgggtttctggagtttaatgagctaagcacatacgtcagaaaccattattgcgcgttcaaaagtcgcctaaggtcactatcagctagcaaatatttcttgtcaaaaatgctccactgacgttccataaattcccctcggtatccaattagagtctcatattcactctcaactcgatcgaggcatgattgaacaagatggattgcacgcaggttctccggccgcttgggtggagaggctattcggctatgactgggcacaacagacaatcggctgctctgatgccgccgtgttccggctgtcagcgcaggggcgcccggttctttttgtcaagaccgacctgtccggtgccctgaatgaactccaagacgaggcagcgcggctatcgtggctggccacgacgggcgttccttgcgcagctgtgctcgacgttgtcactgaagcgggaagggactggctgctattgggcgaagtgccggggcaggatctcctgtcatctcaccttgctcctgccgagaaagtatccatcatggctgatgcaatgcggcggctgcatacgcttgatccggctacctgcccattcgaccaccaagcgaaacatcgcatcgagcgaggacgtactcggatggaagccggtcttgtcgatcaggatgatctggacgaagagcatcaggggctcgcgccagccgaactgttcgccaggctcaaggcgcggatgcccgacggcgaggatctcgtcgtgacccagggcgatgcctgcttgccgaatatcatggtggaaaatggccgcttttctggattcatcgactgtggccggctgggtgtggcggaccgctatcaggacatagcgttggctacccgtgatattgctgaagagcttggcggcgaatgggctgaccgcttcctcgtgctttacggtatcgccgctcccgattcgcagcgcatcgccttctatcgccttcttgacgagttcttctgagcgggactctggggttcggactctagctagagtcaagcagatcgttcaaacatttggcaataaagtttcttaagattgaatcctgttgccggtcttgcgatgattatcatataatttctgttgaattacgttaagcatgtaataattaacatgtaatgcatgacgttatttatgagatgggttttttgattagagtcccgcaattatacatttaatacgcgatagaaaacaaaatatagcgcgcaaactaggataaattatcgcgcgcggtgtcatctatgttactagatcgaccggcatgcaagctgataattcaattcggcgttaattcagtacattaaaaacgtccgcaatgtgttattaagttgtctaagcgtcaatttgtttacaccacaatatatcctgccaccagccagccaacagctccccgaccggcagctcggcacaaaatcaccactcgatacaggcagcccatcagtccgggacggcgtcagcgggagagccgttgtaaggcggcagactttgctcatgttaccgatgctattcggaagaacggcaactaagctgccgggtttgaaacacggatgatctcgcggagggtagcatgttgattgtaacgatgacagagcgttgctgcctgtgatcaattcgggcacgaacccagtggacataagcctcgttcggttcgtaagctgtaatgcaagtagcgtaactgccgtcacgcaactggtccagaaccttgaccgaacgcagcggtggtaacggcgcagtggcggttttcatggcttcttgttatgacatgtttttttggggtacagtctatgcctcgggcatccaagcagcaagcgcgttacgccgtgggtcgatgtttgatgttatggagcagcaacgatgttacgcagcagggcagtcgccctaaaacaaagttaaacatcatgggggaagcggtgatcgccgaagtatcgactcaactatcagaggtagttggcgtcatcgagcgccatctcgaaccgacgttgctggccgtacatttgtacggctccgcagtggatggcggcctgaagccacacagtgatattgatttgctggttacggtgaccgtaaggcttgatgaaacaacgcggcgagctttgatcaacgaccttttggaaacttcggcttcccctggagagagcgagattctccgcgctgtagaagtcaccattgttgtgcacgacgacatcattccgtggcgttatccagctaagcgcgaactgcaatttggagaatggcagcgcaatgacattcttgcaggtatcttcgagccagccacgatcgacattgatctggctatcttgctgacaaaagcaagagaacatagcgttgccttggtaggtccagcggcggaggaactctttgatccggttcctgaacaggatctatttgaggcgctaaatgaaaccttaacgctatggaactcgccgcccgactgggctggcgatgagcgaaatgtagtgcttacgttgtcccgcatttggtacagcgcagtaaccggcaaaatcgcgccgaaggatgtcgctgccgactgggcaatggagcgcctgccggcccagtatcagcccgtcatacttgaagctagacaggcttatcttggacaagaagaagatcgcttggcctcgcgcgcagatcagttggaagaatttgtccactacgtgaaaggcgagatcaccaaggtagtcggcaaataatgtctagctagaaattcgttcaagccgacgccgcttcgccggcgttaactcaagcgattagatgcactaagcacataattgctcacagccaaactatcaggtcaagtctgcttttattatttttaagcgtgcataataagccctacacaaattgggagatatatcatgcatgaccaaaatcccttaacgtgagttttcgttccactgagcgtcagaccccgtagaaaagatcaaaggatcttcttgagatcctttttttctgcgcgtaatctgctgcttgcaaacaaaaaaaccaccgctaccagcggtggtttgtttgccggatcaagagctaccaactctttttccgaaggtaactggcttcagcagagcgcagataccaaatactgtccttctagtgtagccgtagttaggccaccacttcaagaactctgtagcaccgcctacatacctcgctctgctaatcctgttaccagtggctgctgccagtggcgataagtcgtgtcttaccgggttggactcaagacgatagttaccggataaggcgcagcggtcgggctgaacggggggttcgtgcacacagcccagcttggagcgaacgacctacaccgaactgagatacctacagcgtgagctatgagaaagcgccacgcttcccgaagggagaaaggcggacaggtatccggtaagcggcagggtcggaacaggagagcgcacgagggagcttccagggggaaacgcctggtatctttatagtcctgtcgggtttcgccacctctgacttgagcgtcgatttttgtgatgctcgtcaggggggcggagcctatggaaaaacgccagcaacgcggcctttttacggttcctggccttttgctggccttttgctcacatgttctttcctgcgttatcccctgattctgtggataaccgtattaccgcctttgagtgagctgataccgctcgccgcagccgaacgaccgagcgcagcgagtcagtgagcgaggaagcggaagagcgcctgatgcggtattttctccttacgcatctgtgcggtatttcacaccgcatatggtgcactctcagtacaatctgctctgatgccgcatagttaagccagtatacactccgctatcgctacgtgactgggtcatggctgcgccccgacacccgccaacacccgctgacgcgccctgacgggcttgtctgctcccggcatccgcttacagacaagctgtgaccgtctccgggagctgcatgtgtcagaggttttcaccgtcatcaccgaaacgcgcgaggcagggtgccttgatgtgggcgccggcggtcgagtggcgacggcgcggcttgtccgcgccctggtagattgcctggccgtaggccagccatttttgagcggccagcggccgcgataggccgacgcgaagcggcggggcgtagggagcgcagcgaccgaagggtaggcgctttttgcagctcttcggctgtgcgctggccagacagttatgcacaggccaggcgggttttaagagttttaataagttttaaagagttttaggcggaaaaatcgccttttttctcttttatatcagtcacttacatgtgtgaccggttcccaatgtacggctttgggttcccaatgtacgggttccggttcccaatgtacggctttgggttcccaatgtacgtgctatccacaggaaagagaccttttcgacctttttcccctgctagggcaatttgccctagcatctgctccgtacattaggaaccggcggatgcttcgccctcgatcaggttgcggtagcgcatgactaggatcgggccagcctgccccgcctcctccttcaaatcgtactccggcaggtcatttgacccgatcagcttgcgcacggtgaaacagaacttcttgaactctccggcgctgccactgcgttcgtagatcgtcttgaacaaccatctggcttctgccttgcctgcggcgcggcgtgccaggcggtagagaaaacggccgatgccgggatcgatcaaaaagtaatcggggtgaaccgtcagcacgtccgggttcttgccttctgtgatctcgcggtacatccaatcagctagctcgatctcgatgtactccggccgcccggtttcgctctttacgatcttgtagcggctaatcaaggcttcaccctcggataccgtcaccaggcggccgttcttggccttcttcgtacgctgcatggcaacgtgcgtggtgtttaaccgaatgcaggtttctaccaggtcgtctttctgctttccgccatcggctcgccggcagaacttgagtacgtccgcaacgtgtggacggaacacgcggccgggcttgtctcccttcccttcccggtatcggttcatggattcggttagatgggaaaccgccatcagtaccaggtcgtaatcccacacactggccatgccggccggccctgcggaaacctctacgtgcccgtctggaagctcgtagcggatcacctcgccagctcgtcggtcacgcttcgacagacggaaaacggccacgtccatgatgctgcgactatcgcgggtgcccacgtcatagagcatcggaacgaaaaaatctggttgctcgtcgcccttgggcggcttcctaatcgacggcgcaccggctgccggcggttgccgggattctttgcggattcgatcagcggccgcttgccacgattcaccggggcgtgcttctgcctcgatgcgttgccgctgggcggcctgcgcggccttcaacttctccaccaggtcatcacccagcgccgcgccgatttgtaccgggccggatggtttgcgaccgtcacgccgattcctcgggcttgggggttccagtgccattgcagggccggcagacaacccagccgcttacgcctggccaaccgcccgttcctccacacatggggcattccacggcgtcggtgcctggttgttcttgattttccatgccgcctcctttagccgctaaaattcatctactcatttattcatttgctcatttactctggtagctgcgcgatgtattcagatagcagctcggtaatggtcttgccttggcgtaccgcgtacatcttcagcttggtgtgatcctccgccggcaactgaaagttgacccgcttcatggctggcgtgtctgccaggctggccaacgttgcagccttgctgctgcgtgcgctcggacggccggcacttagcgtgtttgtgcttttgctcattttctctttacctcattaactcaaatgagttttgatttaatttcagcggccagcgcctggacctcgcgggcagcgtcgccctcgggttctgattcaagaacggttgtgccggcggcggcagtgcctgggtagctcacgcgctgcgtgatacgggactcaagaatgggcagctcgtacccggccagcgcctcggcaacctcaccgccgatgcgcgtgcctttgatcgcccgcgacacgacaaaggccgcttgtagccttccatccgtgacctcaatgcgctgcttaaccagctccaccaggtcggcggtggcccatatgtcgtaagggcttggctgcaccggaatcagcacgaagtcggctgccttgatcgcggacacagccaagtccgccgcctggggcgctccgtcgatcactacgaagtcgcgccggccgatggccttcacgtcgcggtcaatcgtcgggcggtcgatgccgacaacggttagcggttgatcttcccgcacggccgcccaatcgcgggcactgccctggggatcggaatcgactaacagaacatcggccccggcgagttgcagggcgcgggctagatgggttgcgatggtcgtcttgcctgacccgcctttctggttaagtacagcgataaccttcatgcgttccccttgcgtatttgtttatttactcatcgcatcatatacgcagcgaccgcatgacgcaagctgttttactcaaatacacatcacctttttagacggcggcgctcggtttcttcagcggccaagctggccggccaggccgccagcttggcatcagacaaaccggccaggatttcatgcagccgcacggttgagacgtgcgcgggcggctcgaacacgtacccggccgcgatcatctccgcctcgatctcttcggtaatgaaaaacggttcgtcctggccgtcctggtgcggtttcatgcttgttcctcttggcgttcattctcggcggccgccagggcgtcggcctcggtcaatgcgtcctcacggaaggcaccgcgccgcctggcctcggtgggcgtcacttcctcgctgcgctcaagtgcgcggtacagggtcgagcgatgcacgccaagcagtgcagccgcctctttcacggtgcggccttcctggtcgatcagctcgcgggcgtgcgcgatctgtgccggggtgagggtagggcgggggccaaacttcacgcctcgggccttggcggcctcgcgcccgctccgggtgcggtcgatgattagggaacgctcgaactcggcaatgccggcgaacacggtcaacaccatgcggccggccggcgtggtggtgtcggcccacggctctgccaggctacgcaggcccgcgccggcctcctggatgcgctcggcaatgtccagtaggtcgcgggtgctgcgggccaggcggtctagcctggtcactgtcacaacgtcgccagggcgtaggtggtcaagcatcctggccagctccgggcggtcgcgcctggtgccggtgatcttctcggaaaacagcttggtgcagccggccgcgtgcagttcggcccgttggttggtcaagtcctggtcgtcggtgctgacgcgggcatagcccagcaggccagcggcggcgctcttgttcatggcgtaatgtctccggttctagtcgcaagtattctactttatgcgactaaaacacgcgacaagaaaacgccaggaaaagggcagggcggcagcctgtcgcgtaacttaggacttgtgcgacatgtcgttttcagaagacggctgcactgaacgtcagaagccgactgcactatagcagcggaggggttggatcaaagtactttgatcccgaggggaaccctgtggttggcatgcacatacaaatggacgaacggataaaccttttcacgcccttttaaatatccgttattctaataaacgctcttttctcttaggtttacccgccaatatatcctgtcaaacactgatagtttaaactgaaggcgggaaacgacaatctgatccaagctcaagctaagcttgagctctcccatatggtcgagatctcctttgccccggagatcaccatggacgactttctctatctctacgatctaggaagaaagttcgacggagaaggtgacgataccatgttcaccaccgataatgagaagattagcctcttcaatttcagaaagaatgctgacccacagatggttagagaggcctacgcggcaggtctcatcaagacgatctacccgagtaataatctccaggagatcaaataccttcccaagaaggttaaagatgcagtcaaaagattcaggactaactgcatcaagaacacagagaaagatatatttctcaagatcagaagtactattccagtatggacgattcaaggcttgcttcataaaccaaggcaagtaatagagattggagtctctaagaaagtagttcctactgaatcaaaggccatggagtcaaaaattcagatcgaggatctaacagaactcgccgtgaagactggcgaacagttcatacagagtcttttacgactcaatgacaagaagaaaatcttcgtcaacatggtggagcacgacactctcgtctactccaagaatatcaaagatacagtctcagaagaccaaagggctattgagacttttcaacaaagggtaatatcgggaaacctcctcggattccattgcccagctatctgtcacttcatcaaaaggacagtagaaaaggaaggtggcacctacaaatgccatcattgcgataaaggaaaggctatcgttcaagatgcccctgccgacagtggtcccaaagatggacccccacccacgaggagcatcgtggaaaaagaagacgttccaaccacgtcttcaaagcaagtggattgatgtgatatctccactgacgtaagggatgacgcacaatcccactatccttcgcaagacccttcctctatataaggaagttcatttcatttggagaggactccggtatttttacaacaattaccacaacaaaacaaacaacaaacaacattacaatttactattctagtcgacctgcaggcggccgcactagtgatatcacaagtttgtacaaaaaagcaggctgaattcccaccatggcaaacaagcttttcttggtgtgcgctaccttcgctctttgcttccttttgactaacgctcaggttcagctgcaggaatctggtggtggacttgttcagtctggtggatctctcagactctcttgcgtgcactctaagaccaccttcaccagaaatgctatgggatggtacagacaggctctcggaaaagagagagagcttgttgctaccatcacctctggtggaactaccaactacgctgattctgtgaagggaaggttcaccatctctatggattctgctaagaacaccgtgtacctccagatgaactctctcaagcctgaggataccgctgtgtactactgcaacgtgaacaccagaaggatcttcggaggaaccgttagagaatactggggacaaggtactcaggtcaccgtttcttcacctagaatccctaagccttctacccctcctggatcttcttgtcctcctggaaatatcctcggaggaccttcagtgttcatcttcccacctaagcctaaggatgctctcatgatctcactcacccctaaggttacatgcgttgtggtggatgtgtctgaggatgatcctgatgtgcacgtgtcatggttcgtggataacaaagaggtgcacactgcttggactcagcctagagaagctcagtacaactctaccttcagggtggtgtctgctctccctatccaacaccaagattggatgaggggtaaagagttcaagtgcaaggtgaacaacaaggctctccctgctcctatcgagaggactatctctaaacctaagggaagggctcagacccctcaagtgtatacaattcctccacctagggaacagatgtctaagaagaaggtttcactcacttgcctcgtgaccaacttcttcagtgaggctatctctgttgagtgggagaggaatggtgagcttgagcaggattacaagaacacccctcctatcctcgattctgatggaacctacttcctctactctaagctcaccgtggataccgattcttggttgcagggtgagatcttcacttgctctgttgtgcatgaggctctccacaaccatcacacccagaagaacctcagtagatctcctggtaaagcggccgcacatcatcatcaccatcattgaggatccacccagctttcttgtacaaagtggtgatatcccgcggccatgctagagtccgcaaaaatcaccagtctctctctacaaatctatctctctctatttttctccagaataatgtgtgagtagttcccagataagggaattagggttcttatagggtttcgctcatgtgttgagcatataagaaacccttagtatgtatttgtatttgtaaaatacttctatcaataaaatttctaattcctaaaaccaaaatccagtgacctgcaggcatgcgacgtcg

SEQ ID NO: 366 - DNA, 10353 bp, Artificial Sequence
  pK7WG2-35S: sec_56F11-9GS-56F11_His
ggccctctagaggatccccgggtaccgcgaattatcatacatgagaattaagggagtcacgttatgacccccgccgatgacgcgggacaagccgttttacgtttggaactgacagaaccgcaacgttgaaggagccactcagccgcgggtttctggagtttaatgagctaagcacatacgtcagaaaccattattgcgcgttcaaaagtcgcctaaggtcactatcagctagcaaatatttcttgtcaaaaatgctccactgacgttccataaattcccctcggtatccaattagagtctcatattcactctcaactcgatcgaggcatgattgaacaagatggattgcacgcaggttctccggccgcttgggtggagaggctattcggctatgactgggcacaacagacaatcggctgctctgatgccgccgtgttccggctgtcagcgcaggggcgcccggttctttttgtcaagaccgacctgtccggtgccctgaatgaactccaagacgaggcagcgcggctatcgtggctggccacgacgggcgttccttgcgcagctgtgctcgacgttgtcactgaagcgggaagggactggctgctattgggcgaagtgccggggcaggatctcctgtcatctcaccttgctcctgccgagaaagtatccatcatggctgatgcaatgcggcggctgcatacgcttgatccggctacctgcccattcgaccaccaagcgaaacatcgcatcgagcgaggacgtactcggatggaagccggtcttgtcgatcaggatgatctggacgaagagcatcaggggctcgcgccagccgaactgttcgccaggctcaaggcgcggatgcccgacggcgaggatctcgtcgtgacccagggcgatgcctgcttgccgaatatcatggtggaaaatggccgcttttctggattcatcgactgtggccggctgggtgtggcggaccgctatcaggacatagcgttggctacccgtgatattgctgaagagcttggcggcgaatgggctgaccgcttcctcgtgctttacggtatcgccgctcccgattcgcagcgcatcgccttctatcgccttcttgacgagttcttctgagcgggactctggggttcggactctagctagagtcaagcagatcgttcaaacatttggcaataaagtttcttaagattgaatcctgttgccggtcttgcgatgattatcatataatttctgttgaattacgttaagcatgtaataattaacatgtaatgcatgacgttatttatgagatgggttttttgattagagtcccgcaattatacatttaatacgcgatagaaaacaaaatatagcgcgcaaactaggataaattatcgcgcgcggtgtcatctatgttactagatcgaccggcatgcaagctgataattcaattcggcgttaattcagtacattaaaaacgtccgcaatgtgttattaagttgtctaagcgtcaatttgtttacaccacaatatatcctgccaccagccagccaacagctccccgaccggcagctcggcacaaaatcaccactcgatacaggcagcccatcagtccgggacggcgtcagcgggagagccgttgtaaggcggcagactttgctcatgttaccgatgctattcggaagaacggcaactaagctgccgggtttgaaacacggatgatctcgcggagggtagcatgttgattgtaacgatgacagagcgttgctgcctgtgatcaattcgggcacgaacccagtggacataagcctcgttcggttcgtaagctgtaatgcaagtagcgtaactgccgtcacgcaactggtccagaaccttgaccgaacgcagcggtggtaacggcgcagtggcggttttcatggcttcttgttatgacatgtttttttggggtacagtctatgcctcgggcatccaagcagcaagcgcgttacgccgtgggtcgatgtttgatgttatggagcagcaacgatgttacgcagcagggcagtcgccctaaaacaaagttaaacatcatgggggaagcggtgatcgccgaagtatcgactcaactatcagaggtagttggcgtcatcgagcgccatctcgaaccgacgttgctggccgtacatttgtacggctccgcagtggatggcggcctgaagccacacagtgatattgatttgctggttacggtgaccgtaaggcttgatgaaacaacgcggcgagctttgatcaacgaccttttggaaacttcggcttcccctggagagagcgagattctccgcgctgtagaagtcaccattgttgtgcacgacgacatcattccgtggcgttatccagctaagcgcgaactgcaatttggagaatggcagcgcaatgacattcttgcaggtatcttcgagccagccacgatcgacattgatctggctatcttgctgacaaaagcaagagaacatagcgttgccttggtaggtccagcggcggaggaactctttgatccggttcctgaacaggatctatttgaggcgctaaatgaaaccttaacgctatggaactcgccgcccgactgggctggcgatgagcgaaatgtagtgcttacgttgtcccgcatttggtacagcgcagtaaccggcaaaatcgcgccgaaggatgtcgctgccgactgggcaatggagcgcctgccggcccagtatcagcccgtcatacttgaagctagacaggcttatcttggacaagaagaagatcgcttggcctcgcgcgcagatcagttggaagaatttgtccactacgtgaaaggcgagatcaccaaggtagtcggcaaataatgtctagctagaaattcgttcaagccgacgccgcttcgccggcgttaactcaagcgattagatgcactaagcacataattgctcacagccaaactatcaggtcaagtctgcttttattatttttaagcgtgcataataagccctacacaaattgggagatatatcatgcatgaccaaaatcccttaacgtgagttttcgttccactgagcgtcagaccccgtagaaaagatcaaaggatcttcttgagatcctttttttctgcgcgtaatctgctgcttgcaaacaaaaaaaccaccgctaccagcggtggtttgtttgccggatcaagagctaccaactctttttccgaaggtaactggcttcagcagagcgcagataccaaatactgtccttctagtgtagccgtagttaggccaccacttcaagaactctgtagcaccgcctacatacctcgctctgctaatcctgttaccagtggctgctgccagtggcgataagtcgtgtcttaccgggttggactcaagacgatagttaccggataaggcgcagcggtcgggctgaacggggggttcgtgcacacagcccagcttggagcgaacgacctacaccgaactgagatacctacagcgtgagctatgagaaagcgccacgcttcccgaagggagaaaggcggacaggtatccggtaagcggcagggtcggaacaggagagcgcacgagggagcttccagggggaaacgcctggtatctttatagtcctgtcgggtttcgccacctctgacttgagcgtcgatttttgtgatgctcgtcaggggggcggagcctatggaaaaacgccagcaacgcggcctttttacggttcctggccttttgctggccttttgctcacatgttctttcctgcgttatcccctgattctgtggataaccgtattaccgcctttgagtgagctgataccgctcgccgcagccgaacgaccgagcgcagcgagtcagtgagcgaggaagcggaagagcgcctgatgcggtattttctccttacgcatctgtgcggtatttcacaccgcatatggtgcactctcagtacaatctgctctgatgccgcatagttaagccagtatacactccgctatcgctacgtgactgggtcatggctgcgccccgacacccgccaacacccgctgacgcgccctgacgggcttgtctgctcccggcatccgcttacagacaagctgtgaccgtctccgggagctgcatgtgtcagaggttttcaccgtcatcaccgaaacgcgcgaggcagggtgccttgatgtgggcgccggcggtcgagtggcgacggcgcggcttgtccgcgccctggtagattgcctggccgtaggccagccatttttgagcggccagcggccgcgataggccgacgcgaagcggcggggcgtagggagcgcagcgaccgaagggtaggcgctttttgcagctcttcggctgtgcgctggccagacagttatgcacaggccaggcgggttttaagagttttaataagttttaaagagttttaggcggaaaaatcgccttttttctcttttatatcagtcacttacatgtgtgaccggttcccaatgtacggctttgggttcccaatgtacgggttccggttcccaatgtacggctttgggttcccaatgtacgtgctatccacaggaaagagaccttttcgacctttttcccctgctagggcaatttgccctagcatctgctccgtacattaggaaccggcggatgcttcgccctcgatcaggttgcggtagcgcatgactaggatcgggccagcctgccccgcctcctccttcaaatcgtactccggcaggtcatttgacccgatcagcttgcgcacggtgaaacagaacttcttgaactctccggcgctgccactgcgttcgtagatcgtcttgaacaaccatctggcttctgccttgcctgcggcgcggcgtgccaggcggtagagaaaacggccgatgccgggatcgatcaaaaagtaatcggggtgaaccgtcagcacgtccgggttcttgccttctgtgatctcgcggtacatccaatcagctagctcgatctcgatgtactccggccgcccggtttcgctctttacgatcttgtagcggctaatcaaggcttcaccctcggataccgtcaccaggcggccgttcttggccttcttcgtacgctgcatggcaacgtgcgtggtgtttaaccgaatgcaggtttctaccaggtcgtctttctgctttccgccatcggctcgccggcagaacttgagtacgtccgcaacgtgtggacggaacacgcggccgggcttgtctcccttcccttcccggtatcggttcatggattcggttagatgggaaaccgccatcagtaccaggtcgtaatcccacacactggccatgccggccggccctgcggaaacctctacgtgcccgtctggaagctcgtagcggatcacctcgccagctcgtcggtcacgcttcgacagacggaaaacggccacgtccatgatgctgcgactatcgcgggtgcccacgtcatagagcatcggaacgaaaaaatctggttgctcgtcgcccttgggcggcttcctaatcgacggcgcaccggctgccggcggttgccgggattctttgcggattcgatcagcggccgcttgccacgattcaccggggcgtgcttctgcctcgatgcgttgccgctgggcggcctgcgcggccttcaacttctccaccaggtcatcacccagcgccgcgccgatttgtaccgggccggatggtttgcgaccgtcacgccgattcctcgggcttgggggttccagtgccattgcagggccggcagacaacccagccgcttacgcctggccaaccgcccgttcctccacacatggggcattccacggcgtcggtgcctggttgttcttgattttccatgccgcctcctttagccgctaaaattcatctactcatttattcatttgctcatttactctggtagctgcgcgatgtattcagatagcagctcggtaatggtcttgccttggcgtaccgcgtacatcttcagcttggtgtgatcctccgccggcaactgaaagttgacccgcttcatggctggcgtgtctgccaggctggccaacgttgcagccttgctgctgcgtgcgctcggacggccggcacttagcgtgtttgtgcttttgctcattttctctttacctcattaactcaaatgagttttgatttaatttcagcggccagcgcctggacctcgcgggcagcgtcgccctcgggttctgattcaagaacggttgtgccggcggcggcagtgcctgggtagctcacgcgctgcgtgatacgggactcaagaatgggcagctcgtacccggccagcgcctcggcaacctcaccgccgatgcgcgtgcctttgatcgcccgcgacacgacaaaggccgcttgtagccttccatccgtgacctcaatgcgctgcttaaccagctccaccaggtcggcggtggcccatatgtcgtaagggcttggctgcaccggaatcagcacgaagtcggctgccttgatcgcggacacagccaagtccgccgcctggggcgctccgtcgatcactacgaagtcgcgccggccgatggccttcacgtcgcggtcaatcgtcgggcggtcgatgccgacaacggttagcggttgatcttcccgcacggccgcccaatcgcgggcactgccctggggatcggaatcgactaacagaacatcggccccggcgagttgcagggcgcgggctagatgggttgcgatggtcgtcttgcctgacccgcctttctggttaagtacagcgataaccttcatgcgttccccttgcgtatttgtttatttactcatcgcatcatatacgcagcgaccgcatgacgcaagctgttttactcaaatacacatcacctttttagacggcggcgctcggtttcttcagcggccaagctggccggccaggccgccagcttggcatcagacaaaccggccaggatttcatgcagccgcacggttgagacgtgcgcgggcggctcgaacacgtacccggccgcgatcatctccgcctcgatctcttcggtaatgaaaaacggttcgtcctggccgtcctggtgcggtttcatgcttgttcctcttggcgttcattctcggcggccgccagggcgtcggcctcggtcaatgcgtcctcacggaaggcaccgcgccgcctggcctcggtgggcgtcacttcctcgctgcgctcaagtgcgcggtacagggtcgagcgatgcacgccaagcagtgcagccgcctctttcacggtgcggccttcctggtcgatcagctcgcgggcgtgcgcgatctgtgccggggtgagggtagggcgggggccaaacttcacgcctcgggccttggcggcctcgcgcccgctccgggtgcggtcgatgattagggaacgctcgaactcggcaatgccggcgaacacggtcaacaccatgcggccggccggcgtggtggtgtcggcccacggctctgccaggctacgcaggcccgcgccggcctcctggatgcgctcggcaatgtccagtaggtcgcgggtgctgcgggccaggcggtctagcctggtcactgtcacaacgtcgccagggcgtaggtggtcaagcatcctggccagctccgggcggtcgcgcctggtgccggtgatcttctcggaaaacagcttggtgcagccggccgcgtgcagttcggcccgttggttggtcaagtcctggtcgtcggtgctgacgcgggcatagcccagcaggccagcggcggcgctcttgttcatggcgtaatgtctccggttctagtcgcaagtattctactttatgcgactaaaacacgcgacaagaaaacgccaggaaaagggcagggcggcagcctgtcgcgtaacttaggacttgtgcgacatgtcgttttcagaagacggctgcactgaacgtcagaagccgactgcactatagcagcggaggggttggatcaaagtactttgatcccgaggggaaccctgtggttggcatgcacatacaaatggacgaacggataaaccttttcacgcccttttaaatatccgttattctaataaacgctcttttctcttaggtttacccgccaatatatcctgtcaaacactgatagtttaaactgaaggcgggaaacgacaatctgatccaagctcaagctaagcttgagctctcccatatggtcgagatctcctttgccccggagatcaccatggacgactttctctatctctacgatctaggaagaaagttcgacggagaaggtgacgataccatgttcaccaccgataatgagaagattagcctcttcaatttcagaaagaatgctgacccacagatggttagagaggcctacgcggcaggtctcatcaagacgatctacccgagtaataatctccaggagatcaaataccttcccaagaaggttaaagatgcagtcaaaagattcaggactaactgcatcaagaacacagagaaagatatatttctcaagatcagaagtactattccagtatggacgattcaaggcttgcttcataaaccaaggcaagtaatagagattggagtctctaagaaagtagttcctactgaatcaaaggccatggagtcaaaaattcagatcgaggatctaacagaactcgccgtgaagactggcgaacagttcatacagagtcttttacgactcaatgacaagaagaaaatcttcgtcaacatggtggagcacgacactctcgtctactccaagaatatcaaagatacagtctcagaagaccaaagggctattgagacttttcaacaaagggtaatatcgggaaacctcctcggattccattgcccagctatctgtcacttcatcaaaaggacagtagaaaaggaaggtggcacctacaaatgccatcattgcgataaaggaaaggctatcgttcaagatgcccctgccgacagtggtcccaaagatggacccccacccacgaggagcatcgtggaaaaagaagacgttccaaccacgtcttcaaagcaagtggattgatgtgatatctccactgacgtaagggatgacgcacaatcccactatccttcgcaagacccttcctctatataaggaagttcatttcatttggagaggactccggtatttttacaacaattaccacaacaaaacaaacaacaaacaacattacaatttactattctagtcgacctgcaggcggccgcactagtgatatcacaagtttgtacaaaaaagcaggctgaattcccaccatggcaaacaagcttttcttggtgtgcgctaccttcgctctttgcttccttttgactaacgctcaggttcaattgcaagagtctggtggtggactcgtgcaatctggtggatctcttagactctcttgcgtgcactctaagaccaccttcaccagaaatgctatgggatggtacagacaggctctcggaaaagagagagagcttgttgctaccatcacctctggtggaactaccaactacgctgattctgtgaagggaaggttcaccatctctatggattctgctaagaacaccgtgtacctccagatgaactctctcaagcctgaggataccgctgtgtactactgcaacgtgaacaccagaaggatcttcggaggaaccgttagagaatactggggacaaggtactcaggtcaccgtttcttcaggtggtggtggaagtggtggtggttctcaagttcaactgcaggaatcaggtggtggattggttcagtctggtggttctctcaggttgtcatgcgttcacagtaagactactttcactaggaacgcaatgggatggtataggcaagcacttggtaaagagagggaactcgttgcaactatcacaagtggtggaaccactaattacgcagatagtgttaagggaagattcactattagtatggatagtgcaaagaacactgtttacttgcaaatgaactcattgaagccagaggatacagcagtttattactgtaatgttaacactagaagaattttcggtggtactgtgagagagtattggggacagggaacccaggttacagttagttcagcggccgcacatcatcaccatcaccattgaggatccacccagctttcttgtacaaagtggtgatatcccgcggccatgctagagtccgcaaaaatcaccagtctctctctacaaatctatctctctctatttttctccagaataatgtgtgagtagttcccagataagggaattagggttcttatagggtttcgctcatgtgttgagcatataagaaacccttagtatgtatttgtatttgtaaaatacttctatcaataaaatttctaattcctaaaaccaaaatccagtgacctgcaggcatgcgacgtcg

SEQ ID NO: 367 - DNA, 9963 bp, Artificial Sequence
  pK7WG2-35S: sec_56F11_His
ggccctctagaggatccccgggtaccgcgaattatcatacatgagaattaagggagtcacgttatgacccccgccgatgacgcgggacaagccgttttacgtttggaactgacagaaccgcaacgttgaaggagccactcagccgcgggtttctggagtttaatgagctaagcacatacgtcagaaaccattattgcgcgttcaaaagtcgcctaaggtcactatcagctagcaaatatttcttgtcaaaaatgctccactgacgttccataaattcccctcggtatccaattagagtctcatattcactctcaactcgatcgaggcatgattgaacaagatggattgcacgcaggttctccggccgcttgggtggagaggctattcggctatgactgggcacaacagacaatcggctgctctgatgccgccgtgttccggctgtcagcgcaggggcgcccggttctttttgtcaagaccgacctgtccggtgccctgaatgaactccaagacgaggcagcgcggctatcgtggctggccacgacgggcgttccttgcgcagctgtgctcgacgttgtcactgaagcgggaagggactggctgctattgggcgaagtgccggggcaggatctcctgtcatctcaccttgctcctgccgagaaagtatccatcatggctgatgcaatgcggcggctgcatacgcttgatccggctacctgcccattcgaccaccaagcgaaacatcgcatcgagcgaggacgtactcggatggaagccggtcttgtcgatcaggatgatctggacgaagagcatcaggggctcgcgccagccgaactgttcgccaggctcaaggcgcggatgcccgacggcgaggatctcgtcgtgacccagggcgatgcctgcttgccgaatatcatggtggaaaatggccgcttttctggattcatcgactgtggccggctgggtgtggcggaccgctatcaggacatagcgttggctacccgtgatattgctgaagagcttggcggcgaatgggctgaccgcttcctcgtgctttacggtatcgccgctcccgattcgcagcgcatcgccttctatcgccttcttgacgagttcttctgagcgggactctggggttcggactctagctagagtcaagcagatcgttcaaacatttggcaataaagtttcttaagattgaatcctgttgccggtcttgcgatgattatcatataatttctgttgaattacgttaagcatgtaataattaacatgtaatgcatgacgttatttatgagatgggttttttgattagagtcccgcaattatacatttaatacgcgatagaaaacaaaatatagcgcgcaaactaggataaattatcgcgcgcggtgtcatctatgttactagatcgaccggcatgcaagctgataattcaattcggcgttaattcagtacattaaaaacgtccgcaatgtgttattaagttgtctaagcgtcaatttgtttacaccacaatatatcctgccaccagccagccaacagctccccgaccggcagctcggcacaaaatcaccactcgatacaggcagcccatcagtccgggacggcgtcagcgggagagccgttgtaaggcggcagactttgctcatgttaccgatgctattcggaagaacggcaactaagctgccgggtttgaaacacggatgatctcgcggagggtagcatgttgattgtaacgatgacagagcgttgctgcctgtgatcaattcgggcacgaacccagtggacataagcctcgttcggttcgtaagctgtaatgcaagtagcgtaactgccgtcacgcaactggtccagaaccttgaccgaacgcagcggtggtaacggcgcagtggcggttttcatggcttcttgttatgacatgtttttttggggtacagtctatgcctcgggcatccaagcagcaagcgcgttacgccgtgggtcgatgtttgatgttatggagcagcaacgatgttacgcagcagggcagtcgccctaaaacaaagttaaacatcatgggggaagcggtgatcgccgaagtatcgactcaactatcagaggtagttggcgtcatcgagcgccatctcgaaccgacgttgctggccgtacatttgtacggctccgcagtggatggcggcctgaagccacacagtgatattgatttgctggttacggtgaccgtaaggcttgatgaaacaacgcggcgagctttgatcaacgaccttttggaaacttcggcttcccctggagagagcgagattctccgcgctgtagaagtcaccattgttgtgcacgacgacatcattccgtggcgttatccagctaagcgcgaactgcaatttggagaatggcagcgcaatgacattcttgcaggtatcttcgagccagccacgatcgacattgatctggctatcttgctgacaaaagcaagagaacatagcgttgccttggtaggtccagcggcggaggaactctttgatccggttcctgaacaggatctatttgaggcgctaaatgaaaccttaacgctatggaactcgccgcccgactgggctggcgatgagcgaaatgtagtgcttacgttgtcccgcatttggtacagcgcagtaaccggcaaaatcgcgccgaaggatgtcgctgccgactgggcaatggagcgcctgccggcccagtatcagcccgtcatacttgaagctagacaggcttatcttggacaagaagaagatcgcttggcctcgcgcgcagatcagttggaagaatttgtccactacgtgaaaggcgagatcaccaaggtagtcggcaaataatgtctagctagaaattcgttcaagccgacgccgcttcgccggcgttaactcaagcgattagatgcactaagcacataattgctcacagccaaactatcaggtcaagtctgcttttattatttttaagcgtgcataataagccctacacaaattgggagatatatcatgcatgaccaaaatcccttaacgtgagttttcgttccactgagcgtcagaccccgtagaaaagatcaaaggatcttcttgagatcctttttttctgcgcgtaatctgctgcttgcaaacaaaaaaaccaccgctaccagcggtggtttgtttgccggatcaagagctaccaactctttttccgaaggtaactggcttcagcagagcgcagataccaaatactgtccttctagtgtagccgtagttaggccaccacttcaagaactctgtagcaccgcctacatacctcgctctgctaatcctgttaccagtggctgctgccagtggcgataagtcgtgtcttaccgggttggactcaagacgatagttaccggataaggcgcagcggtcgggctgaacggggggttcgtgcacacagcccagcttggagcgaacgacctacaccgaactgagatacctacagcgtgagctatgagaaagcgccacgcttcccgaagggagaaaggcggacaggtatccggtaagcggcagggtcggaacaggagagcgcacgagggagcttccagggggaaacgcctggtatctttatagtcctgtcgggtttcgccacctctgacttgagcgtcgatttttgtgatgctcgtcaggggggcggagcctatggaaaaacgccagcaacgcggcctttttacggttcctggccttttgctggccttttgctcacatgttctttcctgcgttatcccctgattctgtggataaccgtattaccgcctttgagtgagctgataccgctcgccgcagccgaacgaccgagcgcagcgagtcagtgagcgaggaagcggaagagcgcctgatgcggtattttctccttacgcatctgtgcggtatttcacaccgcatatggtgcactctcagtacaatctgctctgatgccgcatagttaagccagtatacactccgctatcgctacgtgactgggtcatggctgcgccccgacacccgccaacacccgctgacgcgccctgacgggcttgtctgctcccggcatccgcttacagacaagctgtgaccgtctccgggagctgcatgtgtcagaggttttcaccgtcatcaccgaaacgcgcgaggcagggtgccttgatgtgggcgccggcggtcgagtggcgacggcgcggcttgtccgcgccctggtagattgcctggccgtaggccagccatttttgagcggccagcggccgcgataggccgacgcgaagcggcggggcgtagggagcgcagcgaccgaagggtaggcgctttttgcagctcttcggctgtgcgctggccagacagttatgcacaggccaggcgggttttaagagttttaataagttttaaagagttttaggcggaaaaatcgccttttttctcttttatatcagtcacttacatgtgtgaccggttcccaatgtacggctttgggttcccaatgtacgggttccggttcccaatgtacggctttgggttcccaatgtacgtgctatccacaggaaagagaccttttcgacctttttcccctgctagggcaatttgccctagcatctgctccgtacattaggaaccggcggatgcttcgccctcgatcaggttgcggtagcgcatgactaggatcgggccagcctgccccgcctcctccttcaaatcgtactccggcaggtcatttgacccgatcagcttgcgcacggtgaaacagaacttcttgaactctccggcgctgccactgcgttcgtagatcgtcttgaacaaccatctggcttctgccttgcctgcggcgcggcgtgccaggcggtagagaaaacggccgatgccgggatcgatcaaaaagtaatcggggtgaaccgtcagcacgtccgggttcttgccttctgtgatctcgcggtacatccaatcagctagctcgatctcgatgtactccggccgcccggtttcgctctttacgatcttgtagcggctaatcaaggcttcaccctcggataccgtcaccaggcggccgttcttggccttcttcgtacgctgcatggcaacgtgcgtggtgtttaaccgaatgcaggtttctaccaggtcgtctttctgctttccgccatcggctcgccggcagaacttgagtacgtccgcaacgtgtggacggaacacgcggccgggcttgtctcccttcccttcccggtatcggttcatggattcggttagatgggaaaccgccatcagtaccaggtcgtaatcccacacactggccatgccggccggccctgcggaaacctctacgtgcccgtctggaagctcgtagcggatcacctcgccagctcgtcggtcacgcttcgacagacggaaaacggccacgtccatgatgctgcgactatcgcgggtgcccacgtcatagagcatcggaacgaaaaaatctggttgctcgtcgcccttgggcggcttcctaatcgacggcgcaccggctgccggcggttgccgggattctttgcggattcgatcagcggccgcttgccacgattcaccggggcgtgcttctgcctcgatgcgttgccgctgggcggcctgcgcggccttcaacttctccaccaggtcatcacccagcgccgcgccgatttgtaccgggccggatggtttgcgaccgtcacgccgattcctcgggcttgggggttccagtgccattgcagggccggcagacaacccagccgcttacgcctggccaaccgcccgttcctccacacatggggcattccacggcgtcggtgcctggttgttcttgattttccatgccgcctcctttagccgctaaaattcatctactcatttattcatttgctcatttactctggtagctgcgcgatgtattcagatagcagctcggtaatggtcttgccttggcgtaccgcgtacatcttcagcttggtgtgatcctccgccggcaactgaaagttgacccgcttcatggctggcgtgtctgccaggctggccaacgttgcagccttgctgctgcgtgcgctcggacggccggcacttagcgtgtttgtgcttttgctcattttctctttacctcattaactcaaatgagttttgatttaatttcagcggccagcgcctggacctcgcgggcagcgtcgccctcgggttctgattcaagaacggttgtgccggcggcggcagtgcctgggtagctcacgcgctgcgtgatacgggactcaagaatgggcagctcgtacccggccagcgcctcggcaacctcaccgccgatgcgcgtgcctttgatcgcccgcgacacgacaaaggccgcttgtagccttccatccgtgacctcaatgcgctgcttaaccagctccaccaggtcggcggtggcccatatgtcgtaagggcttggctgcaccggaatcagcacgaagtcggctgccttgatcgcggacacagccaagtccgccgcctggggcgctccgtcgatcactacgaagtcgcgccggccgatggccttcacgtcgcggtcaatcgtcgggcggtcgatgccgacaacggttagcggttgatcttcccgcacggccgcccaatcgcgggcactgccctggggatcggaatcgactaacagaacatcggccccggcgagttgcagggcgcgggctagatgggttgcgatggtcgtcttgcctgacccgcctttctggttaagtacagcgataaccttcatgcgttccccttgcgtatttgtttatttactcatcgcatcatatacgcagcgaccgcatgacgcaagctgttttactcaaatacacatcacctttttagacggcggcgctcggtttcttcagcggccaagctggccggccaggccgccagcttggcatcagacaaaccggccaggatttcatgcagccgcacggttgagacgtgcgcgggcggctcgaacacgtacccggccgcgatcatctccgcctcgatctcttcggtaatgaaaaacggttcgtcctggccgtcctggtgcggtttcatgcttgttcctcttggcgttcattctcggcggccgccagggcgtcggcctcggtcaatgcgtcctcacggaaggcaccgcgccgcctggcctcggtgggcgtcacttcctcgctgcgctcaagtgcgcggtacagggtcgagcgatgcacgccaagcagtgcagccgcctctttcacggtgcggccttcctggtcgatcagctcgcgggcgtgcgcgatctgtgccggggtgagggtagggcgggggccaaacttcacgcctcgggccttggcggcctcgcgcccgctccgggtgcggtcgatgattagggaacgctcgaactcggcaatgccggcgaacacggtcaacaccatgcggccggccggcgtggtggtgtcggcccacggctctgccaggctacgcaggcccgcgccggcctcctggatgcgctcggcaatgtccagtaggtcgcgggtgctgcgggccaggcggtctagcctggtcactgtcacaacgtcgccagggcgtaggtggtcaagcatcctggccagctccgggcggtcgcgcctggtgccggtgatcttctcggaaaacagcttggtgcagccggccgcgtgcagttcggcccgttggttggtcaagtcctggtcgtcggtgctgacgcgggcatagcccagcaggccagcggcggcgctcttgttcatggcgtaatgtctccggttctagtcgcaagtattctactttatgcgactaaaacacgcgacaagaaaacgccaggaaaagggcagggcggcagcctgtcgcgtaacttaggacttgtgcgacatgtcgttttcagaagacggctgcactgaacgtcagaagccgactgcactatagcagcggaggggttggatcaaagtactttgatcccgaggggaaccctgtggttggcatgcacatacaaatggacgaacggataaaccttttcacgcccttttaaatatccgttattctaataaacgctcttttctcttaggtttacccgccaatatatcctgtcaaacactgatagtttaaactgaaggcgggaaacgacaatctgatccaagctcaagctaagcttgagctctcccatatggtcgagatctcctttgccccggagatcaccatggacgactttctctatctctacgatctaggaagaaagttcgacggagaaggtgacgataccatgttcaccaccgataatgagaagattagcctcttcaatttcagaaagaatgctgacccacagatggttagagaggcctacgcggcaggtctcatcaagacgatctacccgagtaataatctccaggagatcaaataccttcccaagaaggttaaagatgcagtcaaaagattcaggactaactgcatcaagaacacagagaaagatatatttctcaagatcagaagtactattccagtatggacgattcaaggcttgcttcataaaccaaggcaagtaatagagattggagtctctaagaaagtagttcctactgaatcaaaggccatggagtcaaaaattcagatcgaggatctaacagaactcgccgtgaagactggcgaacagttcatacagagtcttttacgactcaatgacaagaagaaaatcttcgtcaacatggtggagcacgacactctcgtctactccaagaatatcaaagatacagtctcagaagaccaaagggctattgagacttttcaacaaagggtaatatcgggaaacctcctcggattccattgcccagctatctgtcacttcatcaaaaggacagtagaaaaggaaggtggcacctacaaatgccatcattgcgataaaggaaaggctatcgttcaagatgcccctgccgacagtggtcccaaagatggacccccacccacgaggagcatcgtggaaaaagaagacgttccaaccacgtcttcaaagcaagtggattgatgtgatatctccactgacgtaagggatgacgcacaatcccactatccttcgcaagacccttcctctatataaggaagttcatttcatttggagaggactccggtatttttacaacaattaccacaacaaaacaaacaacaaacaacattacaatttactattctagtcgacctgcaggcggccgcactagtgatatcacaagtttgtacaaaaaagcaggctgaattcccaccatggcaaacaagcttttcttggtgtgcgctaccttcgctctttgcttccttttgactaacgctcaggttcagctgcaggaatctggtggtggacttgttcagtctggtggatctctcagactctcttgcgtgcactctaagaccaccttcaccagaaatgctatgggatggtacagacaggctctcggaaaagagagagagcttgttgctaccatcacctctggtggaactaccaactacgctgattctgtgaagggaaggttcaccatctctatggattctgctaagaacaccgtgtacctccagatgaactctctcaagcctgaggataccgctgtgtactactgcaacgtgaacaccagaaggatcttcggaggaaccgttagagaatactggggacaaggtactcaggtcaccgtttcttcagcggccgcacatcatcatcaccatcattgaggatccacccagctttcttgtacaaagtggtgatatcccgcggccatgctagagtccgcaaaaatcaccagtctctctctacaaatctatctctctctatttttctccagaataatgtgtgagtagttcccagataagggaattagggttcttatagggtttcgctcatgtgttgagcatataagaaacccttagtatgtatttgtatttgtaaaatacttctatcaataaaatttctaattcctaaaaccaaaatccagtgacctgcaggcatgcgacgtcg

SEQ ID NO: 368 - DNA, 9903 bp, Artificial Sequence
  pK7WG2-35S: cyto_56F11_His
ggccctctagaggatccccgggtaccgcgaattatcatacatgagaattaagggagtcacgttatgacccccgccgatgacgcgggacaagccgttttacgtttggaactgacagaaccgcaacgttgaaggagccactcagccgcgggtttctggagtttaatgagctaagcacatacgtcagaaaccattattgcgcgttcaaaagtcgcctaaggtcactatcagctagcaaatatttcttgtcaaaaatgctccactgacgttccataaattcccctcggtatccaattagagtctcatattcactctcaactcgatcgaggcatgattgaacaagatggattgcacgcaggttctccggccgcttgggtggagaggctattcggctatgactgggcacaacagacaatcggctgctctgatgccgccgtgttccggctgtcagcgcaggggcgcccggttctttttgtcaagaccgacctgtccggtgccctgaatgaactccaagacgaggcagcgcggctatcgtggctggccacgacgggcgttccttgcgcagctgtgctcgacgttgtcactgaagcgggaagggactggctgctattgggcgaagtgccggggcaggatctcctgtcatctcaccttgctcctgccgagaaagtatccatcatggctgatgcaatgcggcggctgcatacgcttgatccggctacctgcccattcgaccaccaagcgaaacatcgcatcgagcgaggacgtactcggatggaagccggtcttgtcgatcaggatgatctggacgaagagcatcaggggctcgcgccagccgaactgttcgccaggctcaaggcgcggatgcccgacggcgaggatctcgtcgtgacccagggcgatgcctgcttgccgaatatcatggtggaaaatggccgcttttctggattcatcgactgtggccggctgggtgtggcggaccgctatcaggacatagcgttggctacccgtgatattgctgaagagcttggcggcgaatgggctgaccgcttcctcgtgctttacggtatcgccgctcccgattcgcagcgcatcgccttctatcgccttcttgacgagttcttctgagcgggactctggggttcggactctagctagagtcaagcagatcgttcaaacatttggcaataaagtttcttaagattgaatcctgttgccggtcttgcgatgattatcatataatttctgttgaattacgttaagcatgtaataattaacatgtaatgcatgacgttatttatgagatgggttttttgattagagtcccgcaattatacatttaatacgcgatagaaaacaaaatatagcgcgcaaactaggataaattatcgcgcgcggtgtcatctatgttactagatcgaccggcatgcaagctgataattcaattcggcgttaattcagtacattaaaaacgtccgcaatgtgttattaagttgtctaagcgtcaatttgtttacaccacaatatatcctgccaccagccagccaacagctccccgaccggcagctcggcacaaaatcaccactcgatacaggcagcccatcagtccgggacggcgtcagcgggagagccgttgtaaggcggcagactttgctcatgttaccgatgctattcggaagaacggcaactaagctgccgggtttgaaacacggatgatctcgcggagggtagcatgttgattgtaacgatgacagagcgttgctgcctgtgatcaattcgggcacgaacccagtggacataagcctcgttcggttcgtaagctgtaatgcaagtagcgtaactgccgtcacgcaactggtccagaaccttgaccgaacgcagcggtggtaacggcgcagtggcggttttcatggcttcttgttatgacatgtttttttggggtacagtctatgcctcgggcatccaagcagcaagcgcgttacgccgtgggtcgatgtttgatgttatggagcagcaacgatgttacgcagcagggcagtcgccctaaaacaaagttaaacatcatgggggaagcggtgatcgccgaagtatcgactcaactatcagaggtagttggcgtcatcgagcgccatctcgaaccgacgttgctggccgtacatttgtacggctccgcagtggatggcggcctgaagccacacagtgatattgatttgctggttacggtgaccgtaaggcttgatgaaacaacgcggcgagctttgatcaacgaccttttggaaacttcggcttcccctggagagagcgagattctccgcgctgtagaagtcaccattgttgtgcacgacgacatcattccgtggcgttatccagctaagcgcgaactgcaatttggagaatggcagcgcaatgacattcttgcaggtatcttcgagccagccacgatcgacattgatctggctatcttgctgacaaaagcaagagaacatagcgttgccttggtaggtccagcggcggaggaactctttgatccggttcctgaacaggatctatttgaggcgctaaatgaaaccttaacgctatggaactcgccgcccgactgggctggcgatgagcgaaatgtagtgcttacgttgtcccgcatttggtacagcgcagtaaccggcaaaatcgcgccgaaggatgtcgctgccgactgggcaatggagcgcctgccggcccagtatcagcccgtcatacttgaagctagacaggcttatcttggacaagaagaagatcgcttggcctcgcgcgcagatcagttggaagaatttgtccactacgtgaaaggcgagatcaccaaggtagtcggcaaataatgtctagctagaaattcgttcaagccgacgccgcttcgccggcgttaactcaagcgattagatgcactaagcacataattgctcacagccaaactatcaggtcaagtctgcttttattatttttaagcgtgcataataagccctacacaaattgggagatatatcatgcatgaccaaaatcccttaacgtgagttttcgttccactgagcgtcagaccccgtagaaaagatcaaaggatcttcttgagatcctttttttctgcgcgtaatctgctgcttgcaaacaaaaaaaccaccgctaccagcggtggtttgtttgccggatcaagagctaccaactctttttccgaaggtaactggcttcagcagagcgcagataccaaatactgtccttctagtgtagccgtagttaggccaccacttcaagaactctgtagcaccgcctacatacctcgctctgctaatcctgttaccagtggctgctgccagtggcgataagtcgtgtcttaccgggttggactcaagacgatagttaccggataaggcgcagcggtcgggctgaacggggggttcgtgcacacagcccagcttggagcgaacgacctacaccgaactgagatacctacagcgtgagctatgagaaagcgccacgcttcccgaagggagaaaggcggacaggtatccggtaagcggcagggtcggaacaggagagcgcacgagggagcttccagggggaaacgcctggtatctttatagtcctgtcgggtttcgccacctctgacttgagcgtcgatttttgtgatgctcgtcaggggggcggagcctatggaaaaacgccagcaacgcggcctttttacggttcctggccttttgctggccttttgctcacatgttctttcctgcgttatcccctgattctgtggataaccgtattaccgcctttgagtgagctgataccgctcgccgcagccgaacgaccgagcgcagcgagtcagtgagcgaggaagcggaagagcgcctgatgcggtattttctccttacgcatctgtgcggtatttcacaccgcatatggtgcactctcagtacaatctgctctgatgccgcatagttaagccagtatacactccgctatcgctacgtgactgggtcatggctgcgccccgacacccgccaacacccgctgacgcgccctgacgggcttgtctgctcccggcatccgcttacagacaagctgtgaccgtctccgggagctgcatgtgtcagaggttttcaccgtcatcaccgaaacgcgcgaggcagggtgccttgatgtgggcgccggcggtcgagtggcgacggcgcggcttgtccgcgccctggtagattgcctggccgtaggccagccatttttgagcggccagcggccgcgataggccgacgcgaagcggcggggcgtagggagcgcagcgaccgaagggtaggcgctttttgcagctcttcggctgtgcgctggccagacagttatgcacaggccaggcgggttttaagagttttaataagttttaaagagttttaggcggaaaaatcgccttttttctcttttatatcagtcacttacatgtgtgaccggttcccaatgtacggctttgggttcccaatgtacgggttccggttcccaatgtacggctttgggttcccaatgtacgtgctatccacaggaaagagaccttttcgacctttttcccctgctagggcaatttgccctagcatctgctccgtacattaggaaccggcggatgcttcgccctcgatcaggttgcggtagcgcatgactaggatcgggccagcctgccccgcctcctccttcaaatcgtactccggcaggtcatttgacccgatcagcttgcgcacggtgaaacagaacttcttgaactctccggcgctgccactgcgttcgtagatcgtcttgaacaaccatctggcttctgccttgcctgcggcgcggcgtgccaggcggtagagaaaacggccgatgccgggatcgatcaaaaagtaatcggggtgaaccgtcagcacgtccgggttcttgccttctgtgatctcgcggtacatccaatcagctagctcgatctcgatgtactccggccgcccggtttcgctctttacgatcttgtagcggctaatcaaggcttcaccctcggataccgtcaccaggcggccgttcttggccttcttcgtacgctgcatggcaacgtgcgtggtgtttaaccgaatgcaggtttctaccaggtcgtctttctgctttccgccatcggctcgccggcagaacttgagtacgtccgcaacgtgtggacggaacacgcggccgggcttgtctcccttcccttcccggtatcggttcatggattcggttagatgggaaaccgccatcagtaccaggtcgtaatcccacacactggccatgccggccggccctgcggaaacctctacgtgcccgtctggaagctcgtagcggatcacctcgccagctcgtcggtcacgcttcgacagacggaaaacggccacgtccatgatgctgcgactatcgcgggtgcccacgtcatagagcatcggaacgaaaaaatctggttgctcgtcgcccttgggcggcttcctaatcgacggcgcaccggctgccggcggttgccgggattctttgcggattcgatcagcggccgcttgccacgattcaccggggcgtgcttctgcctcgatgcgttgccgctgggcggcctgcgcggccttcaacttctccaccaggtcatcacccagcgccgcgccgatttgtaccgggccggatggtttgcgaccgtcacgccgattcctcgggcttgggggttccagtgccattgcagggccggcagacaacccagccgcttacgcctggccaaccgcccgttcctccacacatggggcattccacggcgtcggtgcctggttgttcttgattttccatgccgcctcctttagccgctaaaattcatctactcatttattcatttgctcatttactctggtagctgcgcgatgtattcagatagcagctcggtaatggtcttgccttggcgtaccgcgtacatcttcagcttggtgtgatcctccgccggcaactgaaagttgacccgcttcatggctggcgtgtctgccaggctggccaacgttgcagccttgctgctgcgtgcgctcggacggccggcacttagcgtgtttgtgcttttgctcattttctctttacctcattaactcaaatgagttttgatttaatttcagcggccagcgcctggacctcgcgggcagcgtcgccctcgggttctgattcaagaacggttgtgccggcggcggcagtgcctgggtagctcacgcgctgcgtgatacgggactcaagaatgggcagctcgtacccggccagcgcctcggcaacctcaccgccgatgcgcgtgcctttgatcgcccgcgacacgacaaaggccgcttgtagccttccatccgtgacctcaatgcgctgcttaaccagctccaccaggtcggcggtggcccatatgtcgtaagggcttggctgcaccggaatcagcacgaagtcggctgccttgatcgcggacacagccaagtccgccgcctggggcgctccgtcgatcactacgaagtcgcgccggccgatggccttcacgtcgcggtcaatcgtcgggcggtcgatgccgacaacggttagcggttgatcttcccgcacggccgcccaatcgcgggcactgccctggggatcggaatcgactaacagaacatcggccccggcgagttgcagggcgcgggctagatgggttgcgatggtcgtcttgcctgacccgcctttctggttaagtacagcgataaccttcatgcgttccccttgcgtatttgtttatttactcatcgcatcatatacgcagcgaccgcatgacgcaagctgttttactcaaatacacatcacctttttagacggcggcgctcggtttcttcagcggccaagctggccggccaggccgccagcttggcatcagacaaaccggccaggatttcatgcagccgcacggttgagacgtgcgcgggcggctcgaacacgtacccggccgcgatcatctccgcctcgatctcttcggtaatgaaaaacggttcgtcctggccgtcctggtgcggtttcatgcttgttcctcttggcgttcattctcggcggccgccagggcgtcggcctcggtcaatgcgtcctcacggaaggcaccgcgccgcctggcctcggtgggcgtcacttcctcgctgcgctcaagtgcgcggtacagggtcgagcgatgcacgccaagcagtgcagccgcctctttcacggtgcggccttcctggtcgatcagctcgcgggcgtgcgcgatctgtgccggggtgagggtagggcgggggccaaacttcacgcctcgggccttggcggcctcgcgcccgctccgggtgcggtcgatgattagggaacgctcgaactcggcaatgccggcgaacacggtcaacaccatgcggccggccggcgtggtggtgtcggcccacggctctgccaggctacgcaggcccgcgccggcctcctggatgcgctcggcaatgtccagtaggtcgcgggtgctgcgggccaggcggtctagcctggtcactgtcacaacgtcgccagggcgtaggtggtcaagcatcctggccagctccgggcggtcgcgcctggtgccggtgatcttctcggaaaacagcttggtgcagccggccgcgtgcagttcggcccgttggttggtcaagtcctggtcgtcggtgctgacgcgggcatagcccagcaggccagcggcggcgctcttgttcatggcgtaatgtctccggttctagtcgcaagtattctactttatgcgactaaaacacgcgacaagaaaacgccaggaaaagggcagggcggcagcctgtcgcgtaacttaggacttgtgcgacatgtcgttttcagaagacggctgcactgaacgtcagaagccgactgcactatagcagcggaggggttggatcaaagtactttgatcccgaggggaaccctgtggttggcatgcacatacaaatggacgaacggataaaccttttcacgcccttttaaatatccgttattctaataaacgctcttttctcttaggtttacccgccaatatatcctgtcaaacactgatagtttaaactgaaggcgggaaacgacaatctgatccaagctcaagctaagcttgagctctcccatatggtcgagatctcctttgccccggagatcaccatggacgactttctctatctctacgatctaggaagaaagttcgacggagaaggtgacgataccatgttcaccaccgataatgagaagattagcctcttcaatttcagaaagaatgctgacccacagatggttagagaggcctacgcggcaggtctcatcaagacgatctacccgagtaataatctccaggagatcaaataccttcccaagaaggttaaagatgcagtcaaaagattcaggactaactgcatcaagaacacagagaaagatatatttctcaagatcagaagtactattccagtatggacgattcaaggcttgcttcataaaccaaggcaagtaatagagattggagtctctaagaaagtagttcctactgaatcaaaggccatggagtcaaaaattcagatcgaggatctaacagaactcgccgtgaagactggcgaacagttcatacagagtcttttacgactcaatgacaagaagaaaatcttcgtcaacatggtggagcacgacactctcgtctactccaagaatatcaaagatacagtctcagaagaccaaagggctattgagacttttcaacaaagggtaatatcgggaaacctcctcggattccattgcccagctatctgtcacttcatcaaaaggacagtagaaaaggaaggtggcacctacaaatgccatcattgcgataaaggaaaggctatcgttcaagatgcccctgccgacagtggtcccaaagatggacccccacccacgaggagcatcgtggaaaaagaagacgttccaaccacgtcttcaaagcaagtggattgatgtgatatctccactgacgtaagggatgacgcacaatcccactatccttcgcaagacccttcctctatataaggaagttcatttcatttggagaggactccggtatttttacaacaattaccacaacaaaacaaacaacaaacaacattacaatttactattctagtcgacctgcaggcggccgcactagtgatatcacaagtttgtacaaaaaagcaggctgaattcccaccatgcaggttcagctgcaggaatctggtggtggacttgttcagtctggtggatctctcagactctcttgcgtgcactctaagaccaccttcaccagaaatgctatgggatggtacagacaggctctcggaaaagagagagagcttgttgctaccatcacctctggtggaactaccaactacgctgattctgtgaagggaaggttcaccatctctatggattctgctaagaacaccgtgtacctccagatgaactctctcaagcctgaggataccgctgtgtactactgcaacgtgaacaccagaaggatcttcggaggaaccgttagagaatactggggacaaggtactcaggtcaccgtttcttcagcggccgcacatcatcatcaccatcattgaggatccacccagctttcttgtacaaagtggtgatatcccgcggccatgctagagtccgcaaaaatcaccagtctctctctacaaatctatctctctctatttttctccagaataatgtgtgagtagttcccagataagggaattagggttcttatagggtttcgctcatgtgttgagcatataagaaacccttagtatgtatttgtatttgtaaaatacttctatcaataaaatttctaattcctaaaaccaaaatccagtgacctgcaggcatgcgacgtcg